European Patent Specification EP 3 891 274 B1, published October 18, 2023. Title: COMPOSITIONS AND METHODS FOR TREATING ORNITHINE TRANSCARBAMYLASE DEFICIENCY. Applicant: ARCTURUS THERAPEUTICS, INC. The sequence listing filed with the application follows.

SEQUENCE LISTING (253 sequences)

SEQ ID NO: 1 - RNA, 1065 nt, Homo sapiens
augcuguuuaaucugaggauccuguuaaacaaugcagcuuuuagaaauggucacaacuucaugguucgaaauuuucgguguggacaaccacuacaaaauaaagugcagcugaagggccgugaccuucucacucuaaaaaacuuuaccggagaagaaauuaaauauaugcuauggcuaucagcagaucugaaauuuaggauaaaacagaaaggagaguauuugccuuuauugcaagggaaguccuuaggcaugauuuuugagaaaagaaguacucgaacaagauugucuacagaaacaggcuuugcacuucugggaggacauccuuguuuucuuaccacacaagauauucauuugggugugaaugaaagucucacggacacggcccguguauugucuagcauggcagaugcaguauuggcucgaguguauaaacaaucagauuuggacacccuggcuaaagaagcauccaucccaauuaucaaugggcugucagauuuguaccauccuauccagauccuggcugauuaccucacgcuccaggaacacuauagcucucugaaaggucuuacccucagcuggaucggggaugggaacaauauccugcacuccaucaugaugagcgcagcgaaauucggaaugcaccuucaggcagcuacuccaaaggguuaugagccggaugcuaguguaaccaaguuggcagagcaguaugccaaagagaaugguaccaagcuguugcugacaaaugauccauuggaagcagcgcauggaggcaauguauuaauuacagacacuuggauaagcaugggacaagaagaggagaagaaaaagcggcuccaggcuuuccaagguuaccagguuacaaugaagacugcuaaaguugcugccucugacuggacauuuuuacacugcuugcccagaaagccagaagaaguggaugaugaagucuuuuauucuccucgaucacuaguguucccagaggcagaaaacagaaaguggacaaucauggcugucauggugucccugcugacagauuacucaccucagcuccagaagccuaaauuuuga

SEQ ID NO: 2 - DNA, 1065 bp, Homo sapiens
atgctgtttaatctgaggatcctgttaaacaatgcagcttttagaaatggtcacaacttcatggttcgaaattttcggtgtggacaaccactacaaaataaagtgcagctgaagggccgtgaccttctcactctaaaaaactttaccggagaagaaattaaatatatgctatggctatcagcagatctgaaatttaggataaaacagaaaggagagtatttgcctttattgcaagggaagtccttaggcatgatttttgagaaaagaagtactcgaacaagattgtctacagaaacaggctttgcacttctgggaggacatccttgttttcttaccacacaagatattcatttgggtgtgaatgaaagtctcacggacacggcccgtgtattgtctagcatggcagatgcagtattggctcgagtgtataaacaatcagatttggacaccctggctaaagaagcatccatcccaattatcaatgggctgtcagatttgtaccatcctatccagatcctggctgattacctcacgctccaggaacactatagctctctgaaaggtcttaccctcagctggatcggggatgggaacaatatcctgcactccatcatgatgagcgcagcgaaattcggaatgcaccttcaggcagctactccaaagggttatgagccggatgctagtgtaaccaagttggcagagcagtatgccaaagagaatggtaccaagctgttgctgacaaatgatccattggaagcagcgcatggaggcaatgtattaattacagacacttggataagcatgggacaagaagaggagaagaaaaagcggctccaggctttccaaggttaccaggttacaatgaagactgctaaagttgctgcctctgactggacatttttacactgcttgcccagaaagccagaagaagtggatgatgaagtcttttattctcctcgatcactagtgttcccagaggcagaaaacagaaagtggacaatcatggctgtcatggtgtccctgctgacagattactcacctcagctccagaagcctaaattttga

SEQ ID NO: 3 - protein, 353 aa, Homo sapiens
MLFNLRILLNNAAFRNGHNFMVRNFRCGQPLQNKVQLKGRDLLTLKNFTGEEIKYMLWLSADLKFRIKQKGEYLPLLQGKSLGMIFEKRSTRTRLSTETGFALLGGHPCFLTTQDIHLGVNESLTDTARVLSSMADAVLARVYKQSDLDTLAKEASIPIFGLSDLYHPIQILADYLTLQEHYSSLKGLTLSWIGDGNNILHSIMMSAAKFGMHLQAATPKGYEPDASVTKLAEQYAKENGTKLLLTNDPLEAAHGGNVLITDTWISMGQEEEKKKRLQAFQGYQVTMKTAKVAASDWTFLHCLPRKPEEVDDEVFYSPRSLVFPEAENRKWTIMAVMVSLLTDYSPQLQKPKF

SEQ ID NO: 4 - protein, 355 aa, Artificial Sequence
  Synthetic construct
MLVFNLRILLNNAAFRNGHNFMVRNFRCGQPLQNRVQLKGRDLLTLKNFTGEEIRYMLWLSADLKFRIKQKGEYLPLLQGKSLGMIFEKRSTRTRLSTETGFALLGGHPCFLTTQDIHLGVNESLTDTARVLSSMADAVLARVYKQSDLDTLAKEASIPIINGLSDLYHPIQILADYLTLQEHYSSLKGLTLSWIGDGNNILHSIMMSAAKFGMHLQAATPKGYEPDASVTKLAEQYAKENGTKLLLTNDPLEAAHGGNVLITDTWISMGQEEEKKKRLQAFQGYQVTMKTAKVAASDWTFLHCLPRKPEEVDDEVFYSPRSLVFPEAENRKWTIMAVMVSLLTDYSPQLQKPKF

SEQ ID NO: 5 - RNA, 129 nt, Artificial Sequence
  Synthetic construct
ucaacacaacauauacaaaacaaacgaaucucaagcaaucaagcauucuacuucuauugcagcaauuuaaaucauuucuuuuaaagcaaaagcaauuuucugaaaauuuucaccauuuacgaacgauag

SEQ ID NO: 6 - RNA, 28 nt, Artificial Sequence
  Synthetic construct
auuauuacaucaaaacaaaaagccgcca

SEQ ID NO: 7 - RNA, 245 nt, Artificial Sequence
  Synthetic construct
cuuaagggggcgcugccuacggagguggcagccaucuccuucucggcaucaagcuuaccauggugccccaggcccugcucuuggucccgcugcugguguucccccucugcuucggcaaguuccccaucuacaccauccccgacaagcuggggccguggagccccaucgacauccaccaccuguccugccccaacaaccucguggucgaggacgagggcugcaccaaccugagcggguucuccuac

SEQ ID NO: 8 - RNA, 177 nt, Artificial Sequence
  Synthetic construct
ugagugucguacagccuccaggccccccccucccgggagagccauaguggucugcggaaccggugaguacaccggaauugccgggaagacuggguccuuucuuggauaaacccacucuaugcccggccauuugggcgugcccccgcaagacugcuagccgaguaguguuggguugcg

SEQ ID NO: 9 - RNA, 89 nt, Artificial Sequence
  Synthetic construct
aauuauugguuaaagaaguauauuagugcuaauuucccuccguuuguccuagcuuuucucuucugucaaccccacacgccuuuggcaca

SEQ ID NO: 10 - RNA, 569 nt, Artificial Sequence
  Synthetic construct
cucccuccccccccccuaacguuacuggccgaagccgcuuggaauaaggccggugugcguuugucuauauguuauuuuccaccauauugccgucuuuuggcaaugugagggcccggaaaccuggcccugucuucuugacgagcauuccuaggggucuuuccccucucgccaaaggaaugcaaggucuguugaaugucgugaaggaagcaguuccucuggaagcuucuugaagacaaacaacgucuguagcgacccuuugcaggcagcggaaccccccaccuggcgacaggugccucugcggccaaaagccacguguauaagauacaccugcaaaggcggcacaaccccagugccacguugugaguuggauaguuguggaaagagucaaauggcucuccucaagcguauucaacaaggggcugaaggaugcccagaagguaccccauuguaugggaucugaucuggggccucggugcacaugcuuuacguguguuuagucgagguuaaaaaacgucuaggccccccgaaccacggggacgugguuuuccuuugaaaaacacgaugauaau

SEQ ID NO: 11 - RNA, 44 nt, Artificial Sequence
  Synthetic construct
gucagcuuucaaacucuuuguuucuuguuuguugauugagaaua

SEQ ID NO: 12 - RNA, 54 nt, Artificial Sequence
  Synthetic construct
cucucgccugagaaaaaaaauccacgaaccaauuucucagcaaccagcagcacg

SEQ ID NO: 13 - RNA, 52 nt, Artificial Sequence
  Synthetic construct
accugugaggguucgaaggaaguagcaguguuuuuuguuccuagaggaagag

SEQ ID NO: 14 - RNA, 71 nt, Artificial Sequence
  Synthetic construct
acacagaaacauucgcaaaaacaaaaucccaguaucaaaauucuucucuuuuuuucauauuucgcaaagac

SEQ ID NO: 15 - RNA, 52 nt, Artificial Sequence
  Synthetic construct
cagaaaaauuugcuacauuguuucacaaacuucaaauauuauucauuuauuu

SEQ ID NO: 16 - RNA, 158 nt, Artificial Sequence
  Synthetic construct
cuagugacugacuaggaucugguuaccacuaaaccagccucaagaacacccgaauggagucucuaagcuacauaauaccaacuuacacuuacaaaauguugucccccaaaauguagccauucguaucugcuccuaauaaaaagaaaguuucuucacau

SEQ ID NO: 17 - RNA, 166 nt, Artificial Sequence
  Synthetic construct
ugcaaggcuggccggaagcccuugccugaaagcaagauuucagccuggaagagggcaaaguggacgggaguggacaggaguggaugcgauaagaugugguuugaagcugaugggugccagcccugcauugcugagucaaucaauaaagagcuuucuuuugacccau

SEQ ID NO: 18 - RNA, 143 nt, Artificial Sequence
  Synthetic construct
acgccgaagccugcagccaugcgaccccacgccaccccgugccuccugccuccgcgcagccugcagcgggagacccuguccccgccccagccguccuccugggguggacccuaguuuaauaaagauucaccaaguuucacgca

SEQ ID NO: 19 - RNA, 220 nt, Artificial Sequence
  Synthetic construct
uagagcggcaaacccuagcuacacuccauagcuaguuucuuuuuuuuuuguuuuuuuuuuuuuuuuuuuuuuuuuuuuuuuuuuuuuuuccuuucuuuuccuucuuuuuuuccucuuuucuugguggcuccaucuuagcccuagucacggcuagcugugaaagguccgugagccgcaugacugcagagagugccguaacuggucucucugcagaucaugu

SEQ ID NO: 20 - RNA, 170 nt, Artificial Sequence
  Synthetic construct
acacaucacaaccacaaccuucucaggcuacccugagaaaaaaagacaugaagacucaggacucaucuuuucuguugguguaaaaucaacacccuaaggaacacaaauuucuuuaaacauuugacuucuugucucugugcugcaauuaauaaaaaauggaaagaaucuac

SEQ ID NO: 21 - RNA, 110 nt, Artificial Sequence
  Synthetic construct
gcuggagccucgguagccguuccuccugcccgcugggccucccaacgggcccuccuccccuccuugcaccggcccuuccuggucuuugaauaaagucugagugggcagca

SEQ ID NO: 22 - RNA, 123 nt, Artificial Sequence
  Synthetic construct
uagugcagucacuggcacaacgcguugcccgguaagccaaucggguauacacggucgucauacugcagacaggguucuucuacuuugcaagauagucuagaguaguaaaauaaauaguauaag

SEQ ID NO: 23 - RNA, 6 nt, Artificial Sequence
  Synthetic construct
gccacc

SEQ ID NO: 24 - RNA, 4 nt, Artificial Sequence
  Synthetic construct
gcca

SEQ ID NO: 25 - RNA, 9 nt, Artificial Sequence
  Synthetic construct
auaagugaa

SEQ ID NO: 26 - RNA, 1368 nt, Artificial Sequence
  Synthetic construct
ucaacacaacauauacaaaacaaacgaaucucaagcaaucaagcauucuacuucuauugcagcaauuuaaaucauuucuuuuaaagcaaaagcaauuuucugaaaauuuucaccauuuacgaacgauagccaccaugcuguuuaaucugaggauccuguuaaacaaugcagcuuuuagaaauggucacaacuucaugguucgaaauuuucgguguggacaaccacuacaaaauaaagugcagcugaagggccgugaccuucucacucuaaaaaacuuuaccggagaagaaauuaaauauaugcuauggcuaucagcagaucugaaauuuaggauaaaacagaaaggagaguauuugccuuuauugcaagggaaguccuuaggcaugauuuuugagaaaagaaguacucgaacaagauugucuacagaaacaggcuuugcacuucugggaggacauccuuguuuucuuaccacacaagauauucauuugggugugaaugaaagucucacggacacggcccguguauugucuagcauggcagaugcaguauuggcucgaguguauaaacaaucagauuuggacacccuggcuaaagaagcauccaucccaauuaucaaugggcugucagauuuguaccauccuauccagauccuggcugauuaccucacgcuccaggaacacuauagcucucugaaaggucuuacccucagcuggaucggggaugggaacaauauccugcacuccaucaugaugagcgcagcgaaauucggaaugcaccuucaggcagcuacuccaaaggguuaugagccggaugcuaguguaaccaaguuggcagagcaguaugccaaagagaaugguaccaagcuguugcugacaaaugauccauuggaagcagcgcauggaggcaauguauuaauuacagacacuuggauaagcaugggacaagaagaggagaagaaaaagcggcuccaggcuuuccaagguuaccagguuacaaugaagacugcuaaaguugcugccucugacuggacauuuuuacacugcuugcccagaaagccagaagaaguggaugaugaagucuuuuauucuccucgaucacuaguguucccagaggcagaaaacagaaaguggacaaucauggcugucauggugucccugcugacagauuacucaccucagcuccagaagccuaaauuuugacucgagcuagugacugacuaggaucugguuaccacuaaaccagccucaagaacacccgaauggagucucuaagcuacauaauaccaacuuacacuuacaaaauguugucccccaaaauguagccauucguaucugcuccuaauaaaaagaaaguuucuucacauucuag

SEQ ID NO: 27 - RNA, 1368 nt, Artificial Sequence
  Synthetic construct
ucaacacaacauauacaaaacaaacgaaucucaagcaaucaagcauucuacuucuauugcagcaauuuaaaucauuucuuuuaaagcaaaagcaauuuucugaaaauuuucaccauuuacgaacgauagccaccaugcucuuuaaucugcgcaucuuacugaacaacgccgcauuccggaacggucacaacuucaugguccgcaauuuccgcuguggccagccgcuucaaaacaagguccagcugaagggacgggaucugcugacacugaagaacuucaccggagaagagaucaaguacaugcuguggcucagcgcagacuugaaguuccggaucaagcagaagggagaauacuugccccugcugcaaggaaagucgcugggaaugauuuuugagaagcggucaacucgcaccagacucuccaccgaaacugguuucgcacugcuuggcgggcacccuugcuuccugacgacucaggacauccaccucggcgugaacgaaucgcuaaccgauaccgccagagugcuuucuuccauggccgacgcggugcuggccaggguguacaagcaguccgaccucgauaccuuggcaaaggaggcuuccauucccaucaucaacggccugagcgaccuguaccacccaauccaaauccuggcugacuaccugacccugcaagagcacuacagcagccugaagggucugacccugucauggauuggcgauggaaacaauauucugcacuccaucaugauguccgccgcgaaguucggaaugcaucugcaagccgccacuccaaaaggauacgaaccggaugcguccgugaccaaguuggcggaacaguacgcgaaggagaacggaaccaagcuucugcugacuaacgacccccucgaggcugcgcaugggggcaacgugcugauuaccgacaccuggaucuccauggggcaggaggaagagaagaagaagagacugcaggcauuccagggguaccaggucaccaugaaaaccgcaaaaguggcagcuucggacuggacuuuccugcauugccugccgaggaagccggaggaagucgacgacgaaguguucuacucgccucggucccugguguuccccgaggccgaaaaccggaaguggaccaucauggccgugaugguguccuugcugacugacuauagcccgcagcugcagaagccuaaguucuagcucgagcuagugacugacuaggaucugguuaccacuaaaccagccucaagaacacccgaauggagucucuaagcuacauaauaccaacuuacacuuacaaaauguugucccccaaaauguagccauucguaucugcuccuaauaaaaagaaaguuucuucacauucuag

SEQ ID NO: 28 - RNA, 1368 nt, Artificial Sequence
  Synthetic construct
ucaacacaacauauacaaaacaaacgaaucucaagcaaucaagcauucuacuucuauugcagcaauuuaaaucauuucuuuuaaagcaaaagcaauuuucugaaaauuuucaccauuuacgaacgauagccaccaugcuguuuaaccuacguauuuugcucaacaaugcagccuuuagaaacggacauaacuuuaugguucgaaacuuucgcugcgggcagccacugcagaacaagguccagcugaaagggagagauuugcucacgcugaagaacuuuacuggcgaagaaaucaaguauaugcugugguuguccgcggaccucaaguuucggauuaagcagaaaggggaguaucugccacugcugcaaggaaagagccucggcaugaucuucgagaagcggagcacucggaccaggcugaguaccgaaacuggcuucgcauuguuggguggacauccauguuuucugacaacgcaggacauucaucugggcgugaacgagagucugacggacacagcucgcguucuguccucuauggcugaugcgguguuggcccgggucuauaagcaguccgauuuggacaccuuggcuaaggaagcuagcauaccgauuaucaaugggcuguccgaccuguaucacccuauucaaauccuggccgacuaccucacacugcaagaacacuauagcucauugaagggacugacccugagcuggauaggggacggaaacaacauccuacauagcauuaugauguccgcugccaaguuuggcaugcaucuucaagccgccacgccaaaggguuaugagcccgacgcgucagugacaaagcuggccgagcaguacgcuaaggagaaugguaccaaauuacugcugacuaaugauccacuggaggcugcacauggcggcaauguacugaucaccgacacauggaucucgaugggccaggaggaagaaaagaagaagaggcuucaggccuuccaaggcuaccaggucaccaugaaaacagcuaagguugcagcaucugauuggaccuuucugcacugucugccaaggaagcccgaagagguggacgaugaaguauucuauagcccacggaguuugguguucccugaggcugaaaauaggaaguggacaauuauggccguaauggugucccuguuaaccgacuacucuccgcaacugcagaaaccuaaguuuuagcucgagcuagugacugacuaggaucugguuaccacuaaaccagccucaagaacacccgaauggagucucuaagcuacauaauaccaacuuacacuuacaaaauguugucccccaaaauguagccauucguaucugcuccuaauaaaaagaaaguuucuucacauucuag

SEQ ID NO: 29 - RNA, 1368 nt, Artificial Sequence
  Synthetic construct
ucaacacaacauauacaaaacaaacgaaucucaagcaaucaagcauucuacuucuauugcagcaauuuaaaucauuucuuuuaaagcaaaagcaauuuucugaaaauuuucaccauuuacgaacgauagccaccaugcuguuuaacuuaaggauccugcugaacaacgccgcuuuucguaacggucauaacuuuaugguccggaacuuuagauguggccagccgcugcagaacaagguucagcugaaggggagggaucugcugaccuugaagaacuuuaccggcgaagagaucaaguacauguuguggcugagcgccgaucugaaguuuaggauuaagcagaagggggaguauuugccacugcugcaaggaaaauccuuggggaugaucuucgagaagcgcuccacuagaacccggcuaagcacagaaaccggcuucgcacuucuggguggacaucccuguuuucugacgacgcaggauauacaccugggcgugaaugagagucugacggacacagcuaggguguugagcagcauggccgaugcaguacuggcccgcguuuauaagcagagcgacuuggacacacuggccaaggaagcgucaauuccgauuaucaaugggcugucagaccuguaucaucccauucaaaucuuggcugacuaucugacccugcaagaacauuacagcucccugaagggccucacguuguccuggauuggcgacggaaacaacauucugcauucgaucaugaugagcgcugcuaaguuuggcaugcaccuccaagccgcuacaccuaagggauaugagccugaugccagcguaaccaagcuggccgaacaguacgcgaaggagaauggcacgaaacugcuguugacaaaugacccacuggaggcagcucacgguggcaacgugcugaucaccgacacguggauaucuaugggacaggaagaagagaagaagaagcggcugcaggcauuccaaggguaucaggucaccaugaaaacggccaagguugcugcauccgacuggacauuucugcauugcuugccccgcaaaccagaagaaguagacgacgaagucuuuuauuccccacggucgcugguguuccccgaggcggagaaucgaaaguggacgauuauggccgugauggugucccugcugacugauuacucuccccaacugcaaaagccuaaguuuuagcucgagcuagugacugacuaggaucugguuaccacuaaaccagccucaagaacacccgaauggagucucuaagcuacauaauaccaacuuacacuuacaaaauguugucccccaaaauguagccauucguaucugcuccuaauaaaaagaaaguuucuucacauucuag

SEQ ID NO: 30 - RNA, 1368 nt, Artificial Sequence
  Synthetic construct
ucaacacaacauauacaaaacaaacgaaucucaagcaaucaagcauucuacuucuauugcagcaauuuaaaucauuucuuuuaaagcaaaagcaauuuucugaaaauuuucaccauuuacgaacgauagccaccaugcuuuucaaccugaggauccuccugaacaacgccgccuuucgcaauggucacaacuuuaugguccggaacuucagaugcggccagccgcugcagaacaagguccagcugaagggacgggaucugcugacucugaagaacuucaccggagaagagaucaaguacaugcuguggcugucggccgaccugaaguucaggaucaagcagaagggagaauaccucccgcugcugcaaggaaagucccugggcaugauuuucgagaagcgcucgaccagaacucgguuguccaccgaaaccggguuugcgcugcugggcggacauccuugcuuccugacgacucaggauauucaccugggagugaacgagucgcugaccgacaccgccagagugcugagcucgauggccgacgccguguuggcacgcguguacaagcaguccgaucuggauacccuggccaaagaagcuuccaucccgaucauuaacgggcugagcgaccucuaccaccccauucaaauccuggccgacuaccugacucugcaagaacacuacagcucgcugaagggguugacucuguccuggaucggcgacggaaacaacauccugcacuccaucaugaugucggccgcaaaguucggcaugcauuugcaagccgccaccccaaagggcuacgaaccagacgcgagcgucaccaagcuggccgaacaguacgcgaaggaaaaugguacuaagcugcugcugaccaacgacccauuggaagcugcccaugguggaaacgugcugaucaccgacaccuggaucucgaugggccaggaagaggagaagaagaagcggcugcaggcguuccagggguaucaggucaccaugaaaacagccaaaguggcagcgucagacuggaccuuccuccacugucugccucgcaagccagaggagguggacgacgagguguucuacuccccucggucccucguguucccugaggcugagaaccggaaguggaccauuauggccgugauggugucacuccugacugauuacuccccgcaacugcagaagcccaaguucuagcucgagcuagugacugacuaggaucugguuaccacuaaaccagccucaagaacacccgaauggagucucuaagcuacauaauaccaacuuacacuuacaaaauguugucccccaaaauguagccauucguaucugcuccuaauaaaaagaaaguuucuucacauucuag

SEQ ID NO: 31 - RNA, 1368 nt, Artificial Sequence
  Synthetic construct
ucaacacaacauauacaaaacaaacgaaucucaagcaaucaagcauucuacuucuauugcagcaauuuaaaucauuucuuuuaaagcaaaagcaauuuucugaaaauuuucaccauuuacgaacgauagccaccaugcuguuuaaccugaggauccuauugaacaaugcugcuuuucguaauggccauaacuuuaugguucggaacuuuagaugcgggcagccacugcagaacaagguccaguugaaaggccgcgaucuguugacauugaagaacuuuaccggcgaagagauuaaguauaugcuguggcugucugcugaccucaaguuucgaaucaagcagaagggcgaauaucucccccugcugcaaggaaagucucucggcaugaucuuugagaagcggaguacccgaacacggcugagcaccgaaacgggcuucgcacugcuggggggccaucccuguuuucugacaacgcaggacauccacuuggggguuaacgaaucauugacugauaccgcccgcguacugucauccauggccgacgcugugcuggcuaggguguacaagcagucagaucuggauacacuggccaaggaagcuagcauaccaaucaucaauggacugagugaccuuuaucacccgauucaaauacuagccgauuaucugacccugcaagagcauuacuccucgcugaaaggccucacgcuguccuggaucggcgacggcaacaacauucugcauaguauuaugaugucugcugccaaauucggcaugcaucugcaagcugcuacgccgaaggguuaugaacccgacgcgucaguuacgaagcucgcugagcaguaugcaaaggagaauggcacaaagcuguugcuuaccaacgauccccuggaagcugcucauggcggcaaugugcugauuacugacaccuggauuucaaugggccaggaggaggagaagaagaagagguuacaggcuuuucaagguuaccaagucacgaugaaaaccgcuaaggucgcagccagcgacuggacauuccugcacugucugccaagaaagccggaagaaguggacgacgagguguucuauuccccgcggucuuugguguuuccggaggccgaaaacaggaaauggaccauuauggccgugaugguaucguugcugacggacuacagcccucaguugcaaaagcccaaguucuagcucgagcuagugacugacuaggaucugguuaccacuaaaccagccucaagaacacccgaauggagucucuaagcuacauaauaccaacuuacacuuacaaaauguugucccccaaaauguagccauucguaucugcuccuaauaaaaagaaaguuucuucacauucuag

SEQ ID NO: 32 - RNA, 1368 nt, Artificial Sequence
  Synthetic construct
ucaacacaacauauacaaaacaaacgaaucucaagcaaucaagcauucuacuucuauugcagcaauuuaaaucauuucuuuuaaagcaaaagcaauuuucugaaaauuuucaccauuuacgaacgauagccaccaugcucuuuaaccuccgcauccuccucaacaacgccgccuuccggaaugggcauaacuucaugguccggaacuucagaugcggccagccccugcaaaacaagguccaguugaagggacgggaccuccuuacgcugaagaacuuuaccggagaagagauuaaguacaugcugugguuguccgcugaccucaaguuccgcauuaagcagaagggagaauaucugccgcugcugcaaggaaagagccugggcaugaucuucgaaaagcgcuccacuagaacccggcugucgacugagacuggauucgccuugcucgguggacacccgugcuuccugacgacccaggacauccaccugggagugaacgagucacuuacggauaccgcgagggugcuguccucaauggccgacgcagugcucgcgcgcguguacaagcagucagaucuggauacccuggccaaggaagccagcauucccaucaucaacggacugagcgaccuuuaccacccaauccagauccucgccgacuacuuaacccugcaagagcacuacagcucccugaagggacugacucuguccuggaucggggauggaaacaacauccugcacuccaucaugaugucugccgcuaaguuugggaugcaucugcaagccgcaaccccuaagggauacgagcccgacgccucggugaccaaacuugcggaacaguacgccaaggaaaacgguaccaagcugcugcugaccaacgacccucuggaagcggcccacggaggaaaugugcugauuaccgacaccuggauuucgaugggccaggaggaggagaagaagaagagacugcaggcguuccagggauaucaggucaccaugaaaaccgccaaggucgccgccagcgacuggaccuuccugcacugucucccucggaaaccggaagaaguggaugacgagguguucuacuccccgcgcucgcugguguucccggaggcugaaaacaggaaguggacaaucauggccgugauggugucccuguugaccgacuacuccccacaacugcagaagcccaaguucuagcucgagcuagugacugacuaggaucugguuaccacuaaaccagccucaagaacacccgaauggagucucuaagcuacauaauaccaacuuacacuuacaaaauguugucccccaaaauguagccauucguaucugcuccuaauaaaaagaaaguuucuucacauucuag

SEQ ID NO: 33 - RNA, 1368 nt, Artificial Sequence
  Synthetic construct
ucaacacaacauauacaaaacaaacgaaucucaagcaaucaagcauucuacuucuauugcagcaauuuaaaucauuucuuuuaaagcaaaagcaauuuucugaaaauuuucaccauuuacgaacgauagccaccaugcuuuucaaucugcgcauccuccugaacaacgccgccuuccgcaauggacacaacuuuaugguccgcaacuuccgcugugggcagccgcugcagaacaagguccagcucaaggggagagaucuccugacccugaagaacuucacuggagaggagaucaaguacaugcuguggcuguccgccgaccugaaauuucggauuaagcagaagggcgaauaccucccacugcugcaaggaaagucuuugggcaugaucuucgaaaagagaagcacccggacccgguugagcaccgaaacuggguucgcgcuccucgguggacacccgugcuuccugaccacccaagauauucaucugggugucaacgaaagccugaccgacaccgccagggugcugucauccauggcugacgcagugcucgcccggguguacaagcagucagaccuggacacccucgccaaggaagcuucgaucccuaucaucaacggacuuuccgaccuguaccaccccauccaaauucuggccgacuaccugacucugcaagaacacuauagcucgcugaaaggacuuacucuguccuggaucggggacggcaacaacauucuccauuccaucaugauguccgcugccaaguucggaaugcaccuucaagcagcgacucccaagggauacgaaccugaugccuccgugacuaagcuggcagagcaguacgccaaggagaacgguacaaagcugcugcucacgaacgacccccuggaggcggcccacggcggaaacgugcugauuaccgauaccuggaucucaaugggccaggaagaggagaagaagaagcggcuccaggcguuucaaggcuaccaggucaccaugaaaaccgcgaaggucgccgccuccgacuggacuuucuugcacugccugccgcggaagcccgaggaaguggaugacgaaguguucuacucgccgagaucguugguguucccugaggccgaaaacaggaaguggaccaucauggccgugauggugucccugcugacugauuacagcccacagcugcagaagccuaaguucuagcucgagcuagugacugacuaggaucugguuaccacuaaaccagccucaagaacacccgaauggagucucuaagcuacauaauaccaacuuacacuuacaaaauguugucccccaaaauguagccauucguaucugcuccuaauaaaaagaaaguuucuucacauucuag

SEQ ID NO: 34 - RNA, 1368 nt, Artificial Sequence
  Synthetic construct
ucaacacaacauauacaaaacaaacgaaucucaagcaaucaagcauucuacuucuauugcagcaauuuaaaucauuucuuuuaaagcaaaagcaauuuucugaaaauuuucaccauuuacgaacgauagccaccaugcuuuucaaucuccgcauccuccuuaacaacgccgcguuuagaaacggccacaacuucaugguccggaacuucagauguggccagccgcuucaaaacaagguccagcugaagggccgggaucuucugacccugaagaacuuuacuggcgaagagaucaaguacaugcucuggcucuccgcggacuugaaguuccgcauuaagcagaagggggaauaccuuccgcugcuucaaggaaagagccucggcaugaucuuugagaagcgcucaaccaggacccgccuuucuacugaaacuggguucgcgcugcucgguggccaccccugcuuccugacgacccaggacauccaccucggagugaacgaaucccucaccgauaccgcccggguguuaucgagcauggcagaugccgugcuggccaggguguacaaacaguccgaucuggacacucuggccaaggaggcgucaauuccuauuaucaacggccuuagugaccucuaccauccgauucagauccuggccgauuaccucacccugcaagaacacuacagcucccugaagggucugacauuguccuggaucggcgacggcaacaacauucuccauuccaucaugauguccgccgcaaaauucggcaugcaucuucaagccgccacgccgaaggguuacgagcccgacgcuuccgugacuaagcucgccgagcaguacgcuaaggagaacggaaccaagcuucugcugacuaacgacccacuagaagcagcccacgggggcaacgugcuuauuacugacaccuggaucuccaugggccaggaagaagagaaaaagaagcggcugcaggcguuccagggauaucaggucaccaugaaaaccgccaaggucgcugccuccgacuggaccuuccugcacugccugccucgcaagccugaagaaguggacgacgagguguucuacucgccacggagccucguguuccccgaggccgagaauagaaaguggaccaucauggccgugauggugucacugcucaccgacuacagcccgcagcuucagaagcccaaguucuagcucgagcuagugacugacuaggaucugguuaccacuaaaccagccucaagaacacccgaauggagucucuaagcuacauaauaccaacuuacacuuacaaaauguugucccccaaaauguagccauucguaucugcuccuaauaaaaagaaaguuucuucacauucuag

SEQ ID NO: 35 - RNA, 1368 nt, Artificial Sequence
  Synthetic construct
ucaacacaacauauacaaaacaaacgaaucucaagcaaucaagcauucuacuucuauugcagcaauuuaaaucauuucuuuuaaagcaaaagcaauuuucugaaaauuuucaccauuuacgaacgauagccaccaugcuuuucaaccugagaauccuccugaacaacgccgccuuccgcaauggucauaacuucaugguccgcaacuuucgcugcggacagccucuccaaaacaagguccagcucaaggggcgcgaccuccucacacugaagaacuucacuggagaagaaaucaaguacaugcuguggcugagcgccgaucugaaguuccggaucaagcagaagggagaguaccuuccucugcugcaagggaaguccuugggaaugauuuucgagaagcgguccacccggaccaggcugagcacugaaacuggcuucgcccugcugggaggccacccuuguuuccugaccacucaggacauccaccugggcgugaacgagucccugaccgauacugccagagugcuguccuccauggccgacgccgugcucgcccggguguacaagcagucagaccucgauacgcuggccaaggaagccuccauucccauuaucaauggucugucggaccucuaccauccaauccaaauccucgccgacuaccugacucugcaagaacacuacagcucacucaagggccucacccucuccuggaucggcgacggaaacaacauccuucacucgauuaugaugucggccgcgaaguucgggaugcaccuccaagcugccacuccaaaaggcuacgagccggaugccucagugacuaaguuggcggaacaguaugcgaaggagaacgguaccaagcuccugcugacuaacgacccgcuggaggccgcccacgggggaaacgugcucaucaccgauacuuggauuuccaugggacaggaggaagagaagaagaagcgguugcaggcauuucagggcuaccaggucaccaugaaaacugccaaagucgccgccagcgacuggaccuuccugcacugccugccccgcaagccugaagaaguggacgacgagguguucuacucuccccggucccucguguucccugaggccgaaaacaggaaguggaccaucauggcugugauggugucccuccugaccgacuacagcccucagcuccaaaaacccaaguuuuagcucgagcuagugacugacuaggaucugguuaccacuaaaccagccucaagaacacccgaauggagucucuaagcuacauaauaccaacuuacacuuacaaaauguugucccccaaaauguagccauucguaucugcuccuaauaaaaagaaaguuucuucacauucuag

SEQ ID NO: 36 - RNA, 1368 nt, Artificial Sequence
  Synthetic construct
ucaacacaacauauacaaaacaaacgaaucucaagcaaucaagcauucuacuucuauugcagcaauuuaaaucauuucuuuuaaagcaaaagcaauuuucugaaaauuuucaccauuuacgaacgauagccaccaugcuuuucaaccugagaauccucuugaacaaugcugcuuuucggaauggccacaacuuuaugguucggaacuuccguugcggccagccuuuacaaaacaagguccagcugaagggccgggauuugcucacacugaagaacuuuacuggggaggagauuaaguauaugcuguggcuguccgcugaccugaaguuuaggaucaagcagaagggcgaauaucugccgcugcugcaagggaaaagucugggcaugauuuuugaaaagcgcucuacccggaccagacugucuacggaaacaggcuuugcccugcugggcggccaccccuguuuucugacaacgcaggacauccaucugggcgugaacgaaucacugaccgauacugcucggguacucaguucuauggcugacgcagugcuggcuaggguguacaagcagagcgacuuggacacacuggcuaaggaggccagcauccccauuaucaauggccugucugauuuguaccaucccauucaaauccuggcugauuaucugacacuacaagagcauuacucaagucugaaggguuugacucucuccuggaucggcgacggcaacaacauuuuacauuccauuaugaugagugcugcuaaguuuggcaugcauuugcaagcugcuaccccaaagggcuaugaaccugacgcuagcguaaccaaguuggccgaacaguaugcuaaagagaauggcaccaagcugcuccugacgaaugacccccuggaagcugcucauggcggaaacguacuuauaacugauacauggauuagcaugggccaggaagaggagaagaagaagagacugcaggccuuccaaggcuaucaggucaccaugaaaacugccaagguugcagcuagcgacuggaccuuccugcacuguuugccgaggaaacccgaggagguggacgaugaagucuuuuauucuccccgcuccuugguguuucccgaggcugaaaaucgaaaguggacgauaauggcagugauggugucccuacugaccgacuauucuccacaacugcagaagccuaaauucuagcucgagcuagugacugacuaggaucugguuaccacuaaaccagccucaagaacacccgaauggagucucuaagcuacauaauaccaacuuacacuuacaaaauguugucccccaaaauguagccauucguaucugcuccuaauaaaaagaaaguuucuucacauucuag

SEQ ID NO: 37 - RNA, 1368 nt, Artificial Sequence
  Synthetic construct
ucaacacaacauauacaaaacaaacgaaucucaagcaaucaagcauucuacuucuauugcagcaauuuaaaucauuucuuuuaaagcaaaagcaauuuucugaaaauuuucaccauuuacgaacgauagccaccaugcuuuucaaucugaggauccugcugaacaacgcugcuuuucgcaacggucauaacuuuaugguucgcaauuuucguuguggccagccgcugcagaacaagguucagcugaagggcagagaucugcugacucugaagaacuucacuggggaagaaaucaaguauauguuauggcuguccgcggaucugaaauuucgaaucaagcagaagggcgaauaucuuccccugcugcaagggaaauccuugggcaugauuuuugagaagaggagcacuaggacuagauugucaacagaaacaggcuuugcuuuguugggcggacaucccugcuuucugacgacacaggauauccaccucggcguaaacgagucccucaccgacacugcuaggguacugagcagcauggccgacgcugugcuagcccggguuuacaagcagucagaccuggacacccuugccaaggaagcuucuauuccaauuaucaacggccugagugaccuguaucacccuauucaaauacucgccgacuauuugacgcuucaagaacauuacagcagccucaagggcuuaaccuugaguuggauaggcgacggcaacaauauccugcauuccauuaugaugucugccgcuaaguuuggcaugcaucuacaagccgcaacacccaagggcuaugaacccgacgcuagcgugaccaagcuggccgagcaguaugcuaaggaaaauggcacaaagcuccuucuuaccaacgauccccuggaggcugcucacggcggcaacgugcugauuaccgauacauggauuagcaugggccaggaggaggagaaaaagaagcggcuccaggcuuuucaaggcuaucaggucaccaugaaaacugcaaaggucgcugccuccgacuggacuuuccugcauugucuaccccgcaagccugaggaaguggacgaugagguguucuacuccccacggagucugguguucccggaagcagagaaucggaaguggaccaucauggcugucauggugucgcucuugacugacuauucuccccaacugcaaaaacccaaguuuuagcucgagcuagugacugacuaggaucugguuaccacuaaaccagccucaagaacacccgaauggagucucuaagcuacauaauaccaacuuacacuuacaaaauguugucccccaaaauguagccauucguaucugcuccuaauaaaaagaaaguuucuucacauucuag

SEQ ID NO: 38 - RNA, 1368 nt, Artificial Sequence
  Synthetic construct
ucaacacaacauauacaaaacaaacgaaucucaagcaaucaagcauucuacuucuauugcagcaauuuaaaucauuucuuuuaaagcaaaagcaauuuucugaaaauuuucaccauuuacgaacgauagccaccauguuauucaaccuucguauccugcuaaacaaugcugcuuuucgcaauggccauaacuuuaugguucgcaacuuuagaugcggccagccgcugcagaacaagguucagcugaagggccgggacuugcugacgcugaaaaacuuuaccggggaagagauuaaguauaugcuguggcuaagcgcugaucugaaguuuaggaucaagcagaagggcgaauaucugccacugcugcaagggaagagucuuggcaugauuuuugaaaagcggucuaccagaacccggcugucgaccgagacagguuuugcucugcuggggggccaucccuguuuucugacaacucaggacauucaccugggcgugaaugagucccugaccgauacugcuaggguguugaguagcauggccgacgcuguacucgcucgaguguauaagcagucugaucuggacacucuggcuaaggaagcuuccauuccuauuaucaacggcuugagcgaccuguaccaccccauucaaauccucgcugauuacuugacuuugcaagaacauuacagcagcuugaagggcuuaacacugagcuggauaggcgacggaaacaacaucuugcauuccauaaugauguccgccgcuaaguucgggaugcaccuccaagcagccacacccaagggcuaugaaccggaugcuuccgugacaaaacuggcugagcaguaugcuaaggagaauggcacgaaacugcugcucaccaacgacccauuggaagcugcacaugguggcaacguacugaucacugacacuuggaucucaaugggccaggaggaagagaagaagaaaaggcugcaggcauuucagggauaccaagucacuaugaaaacugccaaggucgcugccuccgacuggacauuccugcauugucugccacggaagccugaggaagucgaugacgaaguguucuauagcccacgaagcuugguguuucccgaggcugagaauaggaaguggaccauuauggcuguuauggugucccugcucaccgacuauuccccucaacugcaaaaacccaaguuuuagcucgagcuagugacugacuaggaucugguuaccacuaaaccagccucaagaacacccgaauggagucucuaagcuacauaauaccaacuuacacuuacaaaauguugucccccaaaauguagccauucguaucugcuccuaauaaaaagaaaguuucuucacauucuag

SEQ ID NO: 39 - RNA, 1365 nt, Artificial Sequence
  Synthetic construct
ucaacacaacauauacaaaacaaacgaaucucaagcaaucaagcauucuacuucuauugcagcaauuuaaaucauuucuuuuaaagcaaaagcaauuuucugaaaauuuucaccauuuacgaacgauagccaugcuuuuuaaucuccgcauccuccuuaacaacgccgcguuuagaaacggccacaacuucaugguccggaacuucagauguggccagccgcuucaaaacaagguccagcugaagggccgggaucuucugacccugaagaacuuuacuggcgaagagaucaaguacaugcucuggcucuccgcggacuugaaguuccgcauuaagcagaagggggaauaccuuccgcugcuucaaggaaagagccucggcaugaucuuugagaagcgcucaaccaggacccgccuuucuacugaaacuggguucgcgcugcucgguggccaccccugcuuccugacgacccaggacauccaccucggagugaacgaaucccucaccgauaccgcccggguguuaucgagcauggcagaugccgugcuggccaggguguacaaacaguccgaucuggacacucuggccaaggaggcgucaauucccaucaucaacggccugagcgaccuguaccacccaauccaaauccuggcugacuaccugacccugcaagagcacuacagcagccugaagggucugacccugucauggauuggcgauggaaacaauauucugcacuccaucaugauguccgccgcgaaguucggaaugcaucugcaagccgccacgccaaaaggauacgaaccggaugcguccgugacgaaguuggcggaacaguacgcgaaggagaacggaaccaagcuucugcugacuaacgacccccucgaggcugcgcaugggggcaacgugcugauuaccgacaccuggaucuccauggggcaggaggaagagaagaagaagagacugcaggcauuccagggguaccaggucaccaugaaaaccgcaaaaguggcagcuucggacuggacuuuccugcauugccugccgaggaagccggaggaagucgacgacgaaguguucuacucgccucggucccugguguuccccgaggccgaaaaccggaaguggaccaucauggccgugaugguguccuugcugacugacuauagcccgcagcugcagaagccuaaguucuagcucgagcuagugacugacuaggaucugguuaccacuaaaccagccucaagaacacccgaauggagucucuaagcuacauaauaccaacuuacacuuacaaaauguugucccccaaaauguagccauucguaucugcuccuaauaaaaagaaaguuucuucacauucuag

SEQ ID NO: 40 - RNA, 1365 nt, Artificial Sequence
  Synthetic construct
ucaacacaacauauacaaaacaaacgaaucucaagcaaucaagcauucuacuucuauugcagcaauuuaaaucauuucuuuuaaagcaaaagcaauuuucugaaaauuuucaccauuuacgaacgauagccaugcuuuucaaccugagaauccucuugaacaaugcugcuuuucggaauggccacaacuuuaugguucggaacuuccguugcggccagccuuuacaaaacaagguccagcugaagggccgggauuugcucacacugaagaacuuuacuggagaagagaucaaguacaugcuguggcugucggccgaccugaaguucaggaucaagcagaagggagaauaccuuccgcugcuucaaggaaagagccucggcaugaucuuugagaagcgcucaaccaggacccgccuuucuacugaaacuggguucgcgcugcucgguggccaccccugcuuccugacgacccaggacauccaccucggagugaacgaaucccucaccgauaccgcccggguguuaucgagcauggcagaugccgugcuggccaggguguacaaacaguccgaucucgauaccuuggcaaaggaggcuuccauucccaucaucaacggccugagcgaccuguaccacccaauccaaauccuggcugacuaccugacccugcaagagcacuacagcagccugaagggucugacccugucauggauuggcgauggaaacaauauucugcacuccaucaugauguccgccgcgaaguucggaaugcaucugcaagccgccacuccaaaaggauacgaaccggaugcguccgugaccaaguuggcggaacaguacgcgaaggagaacggaaccaagcuucugcugacuaacgacccccucgaggcugcgcaugggggcaacgugcugauuaccgacaccuggaucuccauggggcaggaggaagagaagaagaagagacugcaggcauuccagggguaccaggucaccaugaaaaccgcaaaaguggcagcuucggacuggacuuuccugcauugccugccgaggaagccggaggaagucgacgacgaaguguucuacucgccucggucccugguguuccccgaggccgaaaaccggaaguggaccaucauggccgugaugguguccuugcugacugacuauagcccgcagcugcagaagccuaaguucuagcucgagcuagugacugacuaggaucugguuaccacuaaaccagccucaagaacacccgaauggagucucuaagcuacauaauaccaacuuacacuuacaaaauguugucccccaaaauguagccauucguaucugcuccuaauaaaaagaaaguuucuucacauucuag

SEQ ID NO: 41 - RNA, 1365 nt, Artificial Sequence
  Synthetic construct
ucaacacaacauauacaaaacaaacgaaucucaagcaaucaagcauucuacuucuauugcagcaauuuaaaucauuucuuuuaaagcaaaagcaauuuucugaaaauuuucaccauuuacgaacgauagccaugcuuuucaaccugagaauccucuugaacaaugcugcuuuucggaauggccacaacuuuaugguucggaacuuccguugcggccagccuuuacaaaacaagguccagcugaagggccgggauuugcucacacuaaagaacuuuacuggagaagagaucaaguacaugcuauggcugucggccgaccugaaguuccguaucaagcagaagggagaauaccuuccgcugcuucaaggaaagagccucggcaugaucuuugagaagcgcucaaccaggacccgccuuucuacugaaacuggguucgcgcugcucgguggccaccccugcuuccugacgacccaggacauccaccucggagugaacgaaucccucaccgauaccgcccggguguuaucgagcauggcagaugccgugcuggccaggguguacaaacaguccgaucucgauaccuuggcaaaggaggcuuccauucccaucaucaacggccugagcgaccuguaccacccaauccaaauccuggcugacuaccugacccugcaagagcacuacagcagccugaagggucugacccugucauggauuggcgauggaaacaauauucugcacuccaucaugauguccgccgcgaaguucggaaugcaucugcaagccgccacuccaaaaggauacgaaccggaugcauccgugaccaaguuggcggaacaguacgcgaaggagaacggaaccaagcuccugcugacuaacgacccgcucgaggcugcgcauggggguaacgugcugauuacggacaccuggaucuccauggggcaggaggaagagaagaagaagagacugcaggcauuccagggguaccaggucaccaugaaaaccgcaaaaguggcagcuucggacuggacuuuccugcauugccugccgaggaagccggaggaagucgacgacgaaguguucuacucgccucggucccugguguuccccgaggccgaaaaccggaaguggaccaucauggccgugaugguguccuugcugacugacuauagcccgcagcugcagaagccuaaguucuagcucgagcuagugacugacuaggaucugguuaccacuaaaccagccucaagaacacccgaauggagucucuaagcuacauaauaccaacuuacacuuacaaaauguugucccccaaaauguagccauucguaucugcuccuaauaaaaagaaaguuucuucacauucuag

SEQ ID NO: 42 - RNA, 1365 nt, Artificial Sequence
  Synthetic construct
ucaacacaacauauacaaaacaaacgaaucucaagcaaucaagcauucuacuucuauugcagcaauuuaaaucauuucuuuuaaagcaaaagcaauuuucugaaaauuuucaccauuuacgaacgauagccaugcuuuucaaccugagaauccucuugaacaaugcugcuuuucggaauggccacaacuuuaugguucggaacuuccguugcggccagccuuuacaaaacaagguccagcugaagggccgggauuugcucacacuaaagaacuuuacuggagaagagaucaaguacaugcuauggcugucggccgaccugaaguuccguaucaagcagaagggagaauaccuuccgcugcuucaaggaaagagccucggcaugaucuuugagaagcgcucaaccaggacccgccuuucuacugaaacuggguucgcgcugcucgguggccaccccugcuuccugacgacccaggacauccaccucggagugaacgaaucccucaccgauaccgcccggguguuaucgagcauggcagaugccgugcuggccaggguguacaaacaguccgaucucgauaccuuggcaaaggaggcuuccauucccaucaucaacggccugagcgaccuguaccacccaauccaaauccuggcugacuaccugacccugcaagagcacuacagcagccugaagggucugacccugucauggauuggcgauggaaacaauauucugcacuccaucaugauguccgccgcgaaguucggaaugcaucugcaagccgccacuccaaaaggauacgaaccggaugcguccgugaccaaguuggcggaacaguacgcgaaggagaacggaaccaagcuucugcugacuaacgacccccucgaggcugcgcaugggggcaacgugcugauuaccgacaccuggaucuccauggggcaggaggaagagaagaagaagagacugcaggcauuccagggguaccaggucaccaugaaaaccgcaaaaguggcagcuucggacuggacuuuccugcauugccugccgaggaagccggaggaagucgacgacgaaguguucuacucgccucggucccugguguuccccgaggccgaaaaccggaaguggaccaucauggccgugaugguguccuugcugacugacuauagcccgcagcugcagaagccuaaguucuagcucgagcuagugacugacuaggaucugguuaccacuaaaccagccucaagaacacccgaauggagucucuaagcuacauaauaccaacuuacacuuacaaaauguugucccccaaaauguagccauucguaucugcuccuaauaaaaagaaaguuucuucacauucuag

SEQ ID NO: 43 - RNA, 1371 nt, Artificial Sequence
  Synthetic construct
ucaacacaacauauacaaaacaaacgaaucucaagcaaucaagcauucuacuucuauugcagcaauuuaaaucauuucuuuuaaagcaaaagcaauuuucugaaaauuuucaccauuuacgaacgauagccaccaugcuguucaaccugcgaauccugcugaacaacgccgcuuuucggaacgggcacaacuuuauggugaggaacuuucgcugcggacagccccuccagaauaagguccagcugaagggcagggaccugcugacccugaaaaauuucacaggggaggaaaucaaguauaugcuguggcugucagcugaucugaaguuccggaucaagcagaagggcgaauaucugccucugcuccagggcaaaagccuggggaugaucuucgaaaagcgcaguacucggaccagacugucaaccgagacuggauucgcucugcugggaggacacccuuguuuucugaccacucaggacauucaccugggagugaacgagucccugaccgacacugcucgcguccugagcucuauggccgacgcugugcuggcucgagucuacaaacaguccgaccuggauacccuggccaaggaagcuucuaucccaauuauuaacggccugucagaccuguaucaccccauccagauucuggccgauuaccugacccuccaggagcacuauucuagucugaaagggcugacacugaguuggauuggggacggaaacaauauccugcacucuauuaugaugucagccgccaaguuuggaaugcaccuccaggcugcaaccccaaaaggcuacgaacccgaugccucagugacaaagcuggcugaacaguacgccaaagagaacggcacuaagcugcugcugaccaacgacccucuggaggccgcucacggaggcaacgugcugaucaccgauaccuggauuaguaugggacaggaggaagagaagaagaagcggcuccaggccuuccagggcuaccaggugacaaugaaaaccgcuaaggucgcagccagcgauuggaccuuucugcacugccugcccagaaagcccgaagagguggacgacgaggucuucuacucucccagaagccugguguuucccgaagcugagaauaggaaguggacaauuauggcagugauggucagccugcugacugauuauucaccucagcuccagaaaccaaaguucugauaacucgagcuagugacugacuaggaucugguuaccacuaaaccagccucaagaacacccgaauggagucucuaagcuacauaauaccaacuuacacuuacaaaauguugucccccaaaauguagccauucguaucugcuccuaauaaaaagaaaguuucuucacauucuag

SEQ ID NO: 44 - RNA, 1371 nt, Artificial Sequence
  Synthetic construct
ucaacacaacauauacaaaacaaacgaaucucaagcaaucaagcauucuacuucuauugcagcaauuuaaaucauuucuuuuaaagcaaaagcaauuuucugaaaauuuucaccauuuacgaacgauagccaccaugcuguucaaccugcgcauccugcugaacaacgccgccuuccgcaacggccacaacuucauggugcgcaacuuccgcugcggccagccccugcagaacaaggugcagcugaagggccgcgaccugcugacccugaagaacuucaccggcgaggagaucaaguacaugcuguggcugagcgccgaccugaaguuccgcaucaagcagaagggcgaguaccugccccugcugcagggcaagagccugggcaugaucuucgagaagcgcagcacccgcacccgccugagcaccgagacaggccuggcccugcugggcggccaccccugcuuccugaccacccaggacauccaccugggcgugaacgagagccugaccgacaccgcccgcgugcugagcagcauggccgacgccgugcuggcccgcguguacaagcagagcgaccuggacacccuggccaaggaggccagcauccccaucaucaacggccugagcgaccuguaccaccccauccagauccuggccgacuaccugacccugcaggagcacuacagcagccugaagggccugacccugagcuggaucggcgacggcaacaacauccugcacagcaucaugaugagcgccgccaaguucggcaugcaccugcaggccgccacccccaagggcuacgagcccgacgccagcgugaccaagcuggccgagcaguacgccaaggagaacggcaccaagcugcugcugaccaacgacccccuggaggccgcccacggcggcaacgugcugaucaccgacaccuggaucagcaugggccaggaggaggagaagaagaagcgccugcaggccuuccagggcuaccaggugaccaugaagaccgccaagguggccgccagcgacuggaccuuccugcacugccugccccgcaagcccgaggagguggacgacgagguguucuacagcccccgcagccugguguuccccgaggccgagaaccgcaaguggaccaucauggccgugauggugagccugcugaccgacuacagcccccagcugcagaagcccaaguucugauaacucgagcuagugacugacuaggaucugguuaccacuaaaccagccucaagaacacccgaauggagucucuaagcuacauaauaccaacuuacacuuacaaaauguugucccccaaaauguagccauucguaucugcuccuaauaaaaagaaaguuucuucacauucuag

SEQ ID NO: 45 - RNA, 1371 nt, Artificial Sequence
  Synthetic construct
ucaacacaacauauacaaaacaaacgaaucucaagcaaucaagcauucuacuucuauugcagcaauuuaaaucauuucuuuuaaagcaaaagcaauuuucugaaaauuuucaccauuuacgaacgauagccaccaugcuguucaaccugcgaauccugcugaacaacgccgcuuuucggaacgggcacaacuuuauggugaggaacuuucgcugcggacagccccuccagaauaagguccagcugaagggcagggaccugcugacccugaaaaauuucacaggggaggaaaucaaguauaugcuguggcugucagcugaucugaaguuccggaucaagcagaagggcgaauaucugccucugcuccagggcaaaagccuggggaugaucuucgaaaagcgcaguacucggaccagacugucaaccgagacuggauucgcucugcugggaggacacccuuguuuucugaccacucaggacauucaccugggagugaacgagucccugaccgacacugcucgcguccugagcucuauggccgacgcugugcuagcucgagucuacaaacaguccgaccuggauacccuggccaaggaagcuucuaucccaauuauuaacggccugucagaccuguaucaccccauccagauucuggccgauuaccugacccuccaggagcacuauucuagucugaaagggcugacacugaguuggauuggggacggaaacaauauccugcacucuauuaugaugucagccgccaaguuuggaaugcaccuccaggcugcaaccccaaaaggcuacgaacccgaugccucagugacaaagcuggcugaacaguacgccaaagagaacggcacuaagcugcugcugaccaacgacccucuggaggccgcucacggaggcaacgugcugaucaccgauaccuggauuaguaugggacaggaggaagagaagaagaagcggcuccaggccuuccagggcuaccaggugacaaugaaaaccgcuaaggucgcagccagcgauuggaccuuucugcacugccugcccagaaagcccgaagagguggacgacgaggucuucuacucucccagaagccugguguuucccgaagcugagaauaggaaguggacaauuauggcagugauggucagccugcugacugauuauucaccucagcuccagaaaccaaaguucugauaacucgagcuagugacugacuaggaucugguuaccacuaaaccagccucaagaacacccgaauggagucucuaagcuacauaauaccaacuuacacuuacaaaauguugucccccaaaauguagccauucguaucugcuccuaauaaaaagaaaguuucuucacauucuag

SEQ ID NO: 46 - RNA, 1371 nt, Artificial Sequence
  Synthetic construct
ucaacacaacauauacaaaacaaacgaaucucaagcaaucaagcauucuacuucuauugcagcaauuuaaaucauuucuuuuaaagcaaaagcaauuuucugaaaauuuucaccauuuacgaacgauagccaccaugcuguucaaccugcgaauccugcugaacaaugccgcuuuucggaacgggcacaauuucauggugaggaacuuucgcugcggacagccccuccagaacaagguccagcugaagggcagggaccugcugacccugaaaaauuucacaggggaggaaaucaaguacaugcuguggcugucagccgaucugaaguuccggaucaagcagaagggcgaauaucugccucugcuccagggcaaaagccuggggaugaucuucgaaaagcgcaguacucggaccagacugucaacagagacuggauucgcacugcugggaggacacccauguuuucugaccacacaggacauucaucugggagugaacgagucccugaccgacacagcacgcguccugagcuccauggcugaugcagugcuggcucgagucuacaaacagucugaccuggauacccuggccaaggaagcuucuaucccaaucauuaauggccugagugaccuguaucaccccauccagauucuggccgauuaccugacccuccaggagcauuauucuagucugaaagggcugacacugagcuggauuggggacggaaacaauauccugcacuccauuaugaugagcgccgccaaguuuggaaugcaccuccaggcugcaaccccaaaaggcuacgaacccgaugccuccgugacaaagcuggcagaacaguaugccaaagagaacggcacuaagcugcugcugaccaaugacccucuggaggccgcucacggaggcaacgugcugaucacugauaccuggauuaguaugggacaggaggaagagaagaagaagcggcuccaggccuuccagggcuaccaggugacaaugaaaacugcuaaggucgcagccagcgacuggaccuuucugcauugccugcccagaaagccugaagagguggacgaugaggucuucuacucacccagaagccugguguuuccugaagcugagaauaggaaguggacaaucauggcagugauggucagccugcugacugauuauuccccucagcuccagaaaccaaaguucugauaacucgagcuagugacugacuaggaucugguuaccacuaaaccagccucaagaacacccgaauggagucucuaagcuacauaauaccaacuuacacuuacaaaauguugucccccaaaauguagccauucguaucugcuccuaauaaaaagaaaguuucuucacauucuag

SEQ ID NO: 47 - RNA, 1368 nt, Artificial Sequence
  Synthetic construct
ucaacacaacauauacaaaacaaacgaaucucaagcaaucaagcauucuacuucuauugcagcaauuuaaaucauuucuuuuaaagcaaaagcaauuuucugaaaauuuucaccauuuacgaacgauagccaccaugcuuuucaaccuucgcauucuccucaacaacgccgcguuuagaaacggacacaacuucaugguccgcaacuuccgcugcggacagccgcugcagaacaagguccagcucaagggucgggaucuccugacgcugaagaacuuuaccggcgaagagauuaaguacaugcuguggcuguccgccgaccuuaaguuccggaucaagcagaagggcgaauaccuuccccugcugcaaggaaagucccugggcaugaucuucgagaagcgcaguaccagaaccagacucuccacugaaaccggguucgcgcugcuuggcggccacccguguuuccucacuacgcaagacauccaucuuggcgugaacgagucccuuaccgacaccgccagggugcugucaagcauggccgacgccguccuugcgcgcguguacaagcagucagaccuugauacucuggccaaggaagccuccaucccuauuaucaacggccuauccgaccuuuaccacccgauccagauccucgcugacuaccugacccugcaagaacacuacagcagccucaagggacugacucuguccuggaucggcgacgggaacaacauccugcacucaaucaugaugagcgcagccaaguucggcaugcaucuccaagccgcuacacccaaggguuaugaaccggacgccucugugaccaaguuggcagaacaguacgccaaggagaacgguacuaagcuccuuuuaaccaacgacccccucgaagcagcccauggcgggaaugugcucauuaccgauaccuggauuucgaugggccaggaggaggagaagaagaagcggcugcaggcguuccagggcuaccaggucaccaugaaaacugccaaaguggccgccucggauuggaccuuucuccacugccugccucggaagccugaggagguggacgacgaaguguucuacuccccacggucccucguguuccccgaggccgaaaauaggaaguggaccaucauggccgugauggugucccucuugaccgauuacagcccgcagcuucagaagccuaaauucuagcucgagcuagugacugacuaggaucugguuaccacuaaaccagccucaagaacacccgaauggagucucuaagcuacauaauaccaacuuacacuuacaaaauguugucccccaaaauguagccauucguaucugcuccuaauaaaaagaaaguuucuucacauucuag

SEQ ID NO: 48 - RNA, 1368 nt, Artificial Sequence
  Synthetic construct
ucaacacaacauauacaaaacaaacgaaucucaagcaaucaagcauucuacuucuauugcagcaauuuaaaucauuucuuuuaaagcaaaagcaauuuucugaaaauuuucaccauuuacgaacgauagccaccaugcuuuucaaucuucgcauccuguugaacaacgccgccuuccgcaauggucacaacuucaugguccggaacuucagauguggacagccucuccaaaacaagguccagcugaagggaagggaccucuuaacccucaaaaacuuuacuggagaggagaucaaguacaugcuguggcuuagcgccgaccuuaaguuccggaucaagcagaagggagaguaccucccgcugcugcaaggaaagagucuuggaaugaucuucgagaagcgguccaccagaacucgccucuccacugaaaccggauucgcacuccuggguggacacccgugcuuucugaccacccaagacauccaccucggagugaacgagagccucacggacaccgcgagagugcugucauccauggccgacgccgugcuugcacgggucuacaagcaguccgaucuggacacucuugccaaggaagccuccauuccuaucauuaacggucugucggaucuguaccacccgauucagauccuugcggacuaccucacacuucaagaacacuauucaagccuaaagggucugacccuguccuggaucggagauggaaacaacauucuccauuccaucaugaugagcgcugccaaguucggaaugcaucuccaagcagcgacuccuaaggguuacgagccggacgccucagugacuaagcuggccgagcaguacgccaaggagaacgguaccaaacuguugcuuacuaacgacccgcuugaagcggcccauggaggaaacgugcugauuaccgacaccuggauuucgaugggacaggaagaggagaagaagaagcggcuccaggcguuccagggauaccaggucaccaugaaaacggccaaaguggccgcuagcgauuggaccuuucugcacugccucccgcgcaagccugaagaaguggacgacgaaguguucuacuccccucgcucucuuguguucccggaagccgaaaacaggaaguggaccaucauggccgugauggugucccuccugaccgauuacagcccgcagcugcagaagccuaaguucuagcucgagcuagugacugacuaggaucugguuaccacuaaaccagccucaagaacacccgaauggagucucuaagcuacauaauaccaacuuacacuuacaaaauguugucccccaaaauguagccauucguaucugcuccuaauaaaaagaaaguuucuucacauucuag

SEQ ID NO: 49 - RNA, 1368 nt, Artificial Sequence
  Synthetic construct
ucaacacaacauauacaaaacaaacgaaucucaagcaaucaagcauucuacuucuauugcagcaauuuaaaucauuucuuuuaaagcaaaagcaauuuucugaaaauuuucaccauuuacgaacgauagccaccaugcuuuucaaucuccgcauccuccucaacaacgccgcguuuagaaacggccacaacuucaugguccggaacuucagauguggccagccgcuucagaacaagguccagcucaagggccgggaucuucugacccugaagaacuuuacuggcgaagaaaucaaguacaugcucuggcucuccgccgacuugaaguuccgcauuaagcagaagggggaauaccuuccgcugcugcaaggaaagucgcucggcaugaucuuugagaagcgcucaacccgcaccaggcuguccacugaaaccggguucgcgcugcuugguggccaccccugcuuccugaccacccaagacauucaccucggagugaacgaaucgcucacugauacugcccgggugcugucgucgauggccgaugcagugcuggccaggguguacaaacaguccgaucuggacacucuggccaaggaggcguccaucccuauuaucaacggccuuuccgaccucuaccacccgauucagauccuugccgauuaccucacccugcaagaacacuacucgucacugaagggucugaccuuguccuggaucggcgacggcaacaacauccuccauuccauuaugauguccgccgccaaauucggcaugcaucuucaagccgcaaccccuaaggguuacgagccggacgcuuccgugaccaagcucgccgagcaguacgcuaaggagaacggaaccaagcuucugcugacuaacgacccccuagaggcagcccacgggggcaacgugcuuauuacugacaccuggaucuccaugggacaggaagaagagaagaagaagcgguuacaggcguuccagggcuaucaggucaccaugaaaaccgccaaggucgcugccucggacuggaccuuccugcauugccugccucgcaagcccgaagaaguggacgacgagguguucuacucgccacggucccuuguguucccugaggccgagaauagaaaguggaccauuauggccgugauggugucccuucucaccgacuacucgccgcaacugcagaaacccaaguucuagcucgagcuagugacugacuaggaucugguuaccacuaaaccagccucaagaacacccgaauggagucucuaagcuacauaauaccaacuuacacuuacaaaauguugucccccaaaauguagccauucguaucugcuccuaauaaaaagaaaguuucuucacauucuag

SEQ ID NO: 50 - RNA, 1368 nt, Artificial Sequence
  Synthetic construct
ucaacacaacauauacaaaacaaacgaaucucaagcaaucaagcauucuacuucuauugcagcaauuuaaaucauuucuuuuaaagcaaaagcaauuuucugaaaauuuucaccauuuacgaacgauagccaccaugcuuuucaaucuucgcauccuccucaacaacgccgccuuccggaacggucacaacuucaugguccggaacuuccgcugcggccagccgcuccaaaacaaagugcagcuuaagggccgcgaucuccugacccugaagaacuucaccggagaggaaaucaaguacaugcuguggcucucggcggaccugaaguuuaggauuaagcagaagggggaguaucugccgcugcuccaagggaagucccuuggcaugaucuucgaaaagagguccacccggacucggcucagcaccgaaacagguuuugcacuucuggggggccacccgugcuuccugacgacccaggacauccaucugggugucaacgagaguuugaccgacacugccagagugcugucauccauggcggacgcggugcucgcgagaguguacaagcaguccgaucuugacacccuggcaaaagaggcuucaaucccgaucauuaacggacucucggaucuguaccacccuauccaaaucuuggccgacuaccugacccugcaagaacacuacagcucccugaagggccugacucuuuccuggauuggcgauggaaacaacauucuccauucuauuaugauguccgccgccaaguucggcaugcaccuucaagccgccaccccgaagggcuacgaaccugacgccuccgugacuaagcuagccgaacaguacgcuaaggagaacggcacuaagcuucuccuuaccaacgauccgcuggaggcggcccauggcggaaaugugcuuaucaccgacaccuggauuagcauggggcaggaagaagagaagaagaaacggcuccaggcauuccagggcuaccaggucaccaugaaaacugccaaggucgccgcuagcgacuggaccuuccuccacugucugccucgcaagccugaagaaguggacgacgagguguucuacuccccgcgcucccucguguuuccugaggccgagaacagaaaguggaccaucauggccgugauggugucauuacuuacggacuacagcccgcagcugcagaagccgaaguucuagcucgagcuagugacugacuaggaucugguuaccacuaaaccagccucaagaacacccgaauggagucucuaagcuacauaauaccaacuuacacuuacaaaauguugucccccaaaauguagccauucguaucugcuccuaauaaaaagaaaguuucuucacauucuag

SEQ ID NO: 51 - RNA, 1368 nt, Artificial Sequence
  Synthetic construct
ucaacacaacauauacaaaacaaacgaaucucaagcaaucaagcauucuacuucuauugcagcaauuuaaaucauuucuuuuaaagcaaaagcaauuuucugaaaauuuucaccauuuacgaacgauagccaccaugcuuuuuaacuugagaauccuucugaacaacgccgcuuuccgcaacggucauaacuucaugguccggaacuucagauguggccagccccuccaaaacaaagugcagcugaagggccgggaccuucuuacgcugaagaauuucaccggcgaagaaaucaaguacaugcucuggcuguccgccgaucuuaaguuccgcauuaagcagaagggggaauaccucccgcugcugcaagggaagucgcugggcaugauuuuugagaagcggucaacucgcacccgccuguccacugaaacuggauucgcacugcucgguggccaucccugcuuccugaccacccaagacauccaccucggcgugaacgagucccugacugacaccgcccgggucuuauccucgauggccgaugcugugcuugcgaggguguacaagcaguccgaccucgacacacucgcgaaggaggccuccauccccaucaucaacggccuguccgaccuuuaccacccaauucagauccucgccgauuaccugacccugcaagagcacuacucgucgcucaaggggcuuacccucucguggauuggcgacggcaacaacauccuucacuccaucaugaugucggcagcgaaguucggcaugcaucugcaagccgccacgccuaaggguuaugaaccggaugccucagugaccaagcucgccgaacaguacgcgaaagagaauggaaccaagcuacuucugaccaacgacccccuggaggccgcucacggcggcaacguccucauuaccgauacuuggauuucgaugggacaggaagaggaaaagaagaagagacugcaggcguuccagggauaccaggucaccaugaaaacugccaaaguggcagccuccgacuggaccuuccuucacugccugccgaggaagccugaagagguggacgacgagguguucuacuccccgcgcuccuugguguuuccugaggccgaaaaccggaaguggacuaucauggccgugauggugucccuccucaccgacuacucgccgcaacugcagaagccuaaguucuagcucgagcuagugacugacuaggaucugguuaccacuaaaccagccucaagaacacccgaauggagucucuaagcuacauaauaccaacuuacacuuacaaaauguugucccccaaaauguagccauucguaucugcuccuaauaaaaagaaaguuucuucacauucuag

SEQ ID NO: 52 - RNA, 1368 nt, Artificial Sequence
  Synthetic construct
ucaacacaacauauacaaaacaaacgaaucucaagcaaucaagcauucuacuucuauugcagcaauuuaaaucauuucuuuuaaagcaaaagcaauuuucugaaaauuuucaccauuuacgaacgauagccaccauguuauucaaccuuagaauucuccuuaacaacgccgccuuccggaaugggcauaacuuuaugguccgcaauuuccgcuguggacagccucugcaaaacaagguccagcucaagggccgggaucugcugacucucaagaacuucacuggggaagaaaucaaguacaugcucuggcugagcgccgaccucaaguuccgcaucaagcagaagggagaguaccucccgcugcuccaagggaagucccugggcaugaucuucgagaagagauccacccgcaccagacuuuccacugagacuggcuucgccuugcugggaggccacccaugcuuccugacgacccaggacauucaccuuggcgugaacgagucccugacugacaccgcaaggguguuguccucgauggccgacgccgugcuugcccggguguacaagcagagcgaucuugacacccuggcuaaggaagcuuccauucccaucaucaacggucugagcgaccuguaccacccgauucagauccuggcggacuaccuaacccugcaagagcacuauagcucccugaagggccucacacuuucauggaucggcgacggcaacaacauccugcacucuauuaugaugagcgcugccaaauucggcaugcaccuccaagccgccacgccuaaaggcuacgagcccgacgccucggugaccaagcuugcggagcaguacgcgaaggaaaacggcaccaagcugcuucucaccaacgauccucuggaagcggcccaugguggcaacgugcucauuaccgacacuuggaucuccaugggacaggaggaggaaaagaagaagcggcuccaggcguuucaggguuaccaggucaccaugaaaaccgccaaggucgcagccuccgacuggaccuuccuucauugccuuccgcgcaagcccgaagaaguggacgaugaaguguuuuacucaccucggucacucguguucccggaagcagagaacaggaaauggaccauuauggccgugauggugucccugcucaccgauuacaguccgcaacugcagaagcccaaguucuagcucgagcuagugacugacuaggaucugguuaccacuaaaccagccucaagaacacccgaauggagucucuaagcuacauaauaccaacuuacacuuacaaaauguugucccccaaaauguagccauucguaucugcuccuaauaaaaagaaaguuucuucacauucuag

SEQ ID NO: 53 - RNA, 1368 nt, Artificial Sequence
  Synthetic construct
ucaacacaacauauacaaaacaaacgaaucucaagcaaucaagcauucuacuucuauugcagcaauuuaaaucauuucuuuuaaagcaaaagcaauuuucugaaaauuuucaccauuuacgaacgauagccaccaugcuuuucaaucuccgcauccuccuuaacaacgccgcguuuagaaacggccacaacuucaugguccggaacuucagauguggccagccgcuucaaaacaagguccagcugaagggccgggaucuucugacccugaagaacuuuacuggcgaagagaucaaguacaugcucuggcucuccgcggacuugaaguuccgcauuaagcagaagggggaauaccuuccgcugcuucaaggaaagagccucggcaugaucuuugagaagcgcucaaccaggacccgccuuucuacugaaacuggguucgcgcugcucgguggccaccccugcuuccugacgacccaggacauccaccucggagugaacgaaucccucaccgauaccgcccggguguuaucgagcauggcagaugccgugcuggccaggguguacaaacaguccgaucuggacacucuggccaaggaggcgucaauuccuauuaucaacggccuuagugaccucuaccauccgauucaaauccuggccgauuaccucacccugcaagaacacuacagcucccugaagggucugacauuguccuggaucggcgacggcaacaacauucuccauuccaucaugauguccgccgcaaaauucggcaugcaucuucaagccgccacgccuaaggguuacgaacccgacgcuuccgugacuaagcucgccgagcaguacgcuaaggagaacggaaccaagcugcugcugacuaacgacccgcuagaagcagcccacgggggcaacgugcuuauuacugacaccuggaucuccaugggccaggaggaagagaaaaagaagcggcugcaggcguuccagggauaucaggucaccaugaaaaccgccaaggucgcugccuccgacuggaccuuccugcacugccugccucgcaagccugaagaaguggacgacgagguguucuacucgccacggagccucguguuccccgaggccgagaauagaaaguggaccaucauggccgugauggugucacuucucaccgacuacagcccgcagcuucagaagcccaaguucuagcucgagcuagugacugacuaggaucugguuaccacuaaaccagccucaagaacacccgaauggagucucuaagcuacauaauaccaacuuacacuuacaaaauguugucccccaaaauguagccauucguaucugcuccuaauaaaaagaaaguuucuucacauucuag

SEQ ID NO: 54 - RNA, 1368 nt, Artificial Sequence
  Synthetic construct
ucaacacaacauauacaaaacaaacgaaucucaagcaaucaagcauucuacuucuauugcagcaauuuaaaucauuucuuuuaaagcaaaagcaauuuucugaaaauuuucaccauuuacgaacgauagccaccaugcuuuucaaucuccgcauccuccuuaacaacgccgcguuuagaaacggccacaacuucaugguccggaacuucagauguggccagccgcuucaaaacaagguccagcuuaagggccgggaucuccucacccuuaaaaacuucaccggcgaagagaucaaguacaugcucuggcucuccgcggaccuuaaguuccgcauuaagcagaagggggaauaccuuccgcugcuucaaggaaagagccucggcaugaucuuugagaagcgcucaaccaggaccaggcuuucuacugaaacuggguucgcgcuucucggcggucaucccugcuuccucacgacccaagacauccaccucggagugaacgaaucccucacggauacugcccgcgugcuuucgagcauggcagacgccgugcucgcccggguguacaaacaguccgaucucgacacucucgccaaggaggcgucaauuccuauuaucaacggucuuagugaccuuuaccacccgauccagauccucgccgauuaccucacacuccaagaacacuacagcucccuuaagggucuuacccucuccuggaucggcgacggcaacaacauucuccacuccaucaugauguccgccgcaaaguucggcaugcaucuucaagccgccaccccgaagggcuacgagccugaugcuuccgugacuaagcucgccgagcaguacgcuaaggagaacggaaccaagcuucuucucacuaacgacccacucgaagcagcccaugggggcaacgugcuuaucacugacaccuggaucuccaugggccaggaagaagagaagaagaagcggcuccaggcguuccagggauaucaggucaccaugaaaaccgccaaggucgcugccuccgacuggaccuuucuccacugccucccucgcaaaccugaagaaguggacgacgagguguucuacucgccccggagccucguguuccccgaggccgagaauagaaaguggaccauuauggccgugauggugucacuccucaccgacuacagcccgcagcuucagaagcccaaguucuagcucgagcuagugacugacuaggaucugguuaccacuaaaccagccucaagaacacccgaauggagucucuaagcuacauaauaccaacuuacacuuacaaaauguugucccccaaaauguagccauucguaucugcuccuaauaaaaagaaaguuucuucacauucuag

SEQ ID NO: 55 - RNA, 1368 nt, Artificial Sequence
  Synthetic construct
ucaacacaacauauacaaaacaaacgaaucucaagcaaucaagcauucuacuucuauugcagcaauuuaaaucauuucuuuuaaagcaaaagcaauuuucugaaaauuuucaccauuuacgaacgauagccaccaugcuuuucaaucuccgcauccuccuuaacaacgccgcguuuagaaacggacauaacuucaugguccggaacuucagauguggacagccgcuucaaaacaagguccagcugaagggucgggaucuucugacccugaagaacuuuaccggagaagagaucaaguacaugcucuggcucuccgcggacuugaaguuccgcauuaagcagaagggagaauaccucccgcugcuucaaggaaagagccucggaaugauuuuugagaagcgcucaaccaggacccgccuuucuacugaaacuggauucgcgcugcuggguggacaccccugcuuccugacgacccaggacauccaccucggagugaacgaaucccucacugauaccgcccggguguuaucgagcauggcagaugccgugcuggccaggguguacaaacaguccgaucuggacacucuggccaaggaggcgucaauuccuaucaucaacggacuuagugaccucuaccauccgauucaaauccuggccgacuaccucacccugcaagaacacuacagcucccugaagggucugacauuguccuggaucggagauggaaacaacauucuccacuccaucaugauguccgccgcaaaauucggaaugcaucuucaagccgccacgccuaaggguuacgaacccgacgcuuccgugacuaagcucgccgagcaguacgcuaaggagaacgguaccaagcuucuccugaccaacgacccacuagaagcagcccacgguggaaacgugcuuauuacugacacuuggaucuccaugggacaggaggaagagaaaaagaagcggcugcaggcguuccagggauaucaggucaccaugaaaaccgccaaggucgcugccuccgacuggaccuuccugcacugccugccucgcaagccugaagaaguggacgacgagguguucuacucgccgcggagccucguguuccccgaggccgagaauagaaaguggaccaucauggccgugauggugucacugcucaccgacuacagcccgcagcuucagaagcccaaguucuagcucgagcuagugacugacuaggaucugguuaccacuaaaccagccucaagaacacccgaauggagucucuaagcuacauaauaccaacuuacacuuacaaaauguugucccccaaaauguagccauucguaucugcuccuaauaaaaagaaaguuucuucacauucuag

SEQ ID NO: 56 - RNA, 1368 nt, Artificial Sequence
  Synthetic construct
ucaacacaacauauacaaaacaaacgaaucucaagcaaucaagcauucuacuucuauugcagcaauuuaaaucauuucuuuuaaagcaaaagcaauuuucugaaaauuuucaccauuuacgaacgauagccaccaugcuuuucaaccuccgcauucuccucaacaacgcugccuuccggaauggacauaacuucaugguccggaacuucagaugcggacagccgcuucagaacaagguccagcuuaaggggagagaucuccuuacccucaaaaacuucacuggcgaagaaaucaaguacaugcucuggcuuagugcggaucucaaguuccgcaucaagcagaagggagaauaccucccgcuccuucaaggaaagagccucggcaugauuuuugagaagagguccaccagaacucgccuuucaaccgagacuggguucgcccugcuuggcggucaccccugcuuccucacuacccaagacauccaccucggcgugaacgagagccuuaccgacaccgcccgcgugcucuccucaauggccgacgcugugcucgcccggguguacaagcaguccgaccuugauacucucgccaaggaggccuccaucccaauuaucaacgggcucucugaucucuaccacccuauccaaauccucgcggacuaccucacccuccaagagcacuauagcucgcucaagggccucacccuuuccuggauuggcgacggcaacaacauucuucacucgaucaugauguccgccgccaaguucggcaugcaucuccaagccgcgacccccaagggcuacgagccugacgcauccgugaccaagcucgccgagcaguacgcgaaggaaaauggcaccaagcuucuucucaccaacgacccccuugaggccgcucauggcggcaacgugcucaucacugacacuuggaucagcaugggccaggaggaggaaaagaagaagcgccuucaggcauuccaggguuaccaggucaccaugaaaaccgccaaaguggccgccuccgacuggaccuuucuucacugucucccgcggaagccugaagaaguggaugacgaaguguuuuacuccccucggucacucguguucccggaagcagaaaacaggaaguggaccauuauggcggucauggugucccuccucaccgacuacagcccgcagcuucagaaacccaaguucuagcucgagcuagugacugacuaggaucugguuaccacuaaaccagccucaagaacacccgaauggagucucuaagcuacauaauaccaacuuacacuuacaaaauguugucccccaaaauguagccauucguaucugcuccuaauaaaaagaaaguuucuucacauucuag

SEQ ID NO: 57 - RNA, 1368 nt, Artificial Sequence
  Synthetic construct
ucaacacaacauauacaaaacaaacgaaucucaagcaaucaagcauucuacuucuauugcagcaauuuaaaucauuucuuuuaaagcaaaagcaauuuucugaaaauuuucaccauuuacgaacgauagccaccaugcuuuucaaucuccgcauccuccuuaacaacgcagcguuuagaaacggucacaacuucaugguccggaacuuccgcuguggacagccgcuucaaaacaagguccagcugaagggucgggaccuucugacccugaagaacuuuacuggagaagagaucaaguacaugcuuuggcuguccgcggacuugaaguuccgcauuaagcagaagggagaauaccuuccgcugcuccaaggaaagagccugggaaugaucuuugagaagcgcucaaccaggacccgccuuucuacugaaacuggauucgcgcugcuggguggucacccuugcuuccugacgacccaggacauucaccucggagugaacgagucccucacugauaccgccagaguguuaucgagcauggcagaugccgugcuggcuaggguguacaaacaguccgaucuggacacccuggccaaggaggcaucaauuccuauuaucaacggacuuagugaccucuaccauccgauucaaauccuggccgauuaccucacccugcaagaacacuacagcucccugaagggucugacauuguccuggaucggagauggaaacaacauucuccauuccaucaugauguccgcggccaaguucggaaugcaucuccaagccgccacgccgaaaggauacgagccggacgcuuccgugacuaagcucgccgagcaguacgcuaaggagaacggaaccaagcuucugcugacuaacgacccgcuagaagccgcccacgguggaaacgugcuuauuacugacaccuggaucuccaugggacaggaagaagagaaaaagaagcggcugcaggcguuccagggauaucaggucaccaugaaaaccgccaaggucgccgccuccgacuggaccuuccuucacugccugccucggaagccugaagaaguggacgacgagguguucuacucgccgcggagccucguguucccugaggccgagaauagaaaguggaccaucauggccgugauggugucacuccucaccgacuacagcccgcagcuucagaagccuaaguucuagcucgagcuagugacugacuaggaucugguuaccacuaaaccagccucaagaacacccgaauggagucucuaagcuacauaauaccaacuuacacuuacaaaauguugucccccaaaauguagccauucguaucugcuccuaauaaaaagaaaguuucuucacauucuag

SEQ ID NO: 58 - RNA, 1368 nt, Artificial Sequence
  Synthetic construct
ucaacacaacauauacaaaacaaacgaaucucaagcaaucaagcauucuacuucuauugcagcaauuuaaaucauuucuuuuaaagcaaaagcaauuuucugaaaauuuucaccauuuacgaacgauagccaccaugcuuuucaaucuccgcauucuccucaacaacgcagccuuuagaaacggccacaacuucaugguccggaacuucagauguggccagccgcuucagaacaagguccagcucaagggccgggaccuccucacccucaaaaacuuuaccggcgaagagaucaaguacaugcucuggcuuucggccgaccuuaaguuccgcaucaagcagaagggggaauaccuuccgcugcuucaaggaaagucccucggcaugaucuuugaaaagcgcucgaccaggacccgccuuuccacugaaaccggguucgcgcuucucgguggccaccccugcuuccucaccacccaagacauucaccucggagugaacgaaucccuuaccgauaccgcaagagugcuuucgucgauggccgaugccgugcuugcgcggguguacaagcagucagaucucgacacucucgccaaggaggcguccauuccuauuaucaacggccuuuccgaccuuuaccacccgauucagauccucgccgauuaccucacccugcaagagcacuacucgucacucaagggucuuacccucuccuggaucggcgacggaaacaacauccuccauucgaucaugauguccgccgccaaauucggcaugcaccuccaagccgcgaccccgaaggguuacgagcccgacgcuuccgugaccaagcucgccgaacaguacgcuaaggaaaacggcaccaagcuccuccucacuaacgacccucucgaagcagcccaugggggcaacgugcucauuacugacacuuggaucucgaugggccaggaagaggagaaaaagaagcggcuucaggcguuccagggauaucaggucaccaugaaaaccgccaaggucgcugccucggacuggaccuuccuucacugccuuccgcgcaagccugaagagguggacgaugagguguucuacuccccacggucccuuguguuccccgaggccgagaauaggaaguggaccaucauggccgugauggugucgcuccucacugacuacuccccgcaacuucagaagccuaaguucuagcucgagcuagugacugacuaggaucugguuaccacuaaaccagccucaagaacacccgaauggagucucuaagcuacauaauaccaacuuacacuuacaaaauguugucccccaaaauguagccauucguaucugcuccuaauaaaaagaaaguuucuucacauucuag

SEQ ID NO: 59 - RNA, 1368 nt, Artificial Sequence
  Synthetic construct
ucaacacaacauauacaaaacaaacgaaucucaagcaaucaagcauucuacuucuauugcagcaauuuaaaucauuucuuuuaaagcaaaagcaauuuucugaaaauuuucaccauuuacgaacgauagccaccaugcuguuuaaucugagaauacuucuaaacaacgccgccuuccggaauggccauaacuuuaugguucggaauuuccgcugcggccagccgcugcagaacaagguccagcugaagggaagagacuugcugacccucaagaacuucaccggagaagaaaucaaguauaugcuguggcuguccgccgaccugaaauuccgcaucaagcagaagggcgaauaucugccgcuguugcaagggaagucccuggggaugaucuucgagaagagguccaccagaacacggcuuucaaccgaaaccggguuugcacugcuggguggacaccccuguuuucugaccacucaagauauccaccugggcgugaacgagucccuuaccgacacugcuaggguguuguccagcauggccgaugccguccuggcucgcguguacaagcaguccgaccuggauacccuggcaaaggaagcguccauucccauuaucaacgggcuguccgaccuguaccauccgauucaaauccuggcggacuaccugacucugcaagagcauuacagcagcuugaaggggcuuacucucucguggaucggcgacgggaacaacauccugcacuccaucaugauguccgccgccaaguucgggaugcauuugcaagcugcgaccccgaaagguuacgagcccgaugcuagcguaacuaagcuugccgaacaguacgccaaagagaaugguacaaaacugcuucugacuaacgacccgcuggaagcagcccacggcgggaacgugcugauaaccgacaccuggauuucaauggggcaggaggaagagaagaagaagcgacugcaggcguuccaaggcuaucagguuaccaugaaaaccgccaaaguggcagccagcgauuggacuuuccugcacugucugccgcggaagcccgaggaaguugaugacgaaguauucuacucaccccggagccucguguuccccgaggccgaaaaccggaaguggacuauuauggccgugauggugucgcuguugaccgacuacagcccgcaacugcagaagccgaaguuuuagcucgagcuagugacugacuaggaucugguuaccacuaaaccagccucaagaacacccgaauggagucucuaagcuacauaauaccaacuuacacuuacaaaauguugucccccaaaauguagccauucguaucugcuccuaauaaaaagaaaguuucuucacauucuag

SEQ ID NO: 60 - RNA, 1368 nt, Artificial Sequence
  Synthetic construct
ucaacacaacauauacaaaacaaacgaaucucaagcaaucaagcauucuacuucuauugcagcaauuuaaaucauuucuuuuaaagcaaaagcaauuuucugaaaauuuucaccauuuacgaacgauagccaccaugcuuuucaaccugaggauccuuuugaacaacgccgccuuucgcaacggccacaacuuuaugguccgcaauuuccgcugcgggcagccgcugcagaacaagguccagcugaagggccgggaucugcugacccugaagaacuucaccggggaggaaaucaaguacaugcuuuggcucuccgccgaucugaaguucagaaucaagcagaagggagaguaccucccguugcugcaaggaaagucacucggaaugauuuucgaaaagagaagcacuaggacccgccucucaacugaaaccggguucgcgcugcucgggggccauccguguuuccugacuacccaagacauccaccugggagugaacgagucgcugaccgacaccgcacgcgugcugucauccauggcggacgcagugcuugcccggguguacaagcagucggaccuggacacucuugccaaggaggcaucaauccccaucauuaacggacuguccgaucucuaccacccgauucagauccuggcugacuaccuaacccugcaagagcacuacucaagccugaaggggcugacccugucguggaucggggacggcaacaacauucugcacuccaucaugaugucggcggcuaaguucgggaugcauuugcaagcggcaacuccgaaggguuaugaacccgacgccuccgugaccaagcuggccgaacaguacgccaaggaaaacggaaccaaguugcugcugacuaaugauccccuggaggcggcccacggggggaacgugcugauaaccgauaccuggaucuccauggggcaggaagaagagaagaaaaagcggcugcaggcauuccagggauaccaggucaccaugaaaaccgcaaaaguggcagccagcgacuggacuuuccuccauugccugccgcgaaagccggaggaggucgaugacgagguguucuacuccccgcggucgcugguguucccggaggcggaaaaccggaaguggaccauuauggccgugauggugucacuccugacugacuacagcccgcaacugcagaagccgaaguucuagcucgagcuagugacugacuaggaucugguuaccacuaaaccagccucaagaacacccgaauggagucucuaagcuacauaauaccaacuuacacuuacaaaauguugucccccaaaauguagccauucguaucugcuccuaauaaaaagaaaguuucuucacauucuag

SEQ ID NO: 61 - RNA, 1496 nt, Artificial Sequence
  Synthetic construct
cuuaagggggcgcugccuacggagguggcagccaucuccuucucggcaucaagcuuaccauggugccccaggcccugcucuuggucccgcugcugguguucccccucugcuucggcaaguuccccaucuacaccauccccgacaagcuggggccguggagccccaucgacauccaccaccuguccugccccaacaaccucguggucgaggacgagggcugcaccaaccugagcggguucuccuacaugcuuuucaaucuccgcauccuccuuaacaacgccgcguuuagaaacggccacaacuucaugguccggaacuucagauguggccagccgcuucaaaacaagguccagcugaagggccgggaucuucugacccugaagaacuuuacuggcgaagagaucaaguacaugcucuggcucuccgcggacuugaaguuccgcauuaagcagaagggggaauaccuuccgcugcuucaaggaaagagccucggcaugaucuuugagaagcgcucaaccaggacccgccuuucuacugaaacuggguucgcgcugcucgguggccaccccugcuuccugacgacccaggacauccaccucggagugaacgaaucccucaccgauaccgcccggguguuaucgagcauggcagaugccgugcuggccaggguguacaaacaguccgaucuggacacucuggccaaggaggcgucaauuccuauuaucaacggccuuagugaccucuaccauccgauucagauccuggccgauuaccucacccugcaagaacacuacagcucccugaagggucugacauuguccuggaucggcgacggcaacaacauucuccauuccaucaugauguccgccgcaaaauucggcaugcaucuucaagccgccacgccgaaggguuacgagcccgacgcuuccgugacuaagcucgccgagcaguacgcuaaggagaacggaaccaagcuucugcugacuaacgacccacuagaagcagcccacgggggcaacgugcuuauuacugacaccuggaucuccaugggccaggaagaagagaaaaagaagcggcugcaggcguuccagggauaucaggucaccaugaaaaccgccaaggucgcugccuccgacuggaccuuccugcacugccugccucgcaagccugaagaaguggacgacgagguguucuacucgccacggagccucguguuccccgaggccgagaauagaaaguggaccaucauggccgugauggugucacugcucaccgacuacagcccgcagcuucagaagcccaaguucuagauaagugaaugcaaggcuggccggaagcccuugccugaaagcaagauuucagccuggaagagggcaaaguggacgggaguggacaggaguggaugcgauaagaugugguuugaagcugaugggugccagcccugcauugcugagucaaucaauaaagagcuuucuuuugacccauucuagaucuag

SEQ ID NO: 62 - RNA, 1368 nt, Artificial Sequence
  Synthetic construct
aggaaacuuaagauuauuacaucaaaacaaaaagccgccaaugcuguucaaccugcgcauccugcugaacaacgccgccuuccgcaacggccacaacuucauggugcgcaacuuccgcugcggccagccccugcagaacaaggugcagcugaagggccgcgaccugcugacccugaagaacuucaccggcgaggagaucaaguacaugcuguggcugagcgccgaccugaaguuccgcaucaagcagaagggcgaguaccugccccugcugcagggcaagagccugggcaugaucuucgagaagcgcagcacccgcacccgccugagcaccgagacaggccuggcccugcugggcggccaccccugcuuccugaccacccaggacauccaccugggcgugaacgagagccugaccgacaccgcccgcgugcugagcagcauggccgacgccgugcuggcccgcguguacaagcagagcgaccuggacacccuggccaaggaggccagcauccccaucaucaacggccugagcgaccuguaccaccccauccagauccuggccgacuaccugacccugcaggagcacuacagcagccugaagggccugacccugagcuggaucggcgacggcaacaacauccugcacagcaucaugaugagcgccgccaaguucggcaugcaccugcaggccgccacccccaagggcuacgagcccgacgccagcgugaccaagcuggccgagcaguacgccaaggagaacggcaccaagcugcugcugaccaacgacccccuggaggccgcccacggcggcaacgugcugaucaccgacaccuggaucagcaugggccaggaggaggagaagaagaagcgccugcaggccuuccagggcuaccaggugaccaugaagaccgccaagguggccgccagcgacuggaccuuccugcacugccugccccgcaagcccgaggagguggacgacgagguguucuacagcccccgcagccugguguuccccgaggccgagaaccgcaaguggaccaucauggccgugauggugagccugcugaccgacuacagcccccagcugcagaagcccaaguucugaacgccgaagccugcagccaugcgaccccacgccaccccgugccuccugccuccgcgcagccugcagcgggagacccuguccccgccccagccguccuccugggguggacccuaguuuaauaaagauucaccaaguuucacgcaaaaaaaaaaaaaaaaaaaaaaaaaaaaaaaaaaaaaaaaaaaaaaaaaaaaaaaaaaaaaaaaaaaaaaaaaaaaaaaaaaaaaaaaaaaaaaaaaaaaaaaaaaaaaaaaaaaaaaaaa

SEQ ID NO: 63 - RNA, 1495 nt, Artificial Sequence
  Synthetic construct
cuuaagggggcgcugccuacggagguggcagccaucuccuucucggcaucaagcuuaccauggugccccaggcccugcucuuggucccgcugcugguguucccccucugcuucggcaaguuccccaucuacaccauccccgacaagcuggggccguggagccccaucgacauccaccaccuguccugccccaacaaccucguggucgaggacgagggcugcaccaaccugagcggguucuccuacaugcuguucaaccugcgcauccugcugaacaacgccgccuuccgcaacggccacaacuucauggugcgcaacuuccgcugcggccagccccugcagaacaaggugcagcugaagggccgcgaccugcugacccugaagaacuucaccggcgaggagaucaaguacaugcuguggcugagcgccgaccugaaguuccgcaucaagcagaagggcgaguaccugccccugcugcagggcaagagccugggcaugaucuucgagaagcgcagcacccgcacccgccugagcaccgagacaggccuggcccugcugggcggccaccccugcuuccugaccacccaggacauccaccugggcgugaacgagagccugaccgacaccgcccgcgugcugagcagcauggccgacgccgugcuggcccgcguguacaagcagagcgaccuggacacccuggccaaggaggccagcauccccaucaucaacggccugagcgaccuguaccaccccauccagauccuggccgacuaccugacccugcaggagcacuacagcagccugaagggccugacccugagcuggaucggcgacggcaacaacauccugcacagcaucaugaugagcgccgccaaguucggcaugcaccugcaggccgccacccccaagggcuacgagcccgacgccagcgugaccaagcuggccgagcaguacgccaaggagaacggcaccaagcugcugcugaccaacgacccccuggaggccgcccacggcggcaacgugcugaucaccgacaccuggaucagcaugggccaggaggaggagaagaagaagcgccugcaggccuuccagggcuaccaggugaccaugaagaccgccaagguggccgccagcgacuggaccuuccugcacugccugccccgcaagcccgaggagguggacgacgagguguucuacagcccccgcagccugguguuccccgaggccgagaaccgcaaguggaccaucauggccgugauggugagccugcugaccgacuacagcccccagcugcagaagcccaaguucugaauaagugaugcaaggcuggccggaagcccuugccugaaagcaagauuucagccuggaagagggcaaaguggacgggaguggacaggaguggaugcgauaagaugugguuugaagcugaugggugccagcccugcauugcugagucaaucaauaaagagcuuucuuuugacccauucuagaucuag

SEQ ID NO: 64 - RNA, 1368 nt, Artificial Sequence
  Synthetic construct
aggaaacuuaagauuauuacaucaaaacaaaaagccgccaaugcuuuucaaucuccgcauccuccuuaacaacgccgcguuuagaaacggccacaacuucaugguccggaacuucagauguggccagccgcuucaaaacaagguccagcugaagggccgggaucuucugacccugaagaacuuuacuggcgaagagaucaaguacaugcucuggcucuccgcggacuugaaguuccgcauuaagcagaagggggaauaccuuccgcugcuucaaggaaagagccucggcaugaucuuugagaagcgcucaaccaggacccgccuuucuacugaaacuggguucgcgcugcucgguggccaccccugcuuccugacgacccaggacauccaccucggagugaacgaaucccucaccgauaccgcccggguguuaucgagcauggcagaugccgugcuggccaggguguacaaacaguccgaucuggacacucuggccaaggaggcgucaauuccuauuaucaacggccuuagugaccucuaccauccgauucagauccuggccgauuaccucacccugcaagaacacuacagcucccugaagggucugacauuguccuggaucggcgacggcaacaacauucuccauuccaucaugauguccgccgcaaaauucggcaugcaucuucaagccgccacgccgaaggguuacgagcccgacgcuuccgugacuaagcucgccgagcaguacgcuaaggagaacggaaccaagcuucugcugacuaacgacccacuagaagcagcccacgggggcaacgugcuuauuacugacaccuggaucuccaugggccaggaagaagagaaaaagaagcggcugcaggcguuccagggauaucaggucaccaugaaaaccgccaaggucgcugccuccgacuggaccuuccugcacugccugccucgcaagccugaagaaguggacgacgagguguucuacucgccacggagccucguguuccccgaggccgagaauagaaaguggaccaucauggccgugauggugucacugcucaccgacuacagcccgcagcuucagaagcccaaguucuagacgccgaagccugcagccaugcgaccccacgccaccccgugccuccugccuccgcgcagccugcagcgggagacccuguccccgccccagccguccuccugggguggacccuaguuuaauaaagauucaccaaguuucacgcaaaaaaaaaaaaaaaaaaaaaaaaaaaaaaaaaaaaaaaaaaaaaaaaaaaaaaaaaaaaaaaaaaaaaaaaaaaaaaaaaaaaaaaaaaaaaaaaaaaaaaaaaaaaaaaaaaaaaaaaa

SEQ ID NO: 65 - RNA, 1495 nt, Artificial Sequence
  Synthetic construct
cuuaagggggcgcugccuacggagguggcagccaucuccuucucggcaucaagcuuaccauggugccccaggcccugcucuuggucccgcugcugguguucccccucugcuucggcaaguuccccaucuacaccauccccgacaagcuggggccguggagccccaucgacauccaccaccuguccugccccaacaaccucguggucgaggacgagggcugcaccaaccugagcggguucuccuacaugcuuuucaaccugagaauccucuugaacaaugcugcuuuucggaauggccacaacuuuaugguucggaacuuccguugcggccagccuuuacaaaacaagguccagcugaagggccgggauuugcucacacuaaagaacuuuacuggagaagagaucaaguacaugcuauggcugucggccgaccugaaguuccguaucaagcagaagggagaauaccuuccgcugcuucaaggaaagagccucggcaugaucuuugagaagcgcucaaccaggacccgccuuucuacugaaacuggguucgcgcugcucgguggccaccccugcuuccugacgacccaggacauccaccucggagugaacgaaucccucaccgauaccgcccggguguuaucgagcauggcagaugccgugcuggccaggguguacaaacaguccgaucucgauaccuuggcaaaggaggcuuccauucccaucaucaacggccugagcgaccuguaccacccaauccaaauccuggcugacuaccugacccugcaagagcacuacagcagccugaagggucugacccugucauggauuggcgauggaaacaauauucugcacuccaucaugauguccgccgcgaaguucggaaugcaucugcaagccgccacuccaaaaggauacgaaccggaugcauccgugaccaaguuggcggaacaguacgcgaaggagaacggaaccaagcuccugcugacuaacgacccgcucgaggcugcgcauggggguaacgugcugauuacggacaccuggaucuccauggggcaggaggaagagaagaagaagagacugcaggcauuccagggguaccaggucaccaugaaaaccgcaaaaguggcagcuucggacuggacuuuccugcauugccugccgaggaagccggaggaagucgacgacgaaguguucuacucgccucggucccugguguuccccgaggccgaaaaccggaaguggaccaucauggccgugaugguguccuugcugacugacuauagcccgcagcugcagaagccuaaguucuagauaagugaugcaaggcuggccggaagcccuugccugaaagcaagauuucagccuggaagagggcaaaguggacgggaguggacaggaguggaugcgauaagaugugguuugaagcugaugggugccagcccugcauugcugagucaaucaauaaagagcuuucuuuugacccauucuagaucuag

SEQ ID NO: 66 - RNA, 1475 nt, Artificial Sequence
  Synthetic construct
ugagugucguacagccuccaggccccccccucccgggagagccauaguggucugcggaaccggugaguacaccggaauugccgggaagacuggguccuuucuuggauaaacccacucuaugcccggccauuugggcgugcccccgcaagacugcuagccgaguaguguuggguugcgaugcuguucaaccugcgcauccugcugaacaacgccgccuuccgcaacggccacaacuucauggugcgcaacuuccgcugcggccagccccugcagaacaaggugcagcugaagggccgcgaccugcugacccugaagaacuucaccggcgaggagaucaaguacaugcuguggcugagcgccgaccugaaguuccgcaucaagcagaagggcgaguaccugccccugcugcagggcaagagccugggcaugaucuucgagaagcgcagcacccgcacccgccugagcaccgagacaggccuggcccugcugggcggccaccccugcuuccugaccacccaggacauccaccugggcgugaacgagagccugaccgacaccgcccgcgugcugagcagcauggccgacgccgugcuggcccgcguguacaagcagagcgaccuggacacccuggccaaggaggccagcauccccaucaucaacggccugagcgaccuguaccaccccauccagauccuggccgacuaccugacccugcaggagcacuacagcagccugaagggccugacccugagcuggaucggcgacggcaacaacauccugcacagcaucaugaugagcgccgccaaguucggcaugcaccugcaggccgccacccccaagggcuacgagcccgacgccagcgugaccaagcuggccgagcaguacgccaaggagaacggcaccaagcugcugcugaccaacgacccccuggaggccgcccacggcggcaacgugcugaucaccgacaccuggaucagcaugggccaggaggaggagaagaagaagcgccugcaggccuuccagggcuaccaggugaccaugaagaccgccaagguggccgccagcgacuggaccuuccugcacugccugccccgcaagcccgaggagguggacgacgagguguucuacagcccccgcagccugguguuccccgaggccgagaaccgcaaguggaccaucauggccgugauggugagccugcugaccgacuacagcccccagcugcagaagcccaaguucugaauaagugauagagcggcaaacccuagcuacacuccauagcuaguuucuuuuuuuuuuguuuuuuuuuuuuuuuuuuuuuuuuuuuuuuuuuuuuuuuccuuucuuuuccuucuuuuuuuccucuuuucuugguggcuccaucuuagcccuagucacggcuagcugugaaagguccgugagccgcaugacugcagagagugccguaacuggccucucugcagaucauguucuag

SEQ ID NO: 67 - RNA, 1335 nt, Artificial Sequence
  Synthetic construct
aggaaacuuaagauuauuacaucaaaacaaaaagccgccaaugcuuuucaaucuccgcauccuccuuaacaacgccgcguuuagaaacggccacaacuucaugguccggaacuucagauguggccagccgcuucaaaacaagguccagcugaagggccgggaucuucugacccugaagaacuuuacuggcgaagagaucaaguacaugcucuggcucuccgcggacuugaaguuccgcauuaagcagaagggggaauaccuuccgcugcuucaaggaaagagccucggcaugaucuuugagaagcgcucaaccaggacccgccuuucuacugaaacuggguucgcgcugcucgguggccaccccugcuuccugacgacccaggacauccaccucggagugaacgaaucccucaccgauaccgcccggguguuaucgagcauggcagaugccgugcuggccaggguguacaaacaguccgaucuggacacucuggccaaggaggcgucaauuccuauuaucaacggccuuagugaccucuaccauccgauucagauccuggccgauuaccucacccugcaagaacacuacagcucccugaagggucugacauuguccuggaucggcgacggcaacaacauucuccauuccaucaugauguccgccgcaaaauucggcaugcaucuucaagccgccacgccgaaggguuacgagcccgacgcuuccgugacuaagcucgccgagcaguacgcuaaggagaacggaaccaagcuucugcugacuaacgacccacuagaagcagcccacgggggcaacgugcuuauuacugacaccuggaucuccaugggccaggaagaagagaaaaagaagcggcugcaggcguuccagggauaucaggucaccaugaaaaccgccaaggucgcugccuccgacuggaccuuccugcacugccugccucgcaagccugaagaaguggacgacgagguguucuacucgccacggagccucguguuccccgaggccgagaauagaaaguggaccaucauggccgugauggugucacugcucaccgacuacagcccgcagcuucagaagcccaaguucuaggcuggagccucgguagccguuccuccugcccgcugggccucccaacgggcccuccuccccuccuugcaccggcccuuccuggucuuugaauaaagucugagugggcagcaaaaaaaaaaaaaaaaaaaaaaaaaaaaaaaaaaaaaaaaaaaaaaaaaaaaaaaaaaaaaaaaaaaaaaaaaaaaaaaaaaaaaaaaaaaaaaaaaaaaaaaaaaaaaaaaaaaaaaaaa

SEQ ID NO: 68 - RNA, 1335 nt, Artificial Sequence
  Synthetic construct
aggaaacuuaagauuauuacaucaaaacaaaaagccgccaaugcuguucaaccugcgcauccugcugaacaacgccgccuuccgcaacggccacaacuucauggugcgcaacuuccgcugcggccagccccugcagaacaaggugcagcugaagggccgcgaccugcugacccugaagaacuucaccggcgaggagaucaaguacaugcuguggcugagcgccgaccugaaguuccgcaucaagcagaagggcgaguaccugccccugcugcagggcaagagccugggcaugaucuucgagaagcgcagcacccgcacccgccugagcaccgagacaggccuggcccugcugggcggccaccccugcuuccugaccacccaggacauccaccugggcgugaacgagagccugaccgacaccgcccgcgugcugagcagcauggccgacgccgugcuggcccgcguguacaagcagagcgaccuggacacccuggccaaggaggccagcauccccaucaucaacggccugagcgaccuguaccaccccauccagauccuggccgacuaccugacccugcaggagcacuacagcagccugaagggccugacccugagcuggaucggcgacggcaacaacauccugcacagcaucaugaugagcgccgccaaguucggcaugcaccugcaggccgccacccccaagggcuacgagcccgacgccagcgugaccaagcuggccgagcaguacgccaaggagaacggcaccaagcugcugcugaccaacgacccccuggaggccgcccacggcggcaacgugcugaucaccgacaccuggaucagcaugggccaggaggaggagaagaagaagcgccugcaggccuuccagggcuaccaggugaccaugaagaccgccaagguggccgccagcgacuggaccuuccugcacugccugccccgcaagcccgaggagguggacgacgagguguucuacagcccccgcagccugguguuccccgaggccgagaaccgcaaguggaccaucauggccgugauggugagccugcugaccgacuacagcccccagcugcagaagcccaaguucugagcuggagccucgguagccguuccuccugcccgcugggccucccaacgggcccuccuccccuccuugcaccggcccuuccuggucuuugaauaaagucugagugggcagcaaaaaaaaaaaaaaaaaaaaaaaaaaaaaaaaaaaaaaaaaaaaaaaaaaaaaaaaaaaaaaaaaaaaaaaaaaaaaaaaaaaaaaaaaaaaaaaaaaaaaaaaaaaaaaaaaaaaaaaaa

SEQ ID NO: 69 - RNA, 1335 nt, Artificial Sequence
  Synthetic construct
aggaaacuuaagauuauuacaucaaaacaaaaagccgccaaugcuuuucaaccugagaauccucuugaacaaugcugcuuuucggaauggccacaacuuuaugguucggaacuuccguugcggccagccuuuacaaaacaagguccagcugaagggccgggauuugcucacacuaaagaacuuuacuggagaagagaucaaguacaugcuauggcugucggccgaccugaaguuccguaucaagcagaagggagaauaccuuccgcugcuucaaggaaagagccucggcaugaucuuugagaagcgcucaaccaggacccgccuuucuacugaaacuggguucgcgcugcucgguggccaccccugcuuccugacgacccaggacauccaccucggagugaacgaaucccucaccgauaccgcccggguguuaucgagcauggcagaugccgugcuggccaggguguacaaacaguccgaucucgauaccuuggcaaaggaggcuuccauucccaucaucaacggccugagcgaccuguaccacccaauccaaauccuggcugacuaccugacccugcaagagcacuacagcagccugaagggucugacccugucauggauuggcgauggaaacaauauucugcacuccaucaugauguccgccgcgaaguucggaaugcaucugcaagccgccacuccaaaaggauacgaaccggaugcauccgugaccaaguuggcggaacaguacgcgaaggagaacggaaccaagcuccugcugacuaacgacccgcucgaggcugcgcauggggguaacgugcugauuacggacaccuggaucuccauggggcaggaggaagagaagaagaagagacugcaggcauuccagggguaccaggucaccaugaaaaccgcaaaaguggcagcuucggacuggacuuuccugcauugccugccgaggaagccggaggaagucgacgacgaaguguucuacucgccucggucccugguguuccccgaggccgaaaaccggaaguggaccaucauggccgugaugguguccuugcugacugacuauagcccgcagcugcagaagccuaaguucuaggcuggagccucgguagccguuccuccugcccgcugggccucccaacgggcccuccuccccuccuugcaccggcccuuccuggucuuugaauaaagucugagugggcagcaaaaaaaaaaaaaaaaaaaaaaaaaaaaaaaaaaaaaaaaaaaaaaaaaaaaaaaaaaaaaaaaaaaaaaaaaaaaaaaaaaaaaaaaaaaaaaaaaaaaaaaaaaaaaaaaaaaaaaaaa

SEQ ID NO: 70 - RNA, 1346 nt, Artificial Sequence
  Synthetic construct
aggaaacuuaagaauuauugguuaaagaaguauauuagugcuaauuucccuccguuuguccuagcuuuucucuucugucaaccccacacgccuuuggcacaaugcuuuucaaucuccgcauccuccuuaacaacgccgcguuuagaaacggccacaacuucaugguccggaacuucagauguggccagccgcuucaaaacaagguccagcugaagggccgggaucuucugacccugaagaacuuuacuggcgaagagaucaaguacaugcucuggcucuccgcggacuugaaguuccgcauuaagcagaagggggaauaccuuccgcugcuucaaggaaagagccucggcaugaucuuugagaagcgcucaaccaggacccgccuuucuacugaaacuggguucgcgcugcucgguggccaccccugcuuccugacgacccaggacauccaccucggagugaacgaaucccucaccgauaccgcccggguguuaucgagcauggcagaugccgugcuggccaggguguacaaacaguccgaucuggacacucuggccaaggaggcgucaauuccuauuaucaacggccuuagugaccucuaccauccgauucagauccuggccgauuaccucacccugcaagaacacuacagcucccugaagggucugacauuguccuggaucggcgacggcaacaacauucuccauuccaucaugauguccgccgcaaaauucggcaugcaucuucaagccgccacgccgaaggguuacgagcccgacgcuuccgugacuaagcucgccgagcaguacgcuaaggagaacggaaccaagcuucugcugacuaacgacccacuagaagcagcccacgggggcaacgugcuuauuacugacaccuggaucuccaugggccaggaagaagagaaaaagaagcggcugcaggcguuccagggauaucaggucaccaugaaaaccgccaaggucgcugccuccgacuggaccuuccugcacugccugccucgcaagccugaagaaguggacgacgagguguucuacucgccacggagccucguguuccccgaggccgagaauagaaaguggaccaucauggccgugauggugucacugcucaccgacuacagcccgcagcuucagaagcccaaguucuagcucgagacacaucacaaccacaaccuucucaggcuacccugagaaaaaaagacaugaagacucaggacucaucuuuucuguugguguaaaaucaacacccuaaggaacacaaauuucuuuaaacauuugacuucuugucucugugcugcaauuaauaaaaaauggaaagaaucuaucuag

SEQ ID NO: 71 - RNA, 1346 nt, Artificial Sequence
  Synthetic construct
aggaaacuuaagaauuauugguuaaagaaguauauuagugcuaauuucccuccguuuguccuagcuuuucucuucugucaaccccacacgccuuuggcacaaugcuguucaaccugcgcauccugcugaacaacgccgccuuccgcaacggccacaacuucauggugcgcaacuuccgcugcggccagccccugcagaacaaggugcagcugaagggccgcgaccugcugacccugaagaacuucaccggcgaggagaucaaguacaugcuguggcugagcgccgaccugaaguuccgcaucaagcagaagggcgaguaccugccccugcugcagggcaagagccugggcaugaucuucgagaagcgcagcacccgcacccgccugagcaccgagacaggccuggcccugcugggcggccaccccugcuuccugaccacccaggacauccaccugggcgugaacgagagccugaccgacaccgcccgcgugcugagcagcauggccgacgccgugcuggcccgcguguacaagcagagcgaccuggacacccuggccaaggaggccagcauccccaucaucaacggccugagcgaccuguaccaccccauccagauccuggccgacuaccugacccugcaggagcacuacagcagccugaagggccugacccugagcuggaucggcgacggcaacaacauccugcacagcaucaugaugagcgccgccaaguucggcaugcaccugcaggccgccacccccaagggcuacgagcccgacgccagcgugaccaagcuggccgagcaguacgccaaggagaacggcaccaagcugcugcugaccaacgacccccuggaggccgcccacggcggcaacgugcugaucaccgacaccuggaucagcaugggccaggaggaggagaagaagaagcgccugcaggccuuccagggcuaccaggugaccaugaagaccgccaagguggccgccagcgacuggaccuuccugcacugccugccccgcaagcccgaggagguggacgacgagguguucuacagcccccgcagccugguguuccccgaggccgagaaccgcaaguggaccaucauggccgugauggugagccugcugaccgacuacagcccccagcugcagaagcccaaguucugacucgagacacaucacaaccacaaccuucucaggcuacccugagaaaaaaagacaugaagacucaggacucaucuuuucuguugguguaaaaucaacacccuaaggaacacaaauuucuuuaaacauuugacuucuugucucugugcugcaauuaauaaaaaauggaaagaaucuaucuag

SEQ ID NO: 72 - RNA, 1346 nt, Artificial Sequence
  Synthetic construct
aggaaacuuaagaauuauugguuaaagaaguauauuagugcuaauuucccuccguuuguccuagcuuuucucuucugucaaccccacacgccuuuggcacaaugcuuuucaaccugagaauccucuugaacaaugcugcuuuucggaauggccacaacuuuaugguucggaacuuccguugcggccagccuuuacaaaacaagguccagcugaagggccgggauuugcucacacuaaagaacuuuacuggagaagagaucaaguacaugcuauggcugucggccgaccugaaguuccguaucaagcagaagggagaauaccuuccgcugcuucaaggaaagagccucggcaugaucuuugagaagcgcucaaccaggacccgccuuucuacugaaacuggguucgcgcugcucgguggccaccccugcuuccugacgacccaggacauccaccucggagugaacgaaucccucaccgauaccgcccggguguuaucgagcauggcagaugccgugcuggccaggguguacaaacaguccgaucucgauaccuuggcaaaggaggcuuccauucccaucaucaacggccugagcgaccuguaccacccaauccaaauccuggcugacuaccugacccugcaagagcacuacagcagccugaagggucugacccugucauggauuggcgauggaaacaauauucugcacuccaucaugauguccgccgcgaaguucggaaugcaucugcaagccgccacuccaaaaggauacgaaccggaugcauccgugaccaaguuggcggaacaguacgcgaaggagaacggaaccaagcuccugcugacuaacgacccgcucgaggcugcgcauggggguaacgugcugauuacggacaccuggaucuccauggggcaggaggaagagaagaagaagagacugcaggcauuccagggguaccaggucaccaugaaaaccgcaaaaguggcagcuucggacuggacuuuccugcauugccugccgaggaagccggaggaagucgacgacgaaguguucuacucgccucggucccugguguuccccgaggccgaaaaccggaaguggaccaucauggccgugaugguguccuugcugacugacuauagcccgcagcugcagaagccuaaguucuagcucgagacacaucacaaccacaaccuucucaggcuacccugagaaaaaaagacaugaagacucaggacucaucuuuucuguugguguaaaaucaacacccuaaggaacacaaauuucuuuaaacauuugacuucuugucucugugcugcaauuaauaaaaaauggaaagaaucuaucuag

SEQ ID NO: 73 - RNA, 1222 nt, Artificial Sequence
  Synthetic construct
auuauuacaucaaaacaaaaagccgccaccaugcuguucaaccugcgcauccugcugaacaacgccgccuuccgcaacggccacaacuucauggugcgcaacuuccgcugcggccagccccugcagaacaaggugcagcugaagggccgcgaccugcugacccugaagaacuucaccggcgaggagaucaaguacaugcuguggcugagcgccgaccugaaguuccgcaucaagcagaagggcgaguaccugccccugcugcagggcaagagccugggcaugaucuucgagaagcgcagcacccgcacccgccugagcaccgagacaggcuucgcccugcugggcggccaccccugcuuccugaccacccaggacauccaccugggcgugaacgagagccugaccgacaccgcccgcgugcugagcagcauggccgacgccgugcuggcccgcguguacaagcagagcgaccuggacacccuggccaaggaggccagcauccccaucaucaacggccugagcgaccuguaccaccccauccagauccuggccgacuaccugacccugcaggagcacuacagcagccugaagggccugacccugagcuggaucggcgacggcaacaacauccugcacagcaucaugaugagcgccgccaaguucggcaugcaccugcaggccgccacccccaagggcuacgagcccgacgccagcgugaccaagcuggccgagcaguacgccaaggagaacggcaccaagcugcugcugaccaacgacccccuggaggccgcccacggcggcaacgugcugaucaccgacaccuggaucagcaugggccaggaggaggagaagaagaagcgccugcaggccuuccagggcuaccaggugaccaugaagaccgccaagguggccgccagcgacuggaccuuccugcacugccugccccgcaagcccgaggagguggacgacgagguguucuacagcccccgcagccugguguuccccgaggccgagaaccgcaaguggaccaucauggccgugauggugagccugcugaccgacuacagcccccagcugcagaagcccaaguucugaggucucuaguaaugagcuggagccucgguagccguuccuccugcccgcugggccucccaacgggcccuccuccccuccuugcaccggcccuuccuggucuuugaauaaagucugagugggcaucuag

SEQ ID NO: 74 - RNA, 1346 nt, Artificial Sequence
  Synthetic construct
aggaaacuuaagaauuauugguuaaagaaguauauuagugcuaauuucccuccguuuguccuagcuuuucucuucugucaaccccacacgccuuuggcacaaugcuguucaaccugcgcauccugcugaacaacgccgccuuccgcaacggccacaacuucauggugcgcaacuuccgcugcggccagccccugcagaacaaggugcagcugaagggccgcgaccugcugacccugaagaacuucaccggcgaggagaucaaguacaugcuguggcugagcgccgaccugaaguuccgcaucaagcagaagggcgaguaccugccccugcugcagggcaagagccugggcaugaucuucgagaagcgcagcacccgcacccgccugagcaccgagacaggcuucgcccugcugggcggccaccccugcuuccugaccacccaggacauccaccugggcgugaacgagagccugaccgacaccgcccgcgugcugagcagcauggccgacgccgugcuggcccgcguguacaagcagagcgaccuggacacccuggccaaggaggccagcauccccaucaucaacggccugagcgaccuguaccaccccauccagauccuggccgacuaccugacccugcaggagcacuacagcagccugaagggccugacccugagcuggaucggcgacggcaacaacauccugcacagcaucaugaugagcgccgccaaguucggcaugcaccugcaggccgccacccccaagggcuacgagcccgacgccagcgugaccaagcuggccgagcaguacgccaaggagaacggcaccaagcugcugcugaccaacgacccccuggaggccgcccacggcggcaacgugcugaucaccgacaccuggaucagcaugggccaggaggaggagaagaagaagcgccugcaggccuuccagggcuaccaggugaccaugaagaccgccaagguggccgccagcgacuggaccuuccugcacugccugccccgcaagcccgaggagguggacgacgagguguucuacagcccccgcagccugguguuccccgaggccgagaaccgcaaguggaccaucauggccgugauggugagccugcugaccgacuacagcccccagcugcagaagcccaaguucugacucgagacacaucacaaccacaaccuucucaggcuacccugagaaaaaaagacaugaagacucaggacucaucuuuucuguugguguaaaaucaacacccuaaggaacacaaauuucuuuaaacauuugacuucuugucucugugcugcaauuaauaaaaaauggaaagaaucuaucuag

SEQ ID NO: 75 - RNA, 1368 nt, Artificial Sequence
  Synthetic construct
aggaaacuuaagauuauuacaucaaaacaaaaagccgccaaugcuguucaaccugcgcauccugcugaacaacgccgccuuccgcaacggccacaacuucauggugcgcaacuuccgcugcggccagccccugcagaacaaggugcagcugaagggccgcgaccugcugacccugaagaacuucaccggcgaggagaucaaguacaugcuguggcugagcgccgaccugaaguuccgcaucaagcagaagggcgaguaccugccccugcugcagggcaagagccugggcaugaucuucgagaagcgcagcacccgcacccgccugagcaccgagacaggcuucgcccugcugggcggccaccccugcuuccugaccacccaggacauccaccugggcgugaacgagagccugaccgacaccgcccgcgugcugagcagcauggccgacgccgugcuggcccgcguguacaagcagagcgaccuggacacccuggccaaggaggccagcauccccaucaucaacggccugagcgaccuguaccaccccauccagauccuggccgacuaccugacccugcaggagcacuacagcagccugaagggccugacccugagcuggaucggcgacggcaacaacauccugcacagcaucaugaugagcgccgccaaguucggcaugcaccugcaggccgccacccccaagggcuacgagcccgacgccagcgugaccaagcuggccgagcaguacgccaaggagaacggcaccaagcugcugcugaccaacgacccccuggaggccgcccacggcggcaacgugcugaucaccgacaccuggaucagcaugggccaggaggaggagaagaagaagcgccugcaggccuuccagggcuaccaggugaccaugaagaccgccaagguggccgccagcgacuggaccuuccugcacugccugccccgcaagcccgaggagguggacgacgagguguucuacagcccccgcagccugguguuccccgaggccgagaaccgcaaguggaccaucauggccgugauggugagccugcugaccgacuacagcccccagcugcagaagcccaaguucugaacgccgaagccugcagccaugcgaccccacgccaccccgugccuccugccuccgcgcagccugcagcgggagacccuguccccgccccagccguccuccugggguggacccuaguuuaauaaagauucaccaaguuucacgcaaaaaaaaaaaaaaaaaaaaaaaaaaaaaaaaaaaaaaaaaaaaaaaaaaaaaaaaaaaaaaaaaaaaaaaaaaaaaaaaaaaaaaaaaaaaaaaaaaaaaaaaaaaaaaaaaaaaaaaaa

SEQ ID NO: 76 - RNA, 1496 nt, Artificial Sequence
  Synthetic construct
cuuaagggggcgcugccuacggagguggcagccaucuccuucucggcaucaagcuuaccauggugccccaggcccugcucuuggucccgcugcugguguucccccucugcuucggcaaguuccccaucuacaccauccccgacaagcuggggccguggagccccaucgacauccaccaccuguccugccccaacaaccucguggucgaggacgagggcugcaccaaccugagcggguucuccuacaugcuguucaaccugcgcauccugcugaacaacgccgccuuccgcaacggccacaacuucauggugcgcaacuuccgcugcggccagccccugcagaacaaggugcagcugaagggccgcgaccugcugacccugaagaacuucaccggcgaggagaucaaguacaugcuguggcugagcgccgaccugaaguuccgcaucaagcagaagggcgaguaccugccccugcugcagggcaagagccugggcaugaucuucgagaagcgcagcacccgcacccgccugagcaccgagacaggcuucgcccugcugggcggccaccccugcuuccugaccacccaggacauccaccugggcgugaacgagagccugaccgacaccgcccgcgugcugagcagcauggccgacgccgugcuggcccgcguguacaagcagagcgaccuggacacccuggccaaggaggccagcauccccaucaucaacggccugagcgaccuguaccaccccauccagauccuggccgacuaccugacccugcaggagcacuacagcagccugaagggccugacccugagcuggaucggcgacggcaacaacauccugcacagcaucaugaugagcgccgccaaguucggcaugcaccugcaggccgccacccccaagggcuacgagcccgacgccagcgugaccaagcuggccgagcaguacgccaaggagaacggcaccaagcugcugcugaccaacgacccccuggaggccgcccacggcggcaacgugcugaucaccgacaccuggaucagcaugggccaggaggaggagaagaagaagcgccugcaggccuuccagggcuaccaggugaccaugaagaccgccaagguggccgccagcgacuggaccuuccugcacugccugccccgcaagcccgaggagguggacgacgagguguucuacagcccccgcagccugguguuccccgaggccgagaaccgcaaguggaccaucauggccgugauggugagccugcugaccgacuacagcccccagcugcagaagcccaaguucugaauaagugaaugcaaggcuggccggaagcccuugccugaaagcaagauuucagccuggaagagggcaaaguggacgggaguggacaggaguggaugcgauaagaugugguuugaagcugaugggugccagcccugcauugcugagucaaucaauaaagagcuuucuuuugacccauucuagaucuag

SEQ ID NO: 77 - RNA, 1380 nt, Artificial Sequence
  Synthetic construct
ucaacacaacauauacaaaacaaacgaaucucaagcaaucaagcauucuacuucuauugcagcaauuuaaaucauuucuuuuaaagcaaaagcaauuuucugaaaauuuucaccauuuacgaacgauagccaccaugggcgucuucaaccugcggauccugcugaacaacgccgccuuccggaacggccacaacuucaugguccgcaacuucagaugcggccagccccugcagaacaaggugcagcugaagggccgggaccugcugacccugaagaacuucaccggcgaagagaucaaguacaugcuguggcugagcgccgaccugaaguuccggaucaagcagaagggcgaguaccugccccugcugcaaggcaagagccugggcaugaucuucgagaagcggagcacccggacccggcugagcaccgagacaggcuuugcccugcugggaggccaccccugcuuucugaccacccaggacauccaccugggcgugaacgagagccugaccgacaccgccagagugcugagcagcauggccgacgccgugcuggcccggguguacaagcagagcgaccuggacacccuggccaaagaggccagcauccccaucaucaacggccugagcgaccuguaccaccccauccagauccuggccgacuaccugacccugcaggaacacuacagcucccugaagggccugacccugagcuggaucggcgacggcaacaacauccugcacagcaucaugaugagcgccgccaaguucggcaugcaucugcaggccgccacccccaagggcuacgagccugaugccagcgugaccaagcuggccgagcaguacgccaaagagaacggcaccaagcugcugcugaccaacgacccccuggaagccgcccacggcggcaacgugcugaucaccgacaccuggaucagcaugggccaggaagaggaaaagaagaagcggcugcaggccuuccagggcuaccaggucacaaugaagaccgccaagguggccgccagcgacuggaccuuccugcacugccugccccggaagcccgaagagguggacgacgagguguucuacagcccccggucccugguguuccccgaggccgagaaccggaaguggaccauuauggccgugauggugucccugcugaccgacuacuccccccagcugcagaagcccaaguucuagauaagugaacucgagcuagugacugacuaggaucugguuaccacuaaaccagccucaagaacacccgaauggagucucuaagcuacauaauaccaacuuacacuuacaaaauguugucccccaaaauguagccauucguaucugcuccuaauaaaaagaaaguuucuucacauucuag

SEQ ID NO: 78 - RNA, 1380 nt, Artificial Sequence
  Synthetic construct
ucaacacaacauauacaaaacaaacgaaucucaagcaaucaagcauucuacuucuauugcagcaauuuaaaucauuucuuuuaaagcaaaagcaauuuucugaaaauuuucaccauuuacgaacgauagccaccaugggcgucuucaaccugcggauccugcugaacaacgccgccuuccggaacggccacaacuucaugguccgcaacuucagaugcggccagccccugcagaacagggugcagcugaagggccgggaccugcugacccugaagaacuucaccggcgaagagaucagguacaugcuguggcugagcgccgaccugaaguuccggaucaagcagaagggcgaguaccugccccugcugcaaggcaagagccugggcaugaucuucgagaagcggagcacccggacccggcugagcaccgagacaggcuuugcccugcugggaggccaccccugcuuucugaccacccaggacauccaccugggcgugaacgagagccugaccgacaccgccagagugcugagcagcauggccgacgccgugcuggcccggguguacaagcagagcgaccuggacacccuggccaaagaggccagcauccccaucaucaacggccugagcgaccuguaccaccccauccagauccuggccgacuaccugacccugcaggaacacuacagcucccugaagggccugacccugagcuggaucggcgacggcaacaacauccugcacagcaucaugaugagcgccgccaaguucggcaugcaucugcaggccgccacccccaagggcuacgagccugaugccagcgugaccaagcuggccgagcaguacgccaaagagaacggcaccaagcugcugcugaccaacgacccccuggaagccgcccacggcggcaacgugcugaucaccgacaccuggaucagcaugggccaggaagaggaaaagaagaagcggcugcaggccuuccagggcuaccaggucacaaugaagaccgccaagguggccgccagcgacuggaccuuccugcacugccugccccggaagcccgaagagguggacgacgagguguucuacagcccccggucccugguguuccccgaggccgagaaccggaaguggaccauuauggccgugauggugucccugcugaccgacuacuccccccagcugcagaagcccaaguucuagauaagugaacucgagcuagugacugacuaggaucugguuaccacuaaaccagccucaagaacacccgaauggagucucuaagcuacauaauaccaacuuacacuuacaaaauguugucccccaaaauguagccauucguaucugcuccuaauaaaaagaaaguuucuucacauucuag

SEQ ID NO: 79 - RNA, 1380 nt, Artificial Sequence
  Synthetic construct
ucaacacaacauauacaaaacaaacgaaucucaagcaaucaagcauucuacuucuauugcagcaauuuaaaucauuucuuuuaaagcaaaagcaauuuucugaaaauuuucaccauuuacgaacgauagccaccaugcuggucuucaaccugcggauccugcugaacaacgccgccuuccggaacggccacaacuucaugguccgcaacuucagaugcggccagccccugcagaacagggugcagcugaagggccgggaccugcugacccugaagaacuucaccggcgaagagaucagguacaugcuguggcugagcgccgaccugaaguuccggaucaagcagaagggcgaguaccugccccugcugcaaggcaagagccugggcaugaucuucgagaagcggagcacccggacccggcugagcaccgagacaggcuuugcccugcugggaggccaccccugcuuucugaccacccaggacauccaccugggcgugaacgagagccugaccgacaccgccagagugcugagcagcauggccgacgccgugcuggcccggguguacaagcagagcgaccuggacacccuggccaaagaggccagcauccccaucaucaacggccugagcgaccuguaccaccccauccagauccuggccgacuaccugacccugcaggaacacuacagcucccugaagggccugacccugagcuggaucggcgacggcaacaacauccugcacagcaucaugaugagcgccgccaaguucggcaugcaucugcaggccgccacccccaagggcuacgagccugaugccagcgugaccaagcuggccgagcaguacgccaaagagaacggcaccaagcugcugcugaccaacgacccccuggaagccgcccacggcggcaacgugcugaucaccgacaccuggaucagcaugggccaggaagaggaaaagaagaagcggcugcaggccuuccagggcuaccaggucacaaugaagaccgccaagguggccgccagcgacuggaccuuccugcacugccugccccggaagcccgaagagguggacgacgagguguucuacagcccccggucccugguguuccccgaggccgagaaccggaaguggaccauuauggccgugauggugucccugcugaccgacuacuccccccagcugcagaagcccaaguucuagauaagugaacucgagcuagugacugacuaggaucugguuaccacuaaaccagccucaagaacacccgaauggagucucuaagcuacauaauaccaacuuacacuuacaaaauguugucccccaaaauguagccauucguaucugcuccuaauaaaaagaaaguuucuucacauucuag

SEQ ID NO: 80 - RNA, 1377 nt, Artificial Sequence
  Synthetic construct
ucaacacaacauauacaaaacaaacgaaucucaagcaaucaagcauucuacuucuauugcagcaauuuaaaucauuucuuuuaaagcaaaagcaauuuucugaaaauuuucaccauuuacgaacgauagccaccaugcuguucaaccugaggauccugcugaacaacgcagcuuucaggaacggccacaacuucauggugaggaacuuccggugcggccagccccugcagaacaaggugcagcugaagggcagggaccugcugacccugaagaacuucaccggagaggagaucaaguacaugcuguggcugagcgcagaccugaaguucaggaucaagcagaagggagaguaccugccccugcugcaggggaagucccugggcaugaucuucgagaagaggaguaccaggaccaggcugagcaccgaaaccggcuucgcccugcugggaggacaccccugcuuccugaccacccaggacauccaccugggcgugaacgagagucugaccgacaccgccagggugcugucuagcauggccgacgccgugcuggccaggguguacaagcagucagaccuggacacccuggcuaaggaggccagcauccccaucaucaacggccugagcgaccuguaccaccccauccagauccuggcugacuaccugacccugcaggagcacuacagcucucugaagggccugacccugagcuggaucggcgacgggaacaacauccugcacagcaucaugaugagcgccgccaaguucggcaugcaccugcaggccgcuacccccaaggguuacgagcccgacgccagcgugaccaagcuggcagagcaguacgccaaggagaacggcaccaagcugcugcugaccaacgacccccuggaggccgcccacggaggcaacgugcugaucaccgacaccuggaucagcaugggacaggaggaggagaagaagaagcggcugcaggcuuuccaggguuaccaggugaccaugaagaccgccaagguggcugccagcgacuggaccuuccugcacugccugcccaggaagcccgaggagguggacgacgagguguucuacucucccaggagccugguguuccccgaggccgagaacaggaaguggaccaucauggcugugauggugucccugcugaccgacuacagcccccagcugcagaagcccaaguucugaauaagugaacucgagcuagugacugacuaggaucugguuaccacuaaaccagccucaagaacacccgaauggagucucuaagcuacauaauaccaacuuacacuuacaaaauguugucccccaaaauguagccauucguaucugcuccuaauaaaaagaaaguuucuucacauucuag

SEQ ID NO: 81 - RNA, 1377 nt, Artificial Sequence
  Synthetic construct
ucaacacaacauauacaaaacaaacgaaucucaagcaaucaagcauucuacuucuauugcagcaauuuaaaucauuucuuuuaaagcaaaagcaauuuucugaaaauuuucaccauuuacgaacgauagccaccaugcuguucaaccugaggauccugcugaacaacgcagcuuucaggaacggccacaacuucauggugaggaacuuccggugcggccagccccugcagaacaaggugcagcugaagggcagggaccugcugacccugaagaacuucaccggagaggagaucaaguacaugcuguggcugagcgcagaccugaaguucaggaucaagcagaagggagaguaccugccccugcugcaggggaagucccugggcaugaucuucgagaagaggaguaccaggaccaggcugagcaccgaaaccggcuucgcccugcugggaggacaccccugcuuccugacgacccaggacauccaccucggagugaacgaaucccucaccgauaccgcccggguguuaucaagcauggcagaugccgugcuggccaggguguacaaacaguccgaucuggacacucuggcuaaggaggccagcauccccaucaucaacggccugagcgaccuguaccaccccauccagauccuggcugacuaccugacccugcaggagcacuacagcucucugaagggccugacccugagcuggaucggcgacgggaacaacauccugcacuccaucaugauguccgccgcgaaguucggaaugcaucugcaagccgccacgccaaaaggauacgaaccggaugcgcccgugacaaaguuggcggaacaguacgcuaaggagaacggaaccaagcugcugcugaccaacgacccccuggaggccgcccacggaggcaacgugcugaucaccgacaccuggaucagcaugggacaggaggaggagaagaagaagcggcugcaggcuuuccaggguuaccaggugaccaugaagaccgccaagguggcugccagcgacuggaccuuccugcacugccugcccaggaagcccgaggagguggacgacgagguguucuacucucccaggagccugguguuccccgaggccgagaacaggaaguggaccaucauggcugugauggugucccugcugaccgacuacagcccccagcugcagaagcccaaguucugaauaagugaacucgagcuagugacugacuaggaucugguuaccacuaaaccagccucaagaacacccgaauggagucucuaagcuacauaauaccaacuuacacuuacaaaauguugucccccaaaauguagccauucguaucugcuccuaauaaaaagaaaguuucuucacauucuag

SEQ ID NO: 82 - RNA, 1477 nt, Artificial Sequence
  Synthetic construct
ucaacacaacauauacaaaacaaacgaaucucaagcaaucaagcauucuacuucuauugcagcaauuuaaaucauuucuuuuaaagcaaaagcaauuuucugaaaauuuucaccauuuacgaacgauagccaccaugcuguucaaccugcgcauccugcugaacaacgccgccuuccgcaacggccacaacuucauggugcgcaacuuccgcugcggccagccccugcagaacaaggugcagcugaagggccgcgaccugcugacccugaagaacuucaccggcgaggagaucaaguacaugcuguggcugagcgccgaccugaaguuccgcaucaagcagaagggcgaguaccugccccugcugcagggcaagagccugggcaugaucuucgagaagcgcagcacccgcacccgccugagcaccgagacaggcuucgcccugcugggcggccaccccugcuuccugaccacccaggacauccaccugggcgugaacgagagccugaccgacaccgcccgcgugcugagcagcauggccgacgccgugcuggcccgcguguacaagcagagcgaccuggacacccuggccaaggaggccagcauccccaucaucaacggccugagcgaccuguaccaccccauccagauccuggccgacuaccugacccugcaggagcacuacagcagccugaagggccugacccugagcuggaucggcgacggcaacaacauccugcacagcaucaugaugagcgccgccaaguucggcaugcaccugcaggccgccacccccaagggcuacgagcccgacgccagcgugaccaagcuggccgagcaguacgccaaggagaacggcaccaagcugcugcugaccaacgacccccuggaggccgcccacggcggcaacgugcugaucaccgacaccuggaucagcaugggccaggaggaggagaagaagaagcgccugcaggccuuccagggcuaccaggugaccaugaagaccgccaagguggccgccagcgacuggaccuuccugcacugccugccccgcaagcccgaggagguggacgacgagguguucuacagcccccgcagccugguguuccccgaggccgagaaccgcaaguggaccaucauggccgugauggugagccugcugaccgacuacagcccccagcugcagaagcccaaguucugaauaagugaacucgagcuagugacugacuaggaucugguuaccacuaaaccagccucaagaacacccgaauggagucucuaagcuacauaauaccaacuuacacuuacaaaauguugucccccaaaauguagccauucguaucugcuccuaauaaaaagaaaguuucuucacauucuagaaaaaaaaaaaaaaaaaaaaaaaaaaaaaaaaaaaaaaaaaaaaaaaaaaaaaaaaaaaaaaaaaaaaaaaaaaaaaaaaaaaaaaaaaaaaaaaaaaaa

SEQ ID NO: 83 - RNA, 1371 nt, Artificial Sequence
  Synthetic construct
aggaaacuuaagucaacacaacauauacaaaacaaacgaaucucaagcaaucaagcauucuacuucuauugcagcaauuuaaaucauuucuuuuaaagcaaaagcaauuuucugaaaauuuucaccauuuacgaacgauagccaugcuguucaaccugcgcauccugcugaacaacgccgccuuccgcaacggccacaacuucauggugcgcaacuuccgcugcggccagccccugcagaacaaggugcagcugaagggccgcgaccugcugacccugaagaacuucaccggcgaggagaucaaguacaugcuguggcugagcgccgaccugaaguuccgcaucaagcagaagggcgaguaccugccccugcugcagggcaagagccugggcaugaucuucgagaagcgcagcacccgcacccgccugagcaccgagacaggcuucgcccugcugggcggccaccccugcuuccugaccacccaggacauccaccugggcgugaacgagagccugaccgacaccgcccgcgugcugagcagcauggccgacgccgugcuggcccgcguguacaagcagagcgaccuggacacccuggccaaggaggccagcauccccaucaucaacggccugagcgaccuguaccaccccauccagauccuggccgacuaccugacccugcaggagcacuacagcagccugaagggccugacccugagcuggaucggcgacggcaacaacauccugcacagcaucaugaugagcgccgccaaguucggcaugcaccugcaggccgccacccccaagggcuacgagcccgacgccagcgugaccaagcuggccgagcaguacgccaaggagaacggcaccaagcugcugcugaccaacgacccccuggaggccgcccacggcggcaacgugcugaucaccgacaccuggaucagcaugggccaggaggaggagaagaagaagcgccugcaggccuuccagggcuaccaggugaccaugaagaccgccaagguggccgccagcgacuggaccuuccugcacugccugccccgcaagcccgaggagguggacgacgagguguucuacagcccccgcagccugguguuccccgaggccgagaaccgcaaguggaccaucauggccgugauggugagccugcugaccgacuacagcccccagcugcagaagcccaaguucugacuagugacugacuaggaucugguuaccacuaaaccagccucaagaacacccgaauggagucucuaagcuacauaauaccaacuuacacuuacaaaauguugucccccaaaauguagccauucguaucugcuccuaauaaaaagaaaguuucuucacauucuag

SEQ ID NO: 84 - RNA, 1371 nt, Artificial Sequence
  Synthetic construct
ucaacacaacauauacaaaacaaacgaaucucaagcaaucaagcauucuacuucuauugcagcaauuuaaaucauuucuuuuaaagcaaaagcaauuuucugaaaauuuucaccauuuacgaacgauagccaccaugcuuuucaacuugagaauccugcugaacaacgccgccuuucgcaacggucacaauuuuauggucagaaacuucagaugcggacagccccuccaaaacaagguccagcugaagggccgcgaucuccucacccugaagaacuucacgggggaggagaucaaguacaugcuguggcucuccgcugaccugaaguucaggaucaagcagaagggagaauaucugccgcugcugcaagggaagucccuggggaugauuuucgagaagcggagcacccggacucggcucuccacugaaacugguuucgcccuucugggcggucaccccugcuuccugaccacucaagacauucaccucggagugaacgaguccuugacugacaccgcccgggugcugucgagcauggcagacgccgugcuagcccgcguguacaagcagucagaccucgauacccuggccaaggaggcuucgaucccgaucaucaacggguuguccgaccuguaccacccgauucagauucucgccgacuaccucacccugcaagagcauuacagcucccugaaggggcuuacccuguccuggauuggcgacggaaacaacauccugcacuccauuaugaugucggcggccaaguucggcaugcaccuccaagccgcgaccccuaaggguuacgaaccagacgcgucagugacuaagcuggccgaacaguacgcaaaggaaaauggcacgaagcugcuccugaccaacgauccguuggaagccgcccauggcggaaaugugcucaucaccgacaccuggaucucgaugggacaggaggaagagaagaagaagcggcugcaggcguuccagggcuaccaggucaccaugaaaacugccaagguggccgccagcgacuggaccuuccugcacugccuuccgcgcaagccugaggagguggacgaugaaguguucuacucuccacggucccugguguuccccgaggcggagaaccgcaaauggaccaucauggcugugauggucagccugcugaccgauuacagcccucaguugcaaaagccgaaguuuugauaacucgagcuagugacugacuaggaucugguuaccacuaaaccagccucaagaacacccgaauggagucucuaagcuacauaauaccaacuuacacuuacaaaauguugucccccaaaauguagccauucguaucugcuccuaauaaaaagaaaguuucuucacauucuag

SEQ ID NO: 85 - RNA, 1471 nt, Artificial Sequence
  Synthetic construct
ucaacacaacauauacaaaacaaacgaaucucaagcaaucaagcauucuacuucuauugcagcaauuuaaaucauuucuuuuaaagcaaaagcaauuuucugaaaauuuucaccauuuacgaacgauagccaccaugcuguucaaccuccgcauccuccucaacaacgccgcauucagaaacgggcacaacuucauggucagaaacuuccgcugcgggcaaccccuacaaaacaagguccagcucaaggggcgggaccuccugacccugaagaacuucaccggcgaagagaucaaguacaugcuguggcucuccgccgaccugaaguuccgcaucaagcagaagggagaguaccucccgcugcugcaagggaagucgcuggggaugaucuucgagaagcggucaaccagaacccggcugucaaccgaaaccggguucgcacugcuggggggacacccgugcuuccugaccacccaagacauccaccugggagugaacgaaucgcugaccgacaccgcccgcgugcugagcucaauggcggacgccgugcuggcccgcguguacaagcaguccgaccuggacacccuggccaaggaagcguccaucccgaucaucaacggacuguccgaccuguaccacccgauccagauccuggcagacuaccugacccugcaagaacacuacagcucccugaagggccugacccugucauggaucggggacgggaacaacauccugcacuccauaaugaugucagccgccaaguucggaaugcaccuccaagccgcaaccccgaagggcuacgaaccggacgcaucagugaccaaacuggccgagcaguacgccaaggaaaacggcaccaagcuccugcugaccaacgacccgcuggaggccgcacacggggggaacgugcugaucaccgacaccuggaucuccaugggacaggaggaggaaaagaagaagcggcugcaggcguuccagggguaccaggucaccaugaaaaccgcgaaggucgcggcaucagacuggaccuuccugcacugccugccccggaagccggaagagguggacgacgagguguucuacucgccgcgcucgcugguguuccccgaggcggagaacaggaaguggaccaucauggcggugauggucagccuccugaccgacuacucgccgcagcugcagaagccgaaguucugauaacucgagcuagugacugacuaggaucugguuaccacuaaaccagccucaagaacacccgaauggagucucuaagcuacauaauaccaacuuacacuuacaaaauguugucccccaaaauguagccauucguaucugcuccuaauaaaaagaaaguuucuucacauucuagaaaaaaaaaaaaaaaaaaaaaaaaaaaaaaaaaaaaaaaaaaaaaaaaaaaaaaaaaaaaaaaaaaaaaaaaaaaaaaaaaaaaaaaaaaaaaaaaaaaa

SEQ ID NO: 86 - RNA, 1771 nt, Artificial Sequence
  Synthetic construct
cucccuccccccccccuaacguuacuggccgaagccgcuuggaauaaggccggugugcguuugucuauauguuauuuuccaccauauugccgucuuuuggcaaugugagggcccggaaaccuggcccugucuucuugacgagcauuccuaggggucuuuccccucucgccaaaggaaugcaaggucuguugaaugucgugaaggaagcaguuccucuggaagcuucuugaagacaaacaacgucuguagcgacccuuugcaggcagcggaaccccccaccuggcgacaggugccucugcggccaaaagccacguguauaagauacaccugcaaaggcggcacaaccccagugccacguugugaguuggauaguuguggaaagagucaaauggcucuccucaagcguauucaacaaggggcugaaggaugcccagaagguaccccauuguaugggaucugaucuggggccucggugcacaugcuuuacguguguuuagucgagguuaaaaaacgucuaggccccccgaaccacggggacgugguuuuccuuugaaaaacacgaugauaauaugcuuuucaaucuccgcauccuccuuaacaacgccgcguuuagaaacggccacaacuucaugguccggaacuucagauguggccagccgcuucaaaacaagguccagcugaagggccgggaucuucugacccugaagaacuuuacuggcgaagagaucaaguacaugcucuggcucuccgcggacuugaaguuccgcauuaagcagaagggggaauaccuuccgcugcuucaaggaaagagccucggcaugaucuuugagaagcgcucaaccaggacccgccuuucuacugaaacuggguucgcgcugcucgguggccaccccugcuuccugacgacccaggacauccaccucggagugaacgaaucccucaccgauaccgcccggguguuaucgagcauggcagaugccgugcuggccaggguguacaaacaguccgaucuggacacucuggccaaggaggcgucaauuccuauuaucaacggccuuagugaccucuaccauccgauucagauccuggccgauuaccucacccugcaagaacacuacagcucccugaagggucugacauuguccuggaucggcgacggcaacaacauucuccauuccaucaugauguccgccgcaaaauucggcaugcaucuucaagccgccacgccgaaggguuacgagcccgacgcuuccgugacuaagcucgccgagcaguacgcuaaggagaacggaaccaagcuucugcugacuaacgacccacuagaagcagcccacgggggcaacgugcuuauuacugacaccuggaucuccaugggccaggaagaagagaaaaagaagcggcugcaggcguuccagggauaucaggucaccaugaaaaccgccaaggucgcugccuccgacuggaccuuccugcacugccugccucgcaagccugaagaaguggacgacgagguguucuacucgccacggagccucguguuccccgaggccgagaauagaaaguggaccaucauggccgugauggugucacugcucaccgacuacagcccgcagcuucagaagcccaaguucugaauaaguagauagugcagucacuggcacaacgcguugcccgguaagccaaucggguauacacggucgucauacugcagacaggguucuucuacuuugcaagauagucuagaguaguaaaauaaauaguauaagucuag

SEQ ID NO: 87 - RNA, 1771 nt, Artificial Sequence
  Synthetic construct
cucccuccccccccccuaacguuacuggccgaagccgcuuggaauaaggccggugugcguuugucuauauguuauuuuccaccauauugccgucuuuuggcaaugugagggcccggaaaccuggcccugucuucuugacgagcauuccuaggggucuuuccccucucgccaaaggaaugcaaggucuguugaaugucgugaaggaagcaguuccucuggaagcuucuugaagacaaacaacgucuguagcgacccuuugcaggcagcggaaccccccaccuggcgacaggugccucugcggccaaaagccacguguauaagauacaccugcaaaggcggcacaaccccagugccacguugugaguuggauaguuguggaaagagucaaauggcucuccucaagcguauucaacaaggggcugaaggaugcccagaagguaccccauuguaugggaucugaucuggggccucggugcacaugcuuuacguguguuuagucgagguuaaaaaacgucuaggccccccgaaccacggggacgugguuuuccuuugaaaaacacgaugauaauaugcuuuucaaccugagaauccucuugaacaaugcugcuuuucggaauggccacaacuuuaugguucggaacuuccguugcggccagccuuuacaaaacaagguccagcugaagggccgggauuugcucacacuaaagaacuuuacuggagaagagaucaaguacaugcuauggcugucggccgaccugaaguuccguaucaagcagaagggagaauaccuuccgcugcuucaaggaaagagccucggcaugaucuuugagaagcgcucaaccaggacccgccuuucuacugaaacuggguucgcgcugcucgguggccaccccugcuuccugacgacccaggacauccaccucggagugaacgaaucccucaccgauaccgcccggguguuaucgagcauggcagaugccgugcuggccaggguguacaaacaguccgaucucgauaccuuggcaaaggaggcuuccauucccaucaucaacggccugagcgaccuguaccacccaauccaaauccuggcugacuaccugacccugcaagagcacuacagcagccugaagggucugacccugucauggauuggcgauggaaacaauauucugcacuccaucaugauguccgccgcgaaguucggaaugcaucugcaagccgccacuccaaaaggauacgaaccggaugcauccgugaccaaguuggcggaacaguacgcgaaggagaacggaaccaagcuccugcugacuaacgacccgcucgaggcugcgcauggggguaacgugcugauuacggacaccuggaucuccauggggcaggaggaagagaagaagaagagacugcaggcauuccagggguaccaggucaccaugaaaaccgcaaaaguggcagcuucggacuggacuuuccugcauugccugccgaggaagccggaggaagucgacgacgaaguguucuacucgccucggucccugguguuccccgaggccgaaaaccggaaguggaccaucauggccgugaugguguccuugcugacugacuauagcccgcagcugcagaagccuaaguucugaauaaguagauagugcagucacuggcacaacgcguugcccgguaagccaaucggguauacacggucgucauacugcagacaggguucuucuacuuugcaagauagucuagaguaguaaaauaaauaguauaagucuag

SEQ ID NO: 88 - RNA, 1771 nt, Artificial Sequence
  Synthetic construct
cucccuccccccccccuaacguuacuggccgaagccgcuuggaauaaggccggugugcguuugucuauauguuauuuuccaccauauugccgucuuuuggcaaugugagggcccggaaaccuggcccugucuucuugacgagcauuccuaggggucuuuccccucucgccaaaggaaugcaaggucuguugaaugucgugaaggaagcaguuccucuggaagcuucuugaagacaaacaacgucuguagcgacccuuugcaggcagcggaaccccccaccuggcgacaggugccucugcggccaaaagccacguguauaagauacaccugcaaaggcggcacaaccccagugccacguugugaguuggauaguuguggaaagagucaaauggcucuccucaagcguauucaacaaggggcugaaggaugcccagaagguaccccauuguaugggaucugaucuggggccucggugcacaugcuuuacguguguuuagucgagguuaaaaaacgucuaggccccccgaaccacggggacgugguuuuccuuugaaaaacacgaugauaauaugcuguucaaccugcgcauccugcugaacaacgccgccuuccgcaacggccacaacuucauggugcgcaacuuccgcugcggccagccccugcagaacaaggugcagcugaagggccgcgaccugcugacccugaagaacuucaccggcgaggagaucaaguacaugcuguggcugagcgccgaccugaaguuccgcaucaagcagaagggcgaguaccugccccugcugcagggcaagagccugggcaugaucuucgagaagcgcagcacccgcacccgccugagcaccgagacaggccuggcccugcugggcggccaccccugcuuccugaccacccaggacauccaccugggcgugaacgagagccugaccgacaccgcccgcgugcugagcagcauggccgacgccgugcuggcccgcguguacaagcagagcgaccuggacacccuggccaaggaggccagcauccccaucaucaacggccugagcgaccuguaccaccccauccagauccuggccgacuaccugacccugcaggagcacuacagcagccugaagggccugacccugagcuggaucggcgacggcaacaacauccugcacagcaucaugaugagcgccgccaaguucggcaugcaccugcaggccgccacccccaagggcuacgagcccgacgccagcgugaccaagcuggccgagcaguacgccaaggagaacggcaccaagcugcugcugaccaacgacccccuggaggccgcccacggcggcaacgugcugaucaccgacaccuggaucagcaugggccaggaggaggagaagaagaagcgccugcaggccuuccagggcuaccaggugaccaugaagaccgccaagguggccgccagcgacuggaccuuccugcacugccugccccgcaagcccgaggagguggacgacgagguguucuacagcccccgcagccugguguuccccgaggccgagaaccgcaaguggaccaucauggccgugauggugagccugcugaccgacuacagcccccagcugcagaagcccaaguucugaauaaguagauagugcagucacuggcacaacgcguugcccgguaagccaaucggguauacacggucgucauacugcagacaggguucuucuacuuugcaagauagucuagaguaguaaaauaaauaguauaagucuag

SEQ ID NO: 89 - RNA, 1368 nt, Artificial Sequence; identical to SEQ ID NO: 34
  Synthetic construct

SEQ ID NO: 90 - RNA, 1368 nt, Artificial Sequence; identical to SEQ ID NO: 34
  Synthetic construct

SEQ ID NO: 91 - RNA, 1368 nt, Artificial Sequence; identical to SEQ ID NO: 34
  Synthetic construct

SEQ ID NO: 92 - RNA, 1368 nt, Artificial Sequence; identical to SEQ ID NO: 34
  Synthetic construct

SEQ ID NO: 93 - RNA, 1368 nt, Artificial Sequence; identical to SEQ ID NO: 34
  Synthetic construct

SEQ ID NO: 94 - RNA, 1371 nt, Artificial Sequence
  Synthetic construct
ucaacacaacauauacaaaacaaacgaaucucaagcaaucaagcauucuacuucuauugcagcaauuuaaaucauuucuuuuaaagcaaaagcaauuuucugaaaauuuucaccauuuacgaacgauagccaccaugguguucaaccuccgcauccuccucaacaacgccgcauucagaaacgggcacaacuucauggucagaaacuuccgcugcgggcaaccccuacaaaacaagguccagcucaaggggcgggaccuccugacccugaagaacuucaccggcgaagagaucaaguacaugcuguggcucuccgccgaccugaaguuccgcaucaagcagaagggagaguaccucccgcugcugcaagggaagucgcuggggaugaucuucgagaagcggucaaccagaacccggcugucaaccgaaaccggguucgcacugcuggggggacacccgugcuuccugaccacccaagacauccaccugggagugaacgaaucgcugaccgacaccgcccgcgugcugagcucaauggcggacgccgugcuggcccgcguguacaagcaguccgaccuggacacccuggccaaggaagcguccaucccgaucaucaacggacuguccgaccuguaccacccgauccagauccuggcagacuaccugacccugcaagaacacuacagcucccugaagggccugacccugucauggaucggggacgggaacaacauccugcacuccauaaugaugucagccgccaaguucggaaugcaccuccaagccgcaaccccgaagggcuacgaaccggacgcaucagugaccaaacuggccgagcaguacgccaaggaaaacggcaccaagcuccugcugaccaacgacccgcuggaggccgcacacggggggaacgugcugaucaccgacaccuggaucuccaugggacaggaggaggaaaagaagaagcggcugcaggcguuccagggguaccaggucaccaugaaaaccgcgaaggucgcggcaucagacuggaccuuccugcacugccugccccggaagccggaagagguggacgacgagguguucuacucgccgcgcucgcugguguuccccgaggcggagaacaggaaguggaccaucauggcggugauggucagccuccugaccgacuacucgccgcagcugcagaagccgaaguucugauaacucgagcuagugacugacuaggaucugguuaccacuaaaccagccucaagaacacccgaauggagucucuaagcuacauaauaccaacuuacacuuacaaaauguugucccccaaaauguagccauucguaucugcuccuaauaaaaagaaaguuucuucacauucuag

SEQ ID NO: 95 - RNA, 1371 nt, Artificial Sequence
  Synthetic construct
ucaacacaacauauacaaaacaaacgaaucucaagcaaucaagcauucuacuucuauugcagcaauuuaaaucauuucuuuuaaagcaaaagcaauuuucugaaaauuuucaccauuuacgaacgauagccaccaugguguucaaccuccgcauccuccucaacaacgccgcauucagaaacgggcacaacuucauggucagaaacuuccgcugcgggcaaccccuacaaaaccggguccagcucaaggggcgggaccuccugacccugaagaacuucaccggcgaagagaucaaguacaugcuguggcucuccgccgaccugaaguuccgcaucaagcagaagggagaguaccucccgcugcugcaagggaagucgcuggggaugaucuucgagaagcggucaaccagaacccggcugucaaccgaaaccggguucgcacugcuggggggacacccgugcuuccugaccacccaagacauccaccugggagugaacgaaucgcugaccgacaccgcccgcgugcugagcucaauggcggacgccgugcuggcccgcguguacaagcaguccgaccuggacacccuggccaaggaagcguccaucccgaucaucaacggacuguccgaccuguaccacccgauccagauccuggcagacuaccugacccugcaagaacacuacagcucccugaagggccugacccugucauggaucggggacgggaacaacauccugcacuccauaaugaugucagccgccaaguucggaaugcaccuccaagccgcaaccccgaagggcuacgaaccggacgcaucagugaccaaacuggccgagcaguacgccaaggaaaacggcaccaagcuccugcugaccaacgacccgcuggaggccgcacacggggggaacgugcugaucaccgacaccuggaucuccaugggacaggaggaggaaaagaagaagcggcugcaggcguuccagggguaccaggucaccaugaaaaccgcgaaggucgcggcaucagacuggaccuuccugcacugccugccccggaagccggaagagguggacgacgagguguucuacucgccgcgcucgcugguguuccccgaggcggagaacaggaaguggaccaucauggcggugauggucagccuccugaccgacuacucgccgcagcugcagaagccgaaguucugauaacucgagcuagugacugacuaggaucugguuaccacuaaaccagccucaagaacacccgaauggagucucuaagcuacauaauaccaacuuacacuuacaaaauguugucccccaaaauguagccauucguaucugcuccuaauaaaaagaaaguuucuucacauucuag

SEQ ID NO: 96 - RNA, 1371 nt, Artificial Sequence
  Synthetic construct
ucaacacaacauauacaaaacaaacgaaucucaagcaaucaagcauucuacuucuauugcagcaauuuaaaucauuucuuuuaaagcaaaagcaauuuucugaaaauuuucaccauuuacgaacgauagccaccaugguguucaaccuccgcauccuccucaacaacgccgcauucagaaacgggcacaacuucauggucagaaacuuccgcugcgggcaaccccuacaaaaccggguccagcucaaggggcgggaccuccugacccugaagaacuucaccggcgaagagauccgguacaugcuguggcucuccgccgaccugaaguuccgcaucaagcagaagggagaguaccucccgcugcugcaagggaagucgcuggggaugaucuucgagaagcggucaaccagaacccggcugucaaccgaaaccggguucgcacugcuggggggacacccgugcuuccugaccacccaagacauccaccugggagugaacgaaucgcugaccgacaccgcccgcgugcugagcucaauggcggacgccgugcuggcccgcguguacaagcaguccgaccuggacacccuggccaaggaagcguccaucccgaucaucaacggacuguccgaccuguaccacccgauccagauccuggcagacuaccugacccugcaagaacacuacagcucccugaagggccugacccugucauggaucggggacgggaacaacauccugcacuccauaaugaugucagccgccaaguucggaaugcaccuccaagccgcaaccccgaagggcuacgaaccggacgcaucagugaccaaacuggccgagcaguacgccaaggaaaacggcaccaagcuccugcugaccaacgacccgcuggaggccgcacacggggggaacgugcugaucaccgacaccuggaucuccaugggacaggaggaggaaaagaagaagcggcugcaggcguuccagggguaccaggucaccaugaaaaccgcgaaggucgcggcaucagacuggaccuuccugcacugccugccccggaagccggaagagguggacgacgagguguucuacucgccgcgcucgcugguguuccccgaggcggagaacaggaaguggaccaucauggcggugauggucagccuccugaccgacuacucgccgcagcugcagaagccgaaguucugauaacucgagcuagugacugacuaggaucugguuaccacuaaaccagccucaagaacacccgaauggagucucuaagcuacauaauaccaacuuacacuuacaaaauguugucccccaaaauguagccauucguaucugcuccuaauaaaaagaaaguuucuucacauucuag

SEQ ID NO: 97 - RNA, 1371 nt, Artificial Sequence
  Synthetic construct
ucaacacaacauauacaaaacaaacgaaucucaagcaaucaagcauucuacuucuauugcagcaauuuaaaucauuucuuuuaaagcaaaagcaauuuucugaaaauuuucaccauuuacgaacgauagccaccaugcuggucaaccuccgcauccuccucaacaacgccgcauucagaaacgggcacaacuucauggucagaaacuuccgcugcgggcaaccccuacaaaacaagguccagcucaaggggcgggaccuccugacccugaagaacuucaccggcgaagagaucaaguacaugcuguggcucuccgccgaccugaaguuccgcaucaagcagaagggagaguaccucccgcugcugcaagggaagucgcuggggaugaucuucgagaagcggucaaccagaacccggcugucaaccgaaaccggguucgcacugcuggggggacacccgugcuuccugaccacccaagacauccaccugggagugaacgaaucgcugaccgacaccgcccgcgugcugagcucaauggcggacgccgugcuggcccgcguguacaagcaguccgaccuggacacccuggccaaggaagcguccaucccgaucaucaacggacuguccgaccuguaccacccgauccagauccuggcagacuaccugacccugcaagaacacuacagcucccugaagggccugacccugucauggaucggggacgggaacaacauccugcacuccauaaugaugucagccgccaaguucggaaugcaccuccaagccgcaaccccgaagggcuacgaaccggacgcaucagugaccaaacuggccgagcaguacgccaaggaaaacggcaccaagcuccugcugaccaacgacccgcuggaggccgcacacggggggaacgugcugaucaccgacaccuggaucuccaugggacaggaggaggaaaagaagaagcggcugcaggcguuccagggguaccaggucaccaugaaaaccgcgaaggucgcggcaucagacuggaccuuccugcacugccugccccggaagccggaagagguggacgacgagguguucuacucgccgcgcucgcugguguuccccgaggcggagaacaggaaguggaccaucauggcggugauggucagccuccugaccgacuacucgccgcagcugcagaagccgaaguucugauaacucgagcuagugacugacuaggaucugguuaccacuaaaccagccucaagaacacccgaauggagucucuaagcuacauaauaccaacuuacacuuacaaaauguugucccccaaaauguagccauucguaucugcuccuaauaaaaagaaaguuucuucacauucuag

SEQ ID NO: 98 - RNA, 1471 nt, Artificial Sequence
  Synthetic construct
ucaacacaacauauacaaaacaaacgaaucucaagcaaucaagcauucuacuucuauugcagcaauuuaaaucauuucuuuuaaagcaaaagcaauuuucugaaaauuuucaccauuuacgaacgauagccaccaugcuggucaaccuccgcauccuccucaacaacgccgcauucagaaacgggcacaacuucauggucagaaacuuccgcugcgggcaaccccuacaaaaccggguccagcucaaggggcgggaccuccugacccugaagaacuucaccggcgaagagaucaaguacaugcuguggcucuccgccgaccugaaguuccgcaucaagcagaagggagaguaccucccgcugcugcaagggaagucgcuggggaugaucuucgagaagcggucaaccagaacccggcugucaaccgaaaccggguucgcacugcuggggggacacccgugcuuccugaccacccaagacauccaccugggagugaacgaaucgcugaccgacaccgcccgcgugcugagcucaauggcggacgccgugcuggcccgcguguacaagcaguccgaccuggacacccuggccaaggaagcguccaucccgaucaucaacggacuguccgaccuguaccacccgauccagauccuggcagacuaccugacccugcaagaacacuacagcucccugaagggccugacccugucauggaucggggacgggaacaacauccugcacuccauaaugaugucagccgccaaguucggaaugcaccuccaagccgcaaccccgaagggcuacgaaccggacgcaucagugaccaaacuggccgagcaguacgccaaggaaaacggcaccaagcuccugcugaccaacgacccgcuggaggccgcacacggggggaacgugcugaucaccgacaccuggaucuccaugggacaggaggaggaaaagaagaagcggcugcaggcguuccagggguaccaggucaccaugaaaaccgcgaaggucgcggcaucagacuggaccuuccugcacugccugccccggaagccggaagagguggacgacgagguguucuacucgccgcgcucgcugguguuccccgaggcggagaacaggaaguggaccaucauggcggugauggucagccuccugaccgacuacucgccgcagcugcagaagccgaaguucugauaacucgagcuagugacugacuaggaucugguuaccacuaaaccagccucaagaacacccgaauggagucucuaagcuacauaauaccaacuuacacuuacaaaauguugucccccaaaauguagccauucguaucugcuccuaauaaaaagaaaguuucuucacauucuagaaaaaaaaaaaaaaaaaaaaaaaaaaaaaaaaaaaaaaaaaaaaaaaaaaaaaaaaaaaaaaaaaaaaaaaaaaaaaaaaaaaaaaaaaaaaaaaaaaaa

SEQ ID NO: 99 - RNA, 1371 nt, Artificial Sequence
  Synthetic construct
ucaacacaacauauacaaaacaaacgaaucucaagcaaucaagcauucuacuucuauugcagcaauuuaaaucauuucuuuuaaagcaaaagcaauuuucugaaaauuuucaccauuuacgaacgauagccaccaugcuggucaaccuccgcauccuccucaacaacgccgcauucagaaacgggcacaacuucauggucagaaacuuccgcugcgggcaaccccuacaaaaccggguccagcucaaggggcgggaccuccugacccugaagaacuucaccggcgaagagauccgguacaugcuguggcucuccgccgaccugaaguuccgcaucaagcagaagggagaguaccucccgcugcugcaagggaagucgcuggggaugaucuucgagaagcggucaaccagaacccggcugucaaccgaaaccggguucgcacugcuggggggacacccgugcuuccugaccacccaagacauccaccugggagugaacgaaucgcugaccgacaccgcccgcgugcugagcucaauggcggacgccgugcuggcccgcguguacaagcaguccgaccuggacacccuggccaaggaagcguccaucccgaucaucaacggacuguccgaccuguaccacccgauccagauccuggcagacuaccugacccugcaagaacacuacagcucccugaagggccugacccugucauggaucggggacgggaacaacauccugcacuccauaaugaugucagccgccaaguucggaaugcaccuccaagccgcaaccccgaagggcuacgaaccggacgcaucagugaccaaacuggccgagcaguacgccaaggaaaacggcaccaagcuccugcugaccaacgacccgcuggaggccgcacacggggggaacgugcugaucaccgacaccuggaucuccaugggacaggaggaggaaaagaagaagcggcugcaggcguuccagggguaccaggucaccaugaaaaccgcgaaggucgcggcaucagacuggaccuuccugcacugccugccccggaagccggaagagguggacgacgagguguucuacucgccgcgcucgcugguguuccccgaggcggagaacaggaaguggaccaucauggcggugauggucagccuccugaccgacuacucgccgcagcugcagaagccgaaguucugauaacucgagcuagugacugacuaggaucugguuaccacuaaaccagccucaagaacacccgaauggagucucuaagcuacauaauaccaacuuacacuuacaaaauguugucccccaaaauguagccauucguaucugcuccuaauaaaaagaaaguuucuucacauucuag

SEQ ID NO: 100 - RNA, 1471 nt, Artificial Sequence
  Synthetic construct
ucaacacaacauauacaaaacaaacgaaucucaagcaaucaagcauucuacuucuauugcagcaauuuaaaucauuucuuuuaaagcaaaagcaauuuucugaaaauuuucaccauuuacgaacgauagccaccaugcuggucaaccugcgcauccugcugaacaacgccgccuuccgcaacggccacaacuucauggugcgcaacuuccgcugcggccagccccugcagaacaaggugcagcugaagggccgcgaccugcugacccugaagaacuucaccggcgaggagaucaaguacaugcuguggcugagcgccgaccugaaguuccgcaucaagcagaagggcgaguaccugccccugcugcagggcaagagccugggcaugaucuucgagaagcgcagcacccgcacccgccugagcaccgagacaggcuucgcccugcugggcggccaccccugcuuccugaccacccaggacauccaccugggcgugaacgagagccugaccgacaccgcccgcgugcugagcagcauggccgacgccgugcuggcccgcguguacaagcagagcgaccuggacacccuggccaaggaggccagcauccccaucaucaacggccugagcgaccuguaccaccccauccagauccuggccgacuaccugacccugcaggagcacuacagcagccugaagggccugacccugagcuggaucggcgacggcaacaacauccugcacagcaucaugaugagcgccgccaaguucggcaugcaccugcaggccgccacccccaagggcuacgagcccgacgccagcgugaccaagcuggccgagcaguacgccaaggagaacggcaccaagcugcugcugaccaacgacccccuggaggccgcccacggcggcaacgugcugaucaccgacaccuggaucagcaugggccaggaggaggagaagaagaagcgccugcaggccuuccagggcuaccaggugaccaugaagaccgccaagguggccgccagcgacuggaccuuccugcacugccugccccgcaagcccgaggagguggacgacgagguguucuacagcccccgcagccugguguuccccgaggccgagaaccgcaaguggaccaucauggccgugauggugagccugcugaccgacuacagcccccagcugcagaagcccaaguucugauaacucgagcuagugacugacuaggaucugguuaccacuaaaccagccucaagaacacccgaauggagucucuaagcuacauaauaccaacuuacacuuacaaaauguugucccccaaaauguagccauucguaucugcuccuaauaaaaagaaaguuucuucacauucuagaaaaaaaaaaaaaaaaaaaaaaaaaaaaaaaaaaaaaaaaaaaaaaaaaaaaaaaaaaaaaaaaaaaaaaaaaaaaaaaaaaaaaaaaaaaaaaaaaaaa

SEQ ID NO: 101 - RNA, 1371 nt, Artificial Sequence
  Synthetic construct
ucaacacaacauauacaaaacaaacgaaucucaagcaaucaagcauucuacuucuauugcagcaauuuaaaucauuucuuuuaaagcaaaagcaauuuucugaaaauuuucaccauuuacgaacgauagccaccaugcuggucaaccugcgcauccugcugaacaacgccgccuuccgcaacggccacaacuucauggugcgcaacuuccgcugcggccagccccugcagaaccgggugcagcugaagggccgcgaccugcugacccugaagaacuucaccggcgaggagaucaaguacaugcuguggcugagcgccgaccugaaguuccgcaucaagcagaagggcgaguaccugccccugcugcagggcaagagccugggcaugaucuucgagaagcgcagcacccgcacccgccugagcaccgagacaggcuucgcccugcugggcggccaccccugcuuccugaccacccaggacauccaccugggcgugaacgagagccugaccgacaccgcccgcgugcugagcagcauggccgacgccgugcuggcccgcguguacaagcagagcgaccuggacacccuggccaaggaggccagcauccccaucaucaacggccugagcgaccuguaccaccccauccagauccuggccgacuaccugacccugcaggagcacuacagcagccugaagggccugacccugagcuggaucggcgacggcaacaacauccugcacagcaucaugaugagcgccgccaaguucggcaugcaccugcaggccgccacccccaagggcuacgagcccgacgccagcgugaccaagcuggccgagcaguacgccaaggagaacggcaccaagcugcugcugaccaacgacccccuggaggccgcccacggcggcaacgugcugaucaccgacaccuggaucagcaugggccaggaggaggagaagaagaagcgccugcaggccuuccagggcuaccaggugaccaugaagaccgccaagguggccgccagcgacuggaccuuccugcacugccugccccgcaagcccgaggagguggacgacgagguguucuacagcccccgcagccugguguuccccgaggccgagaaccgcaaguggaccaucauggccgugauggugagccugcugaccgacuacagcccccagcugcagaagcccaaguucugauaacucgagcuagugacugacuaggaucugguuaccacuaaaccagccucaagaacacccgaauggagucucuaagcuacauaauaccaacuuacacuuacaaaauguugucccccaaaauguagccauucguaucugcuccuaauaaaaagaaaguuucuucacauucuag

SEQ ID NO: 102 - RNA, 1368 nt, Artificial Sequence
  Synthetic construct
ucaacacaacauauacaaaacaaacgaaucucaagcaaucaagcauucuacuucuauugcagcaauuuaaaucauuucuuuuaaagcaaaagcaauuuucugaaaauuuucaccauuuacgaacgauagccaccaugcuugucaaucuccgcauccuccuuaacaacgccgcguuuagaaacggccacaacuucaugguccggaacuucagauguggccagccgcuucaaaacaagguccagcugaagggccgggaucuucugacccugaagaacuuuacuggcgaagagaucaaguacaugcucuggcucuccgcggacuugaaguuccgcauuaagcagaagggggaauaccuuccgcugcuucaaggaaagagccucggcaugaucuuugagaagcgcucaaccaggacccgccuuucuacugaaacuggguucgcgcugcucgguggccaccccugcuuccugacgacccaggacauccaccucggagugaacgaaucccucaccgauaccgcccggguguuaucgagcauggcagaugccgugcuggccaggguguacaaacaguccgaucuggacacucuggccaaggaggcgucaauuccuauuaucaacggccuuagugaccucuaccauccgauucagauccuggccgauuaccucacccugcaagaacacuacagcucccugaagggucugacauuguccuggaucggcgacggcaacaacauucuccauuccaucaugauguccgccgcaaaauucggcaugcaucuucaagccgccacgccgaaggguuacgagcccgacgcuuccgugacuaagcucgccgagcaguacgcuaaggagaacggaaccaagcuucugcugacuaacgacccacuagaagcagcccacgggggcaacgugcuuauuacugacaccuggaucuccaugggccaggaagaagagaaaaagaagcggcugcaggcguuccagggauaucaggucaccaugaaaaccgccaaggucgcugccuccgacuggaccuuccugcacugccugccucgcaagccugaagaaguggacgacgagguguucuacucgccacggagccucguguuccccgaggccgagaauagaaaguggaccaucauggccgugauggugucacugcucaccgacuacagcccgcagcuucagaagcccaaguucuagcucgagcuagugacugacuaggaucugguuaccacuaaaccagccucaagaacacccgaauggagucucuaagcuacauaauaccaacuuacacuuacaaaauguugucccccaaaauguagccauucguaucugcuccuaauaaaaagaaaguuucuucacauucuag

SEQ ID NO: 103 - RNA, 1368 nt, Artificial Sequence
  Synthetic construct
ucaacacaacauauacaaaacaaacgaaucucaagcaaucaagcauucuacuucuauugcagcaauuuaaaucauuucuuuuaaagcaaaagcaauuuucugaaaauuuucaccauuuacgaacgauagccaccaugcuugucaaucuccgcauccuccuuaacaacgccgcguuuagaaacggccacaacuucaugguccggaacuucagauguggccagccgcuucaaaaccggguccagcugaagggccgggaucuucugacccugaagaacuuuacuggcgaagagaucaaguacaugcucuggcucuccgcggacuugaaguuccgcauuaagcagaagggggaauaccuuccgcugcuucaaggaaagagccucggcaugaucuuugagaagcgcucaaccaggacccgccuuucuacugaaacuggguucgcgcugcucgguggccaccccugcuuccugacgacccaggacauccaccucggagugaacgaaucccucaccgauaccgcccggguguuaucgagcauggcagaugccgugcuggccaggguguacaaacaguccgaucuggacacucuggccaaggaggcgucaauuccuauuaucaacggccuuagugaccucuaccauccgauucagauccuggccgauuaccucacccugcaagaacacuacagcucccugaagggucugacauuguccuggaucggcgacggcaacaacauucuccauuccaucaugauguccgccgcaaaauucggcaugcaucuucaagccgccacgccgaaggguuacgagcccgacgcuuccgugacuaagcucgccgagcaguacgcuaaggagaacggaaccaagcuucugcugacuaacgacccacuagaagcagcccacgggggcaacgugcuuauuacugacaccuggaucuccaugggccaggaagaagagaaaaagaagcggcugcaggcguuccagggauaucaggucaccaugaaaaccgccaaggucgcugccuccgacuggaccuuccugcacugccugccucgcaagccugaagaaguggacgacgagguguucuacucgccacggagccucguguuccccgaggccgagaauagaaaguggaccaucauggccgugauggugucacugcucaccgacuacagcccgcagcuucagaagcccaaguucuagcucgagcuagugacugacuaggaucugguuaccacuaaaccagccucaagaacacccgaauggagucucuaagcuacauaauaccaacuuacacuuacaaaauguugucccccaaaauguagccauucguaucugcuccuaauaaaaagaaaguuucuucacauucuag

SEQ ID NO: 104 - RNA, 1371 nt, Artificial Sequence
  Synthetic construct
ucaacacaacauauacaaaacaaacgaaucucaagcaaucaagcauucuacuucuauugcagcaauuuaaaucauuucuuuuaaagcaaaagcaauuuucugaaaauuuucaccauuuacgaacgauagccaccaugggccuugucaaucuccgcauccuccuuaacaacgccgcguuuagaaacggccacaacuucaugguccggaacuucagauguggccagccgcuucaaaacaagguccagcugaagggccgggaucuucugacccugaagaacuuuacuggcgaagagaucaaguacaugcucuggcucuccgcggacuugaaguuccgcauuaagcagaagggggaauaccuuccgcugcuucaaggaaagagccucggcaugaucuuugagaagcgcucaaccaggacccgccuuucuacugaaacuggguucgcgcugcucgguggccaccccugcuuccugacgacccaggacauccaccucggagugaacgaaucccucaccgauaccgcccggguguuaucgagcauggcagaugccgugcuggccaggguguacaaacaguccgaucuggacacucuggccaaggaggcgucaauuccuauuaucaacggccuuagugaccucuaccauccgauucagauccuggccgauuaccucacccugcaagaacacuacagcucccugaagggucugacauuguccuggaucggcgacggcaacaacauucuccauuccaucaugauguccgccgcaaaauucggcaugcaucuucaagccgccacgccgaaggguuacgagcccgacgcuuccgugacuaagcucgccgagcaguacgcuaaggagaacggaaccaagcuucugcugacuaacgacccacuagaagcagcccacgggggcaacgugcuuauuacugacaccuggaucuccaugggccaggaagaagagaaaaagaagcggcugcaggcguuccagggauaucaggucaccaugaaaaccgccaaggucgcugccuccgacuggaccuuccugcacugccugccucgcaagccugaagaaguggacgacgagguguucuacucgccacggagccucguguuccccgaggccgagaauagaaaguggaccaucauggccgugauggugucacugcucaccgacuacagcccgcagcuucagaagcccaaguucuagcucgagcuagugacugacuaggaucugguuaccacuaaaccagccucaagaacacccgaauggagucucuaagcuacauaauaccaacuuacacuuacaaaauguugucccccaaaauguagccauucguaucugcuccuaauaaaaagaaaguuucuucacauucuag

SEQ ID NO: 105 - RNA, 1485 nt, Artificial Sequence
  Synthetic construct
ucaacacaacauauacaaaacaaacgaaucucaagcaaucaagcauucuacuucuauugcagcaauuuaaaucauuucuuuuaaagcaaaagcaauuuucugaaaauuuucaccauuuacgaacgauagccaccaugggccuugucaaucuccgcauccuccuuaacaacgccgcguuuagaaacggccacaacuucaugguccggaacuucagauguggccagccgcuucaaaaccggguccagcugaagggccgggaucuucugacccugaagaacuuuacuggcgaagagaucaaguacaugcucuggcucuccgcggacuugaaguuccgcauuaagcagaagggggaauaccuuccgcugcuucaaggaaagagccucggcaugaucuuugagaagcgcucaaccaggacccgccuuucuacugaaacuggguucgcgcugcucgguggccaccccugcuuccugacgacccaggacauccaccucggagugaacgaaucccucaccgauaccgcccggguguuaucgagcauggcagaugccgugcuggccaggguguacaaacaguccgaucuggacacucuggccaaggaggcgucaauuccuauuaucaacggccuuagugaccucuaccauccgauucagauccuggccgauuaccucacccugcaagaacacuacagcucccugaagggucugacauuguccuggaucggcgacggcaacaacauucuccauuccaucaugauguccgccgcaaaauucggcaugcaucuucaagccgccacgccgaaggguuacgagcccgacgcuuccgugacuaagcucgccgagcaguacgcuaaggagaacggaaccaagcuucugcugacuaacgacccacuagaagcagcccacgggggcaacgugcuuauuacugacaccuggaucuccaugggccaggaagaagagaaaaagaagcggcugcaggcguuccagggauaucaggucaccaugaaaaccgccaaggucgcugccuccgacuggaccuuccugcacugccugccucgcaagccugaagaaguggacgacgagguguucuacucgccacggagccucguguuccccgaggccgagaauagaaaguggaccaucauggccgugauggugucacugcucaccgacuacagcccgcagcuucagaagcccaaguucuagcucgagcuagugacugacuaggaucugguuaccacuaaaccagccucaagaacacccgaauggagucucuaagcuacauaauaccaacuuacacuuacaaaauguugucccccaaaauguagccauucguaucugcuccuaauaaaaagaaaguuucuucacauucuagaaaaaaaaaaaaaaaaaaaaaaaaaaaaaaaaaaaaaaaaaaaaaaaaaaaaaaaaaaaaaaaaaaaaaaaaaaaaaaaaaaaaaaaaaaaaaaaaaaaaaaaaaaaaaaaaaa

SEQ ID NO: 106 - RNA, 1374 nt, Artificial Sequence
  Synthetic construct
ucaacacaacauauacaaaacaaacgaaucucaagcaaucaagcauucuacuucuauugcagcaauuuaaaucauuucuuuuaaagcaaaagcaauuuucugaaaauuuucaccauuuacgaacgauagccaccaugggcggacuugucaaucuccgcauccuccuuaacaacgccgcguuuagaaacggccacaacuucaugguccggaacuucagauguggccagccgcuucaaaacaagguccagcugaagggccgggaucuucugacccugaagaacuuuacuggcgaagagaucaaguacaugcucuggcucuccgcggacuugaaguuccgcauuaagcagaagggggaauaccuuccgcugcuucaaggaaagagccucggcaugaucuuugagaagcgcucaaccaggacccgccuuucuacugaaacuggguucgcgcugcucgguggccaccccugcuuccugacgacccaggacauccaccucggagugaacgaaucccucaccgauaccgcccggguguuaucgagcauggcagaugccgugcuggccaggguguacaaacaguccgaucuggacacucuggccaaggaggcgucaauuccuauuaucaacggccuuagugaccucuaccauccgauucagauccuggccgauuaccucacccugcaagaacacuacagcucccugaagggucugacauuguccuggaucggcgacggcaacaacauucuccauuccaucaugauguccgccgcaaaauucggcaugcaucuucaagccgccacgccgaaggguuacgagcccgacgcuuccgugacuaagcucgccgagcaguacgcuaaggagaacggaaccaagcuucugcugacuaacgacccacuagaagcagcccacgggggcaacgugcuuauuacugacaccuggaucuccaugggccaggaagaagagaaaaagaagcggcugcaggcguuccagggauaucaggucaccaugaaaaccgccaaggucgcugccuccgacuggaccuuccugcacugccugccucgcaagccugaagaaguggacgacgagguguucuacucgccacggagccucguguuccccgaggccgagaauagaaaguggaccaucauggccgugauggugucacugcucaccgacuacagcccgcagcuucagaagcccaaguucuagcucgagcuagugacugacuaggaucugguuaccacuaaaccagccucaagaacacccgaauggagucucuaagcuacauaauaccaacuuacacuuacaaaauguugucccccaaaauguagccauucguaucugcuccuaauaaaaagaaaguuucuucacauucuag

SEQ ID NO: 107 - RNA, 1377 nt, Artificial Sequence
  Synthetic construct
ucaacacaacauauacaaaacaaacgaaucucaagcaaucaagcauucuacuucuauugcagcaauuuaaaucauuucuuuuaaagcaaaagcaauuuucugaaaauuuucaccauuuacgaacgauagccauggcccuuuucaaucuccgcauccuccuuaacaacgccgcguuuagaaacggccacaacuucaugguccggaacuucagauguggccagccgcuucaaggcaagguccagcugaagggccgggaucuucugacccugaagaacuuuacuggcgaagagaucaaguacaugcucuggcucuccgcggacuugaaguuccgcauuaagcagaagggggaauaccuuccgcugcuucaaggaaagagccucggcaugaucuuugagaagcgcucaaccaggacccgccuuucuacugaaacuggguucgcgcugcucgguggccaccccugcuuccugacgacccaggacauccaccucggagugaacgaaucccucaccgauaccgcccggguguuaucgagcauggcagaugccgugcuggccaggguguacaaacaguccgaucuggacacucuggccaaggaggcgucaauuccuauuaucaacggccuuagugaccucuaccauccgauucagauccuggccgauuaccucacccugcaagaacacuacagcucccugaagggucugacauuguccuggaucggcgacggcaacaacauucuccauuccaucaugauguccgccgcaaaauucggcaugcaucuucaagccgccacgccgaaggguuacgagcccgacgcuuccgugacuaagcucgccgagcaguacgcuaaggagaacggaaccaagcuucugcugacuaacgacccacuagaagcagcccacgggggcaacgugcuuauuacugacaccuggaucuccaugggccaggaagaagagaaaaagaagcggcugcaggcguuccagggauaucaggucaccaugaaaaccgccaaggucgcugccuccgacuggaccuuccugcacugccugccucgcaagccugaagaaguggacgacgagguguucuacucgccacggagccucguguuccccgaggccgagaauagaaaguggaccaucauggccgugauggugucacugcucaccgacuacagcccgcagcuucagaagcccaaguucuagauaagugaacucgagcuagugacugacuaggaucugguuaccacuaaaccagccucaagaacacccgaauggagucucuaagcuacauaauaccaacuuacacuuacaaaauguugucccccaaaauguagccauucguaucugcuccuaauaaaaagaaaguuucuucacauucuag

SEQ ID NO: 108 - RNA, 1377 nt, Artificial Sequence
  Synthetic construct
ucaacacaacauauacaaaacaaacgaaucucaagcaaucaagcauucuacuucuauugcagcaauuuaaaucauuucuuuuaaagcaaaagcaauuuucugaaaauuuucaccauuuacgaacgauagccauggcccuuuucaaucuccgcauccuccuuaacaacgccgcguuuagaaacggccacaacuucaugguccggaacuucagauguggccagccgcuucaaggccggguccagcugaagggccgggaucuucugacccugaagaacuuuacuggcgaagagaucaaguacaugcucuggcucuccgcggacuugaaguuccgcauuaagcagaagggggaauaccuuccgcugcuucaaggaaagagccucggcaugaucuuugagaagcgcucaaccaggacccgccuuucuacugaaacuggguucgcgcugcucgguggccaccccugcuuccugacgacccaggacauccaccucggagugaacgaaucccucaccgauaccgcccggguguuaucgagcauggcagaugccgugcuggccaggguguacaaacaguccgaucuggacacucuggccaaggaggcgucaauuccuauuaucaacggccuuagugaccucuaccauccgauucagauccuggccgauuaccucacccugcaagaacacuacagcucccugaagggucugacauuguccuggaucggcgacggcaacaacauucuccauuccaucaugauguccgccgcaaaauucggcaugcaucuucaagccgccacgccgaaggguuacgagcccgacgcuuccgugacuaagcucgccgagcaguacgcuaaggagaacggaaccaagcuucugcugacuaacgacccacuagaagcagcccacgggggcaacgugcuuauuacugacaccuggaucuccaugggccaggaagaagagaaaaagaagcggcugcaggcguuccagggauaucaggucaccaugaaaaccgccaaggucgcugccuccgacuggaccuuccugcacugccugccucgcaagccugaagaaguggacgacgagguguucuacucgccacggagccucguguuccccgaggccgagaauagaaaguggaccaucauggccgugauggugucacugcucaccgacuacagcccgcagcuucagaagcccaaguucuagauaagugaacucgagcuagugacugacuaggaucugguuaccacuaaaccagccucaagaacacccgaauggagucucuaagcuacauaauaccaacuuacacuuacaaaauguugucccccaaaauguagccauucguaucugcuccuaauaaaaagaaaguuucuucacauucuag

SEQ ID NO: 109 - RNA, 1377 nt, Artificial Sequence
  Synthetic construct
ucaacacaacauauacaaaacaaacgaaucucaagcaaucaagcauucuacuucuauugcagcaauuuaaaucauuucuuuuaaagcaaaagcaauuuucugaaaauuuucaccauuuacgaacgauagccauggcccuuuucaaucuccgcauccuccuuaacaacgccgcguuuagaaacggccacaacuucaugguccggaacuucagauguggccagccgcuucaaggccggguccagcugaagggccgggaucuucugacccugaagaacuuuacuggcgaagagaucagguacaugcucuggcucuccgcggacuugaaguuccgcauuaagcagaagggggaauaccuuccgcugcuucaaggaaagagccucggcaugaucuuugagaagcgcucaaccaggacccgccuuucuacugaaacuggguucgcgcugcucgguggccaccccugcuuccugacgacccaggacauccaccucggagugaacgaaucccucaccgauaccgcccggguguuaucgagcauggcagaugccgugcuggccaggguguacaaacaguccgaucuggacacucuggccaaggaggcgucaauuccuauuaucaacggccuuagugaccucuaccauccgauucagauccuggccgauuaccucacccugcaagaacacuacagcucccugaagggucugacauuguccuggaucggcgacggcaacaacauucuccauuccaucaugauguccgccgcaaaauucggcaugcaucuucaagccgccacgccgaaggguuacgagcccgacgcuuccgugacuaagcucgccgagcaguacgcuaaggagaacggaaccaagcuucugcugacuaacgacccacuagaagcagcccacgggggcaacgugcuuauuacugacaccuggaucuccaugggccaggaagaagagaaaaagaagcggcugcaggcguuccagggauaucaggucaccaugaaaaccgccaaggucgcugccuccgacuggaccuuccugcacugccugccucgcaagccugaagaaguggacgacgagguguucuacucgccacggagccucguguuccccgaggccgagaauagaaaguggaccaucauggccgugauggugucacugcucaccgacuacagcccgcagcuucagaagcccaaguucuagauaagugaacucgagcuagugacugacuaggaucugguuaccacuaaaccagccucaagaacacccgaauggagucucuaagcuacauaauaccaacuuacacuuacaaaauguugucccccaaaauguagccauucguaucugcuccuaauaaaaagaaaguuucuucacauucuag

SEQ ID NO: 110 - RNA, 1377 nt, Artificial Sequence
  Synthetic construct
ucaacacaacauauacaaaacaaacgaaucucaagcaaucaagcauucuacuucuauugcagcaauuuaaaucauuucuuuuaaagcaaaagcaauuuucugaaaauuuucaccauuuacgaacgauagccauggcccuugucaaucuccgcauccuccuuaacaacgccgcguuuagaaacggccacaacuucaugguccggaacuucagauguggccagccgcuucaaggcaggguccagcugaagggccgggaucuucugacccugaagaacuuuacuggcgaagagaucaaguacaugcucuggcucuccgcggacuugaaguuccgcauuaagcagaagggggaauaccuuccgcugcuucaaggaaagagccucggcaugaucuuugagaagcgcucaaccaggacccgccuuucuacugaaacuggguucgcgcugcucgguggccaccccugcuuccugacgacccaggacauccaccucggagugaacgaaucccucaccgauaccgcccggguguuaucgagcauggcagaugccgugcuggccaggguguacaaacaguccgaucuggacacucuggccaaggaggcgucaauuccuauuaucaacggccuuagugaccucuaccauccgauucagauccuggccgauuaccucacccugcaagaacacuacagcucccugaagggucugacauuguccuggaucggcgacggcaacaacauucuccauuccaucaugauguccgccgcaaaauucggcaugcaucuucaagccgccacgccgaaggguuacgagcccgacgcuuccgugacuaagcucgccgagcaguacgcuaaggagaacggaaccaagcuucugcugacuaacgacccacuagaagcagcccacgggggcaacgugcuuauuacugacaccuggaucuccaugggccaggaagaagagaaaaagaagcggcugcaggcguuccagggauaucaggucaccaugaaaaccgccaaggucgcugccuccgacuggaccuuccugcacugccugccucgcaagccugaagaaguggacgacgagguguucuacucgccacggagccucguguuccccgaggccgagaauagaaaguggaccaucauggccgugauggugucacugcucaccgacuacagcccgcagcuucagaagcccaaguucuaagugaauagacucgagcuagugacugacuaggaucugguuaccacuaaaccagccucaagaacacccgaauggagucucuaagcuacauaauaccaacuuacacuuacaaaauguugucccccaaaauguagccauucguaucugcuccuaauaaaaagaaaguuucuucacauucuag

SEQ ID NO: 111 - RNA, 1496 nt, Artificial Sequence
  Synthetic construct
ucaacacaacauauacaaaacaaacgaaucucaagcaaucaagcauucuacuucuauugcagcaauuuaaaucauuucuuuuaaagcaaaagcaauuuucugaaaauuuucaccauuuacgaacgauagccauggcccuuuucaaucuccgcauccuccuuaacaacgccgcguuuagaaacggccacaacuucaugguccggaacuucagauguggccagccgcuucaagucaagguccagcugaagggccgggaucuucugacccugaagaacuuuacuggcgaagagaucaaguacaugcucuggcucuccgcggacuugaaguuccgcauuaagcagaagggggaauaccuuccgcugcuucaaggaaagagccucggcaugaucuuugagaagcgcucaaccaggacccgccuuucuacugaaacuggguucgcgcugcucgguggccaccccugcuuccugacgacccaggacauccaccucggagugaacgaaucccucaccgauaccgcccggguguuaucgagcauggcagaugccgugcuggccaggguguacaaacaguccgaucuggacacucuggccaaggaggcgucaauuccuauuaucaacggccuuagugaccucuaccauccgauucagauccuggccgauuaccucacccugcaagaacacuacagcucccugaagggucugacauuguccuggaucggcgacggcaacaacauucuccauuccaucaugauguccgccgcaaaauucggcaugcaucuucaagccgccacgccgaaggguuacgagcccgacgcuuccgugacuaagcucgccgagcaguacgcuaaggagaacggaaccaagcuucugcugacuaacgacccacuagaagcagcccacgggggcaacgugcuuauuacugacaccuggaucuccaugggccaggaagaagagaaaaagaagcggcugcaggcguuccagggauaucaggucaccaugaaaaccgccaaggucgcugccuccgacuggaccuuccugcacugccugccucgcaagccugaagaaguggacgacgagguguucuacucgccacggagccucguguuccccgaggccgagaauagaaaguggaccaucauggccgugauggugucacugcucaccgacuacagcccgcagcuucagaagcccaaguucuagauaagugaacucgagcuagugacugacuaggaucugguuaccacuaaaccagccucaagaacacccgaauggagucucuaagcuacauaauaccaacuuacacuuacaaaauguugucccccaaaauguagccauucguaucugcuccuaauaaaaagaaaguuucuucacauucuagaaaaaaaaaaaaaaaaaaaaaaaaaaaaaaaaaaaaaaaaaaaaaaaaaaaaaaaaaaaaaaaaaaaaaaaaaaaaaaaaaaaaaaaaaaaaaaaaaaaaaaaaaaaaaaaaaaaaaaa

SEQ ID NO: 112 - RNA, 1377 nt, Artificial Sequence
  Synthetic construct
ucaacacaacauauacaaaacaaacgaaucucaagcaaucaagcauucuacuucuauugcagcaauuuaaaucauuucuuuuaaagcaaaagcaauuuucugaaaauuuucaccauuuacgaacgauagccauggcccuuuucaaucuccgcauccuccuuaacaacgccgcguuuagaaacggccacaacuucaugguccggaacuucagauguggccagccgcuucaagucaggguccagcugaagggccgggaucuucugacccugaagaacuuuacuggcgaagagaucaaguacaugcucuggcucuccgcggacuugaaguuccgcauuaagcagaagggggaauaccuuccgcugcuucaaggaaagagccucggcaugaucuuugagaagcgcucaaccaggacccgccuuucuacugaaacuggguucgcgcugcucgguggccaccccugcuuccugacgacccaggacauccaccucggagugaacgaaucccucaccgauaccgcccggguguuaucgagcauggcagaugccgugcuggccaggguguacaaacaguccgaucuggacacucuggccaaggaggcgucaauuccuauuaucaacggccuuagugaccucuaccauccgauucagauccuggccgauuaccucacccugcaagaacacuacagcucccugaagggucugacauuguccuggaucggcgacggcaacaacauucuccauuccaucaugauguccgccgcaaaauucggcaugcaucuucaagccgccacgccgaaggguuacgagcccgacgcuuccgugacuaagcucgccgagcaguacgcuaaggagaacggaaccaagcuucugcugacuaacgacccacuagaagcagcccacgggggcaacgugcuuauuacugacaccuggaucuccaugggccaggaagaagagaaaaagaagcggcugcaggcguuccagggauaucaggucaccaugaaaaccgccaaggucgcugccuccgacuggaccuuccugcacugccugccucgcaagccugaagaaguggacgacgagguguucuacucgccacggagccucguguuccccgaggccgagaauagaaaguggaccaucauggccgugauggugucacugcucaccgacuacagcccgcagcuucagaagcccaaguucuagauaagugaacucgagcuagugacugacuaggaucugguuaccacuaaaccagccucaagaacacccgaauggagucucuaagcuacauaauaccaacuuacacuuacaaaauguugucccccaaaauguagccauucguaucugcuccuaauaaaaagaaaguuucuucacauucuag

SEQ ID NO: 113 - RNA, 1282 nt, Artificial Sequence
  Synthetic construct
ggcagaaaaauuugcuacauuguuucacaaacuucaaauauuauucauuuauuuagaucuauuauuacaucaaaacaaaaagccgccaccaugcuguucaaccugcgcauccugcugaacaacgccgccuuccgcaacggccacaacuucauggugcgcaacuuccgcugcggccagccccugcagaacaaggugcagcugaagggccgcgaccugcugacccugaagaacuucaccggcgaggagaucaaguacaugcuguggcugagcgccgaccugaaguuccgcaucaagcagaagggcgaguaccugccccugcugcagggcaagagccugggcaugaucuucgagaagcgcagcacccgcacccgccugagcaccgagacaggcuucgcccugcugggcggccaccccugcuuccugaccacccaggacauccaccugggcgugaacgagagccugaccgacaccgcccgcgugcugagcagcauggccgacgccgugcuggcccgcguguacaagcagagcgaccuggacacccuggccaaggaggccagcauccccaucaucaacggccugagcgaccuguaccaccccauccagauccuggccgacuaccugacccugcaggagcacuacagcagccugaagggccugacccugagcuggaucggcgacggcaacaacauccugcacagcaucaugaugagcgccgccaaguucggcaugcaccugcaggccgccacccccaagggcuacgagcccgacgccagcgugaccaagcuggccgagcaguacgccaaggagaacggcaccaagcugcugcugaccaacgacccccuggaggccgcccacggcggcaacgugcugaucaccgacaccuggaucagcaugggccaggaggaggagaagaagaagcgccugcaggccuuccagggcuaccaggugaccaugaagaccgccaagguggccgccagcgacuggaccuuccugcacugccugccccgcaagcccgaggagguggacgacgagguguucuacagcccccgcagccugguguuccccgaggccgagaaccgcaaguggaccaucauggccgugauggugagccugcugaccgacuacagcccccagcugcagaagcccaaguucugaggucucuaguaaugagcuggagccucgguagccguuccuccugcccgcugggccucccaacgggcccuccuccccuccuugcaccggcccuuccuggucuuugaauaaagucugagugggcaucuag

SEQ ID NO: 114 - RNA, 1285 nt, Artificial Sequence
  Synthetic construct
ggcagaaaaauuugcuacauuguuucacaaacuucaaauauuauucauuuauuuagaucuauuauuacaucaaaacaaaaagccgccaccaugggaguauucaaccugcgcauccugcugaacaacgccgccuuccgcaacggccacaacuucauggugcgcaacuuccgcugcggccagccccugcagaacaaggugcagcugaagggccgcgaccugcugacccugaagaacuucaccggcgaggagaucaaguacaugcuguggcugagcgccgaccugaaguuccgcaucaagcagaagggcgaguaccugccccugcugcagggcaagagccugggcaugaucuucgagaagcgcagcacccgcacccgccugagcaccgagacaggcuucgcccugcugggcggccaccccugcuuccugaccacccaggacauccaccugggcgugaacgagagccugaccgacaccgcccgcgugcugagcagcauggccgacgccgugcuggcccgcguguacaagcagagcgaccuggacacccuggccaaggaggccagcauccccaucaucaacggccugagcgaccuguaccaccccauccagauccuggccgacuaccugacccugcaggagcacuacagcagccugaagggccugacccugagcuggaucggcgacggcaacaacauccugcacagcaucaugaugagcgccgccaaguucggcaugcaccugcaggccgccacccccaagggcuacgagcccgacgccagcgugaccaagcuggccgagcaguacgccaaggagaacggcaccaagcugcugcugaccaacgacccccuggaggccgcccacggcggcaacgugcugaucaccgacaccuggaucagcaugggccaggaggaggagaagaagaagcgccugcaggccuuccagggcuaccaggugaccaugaagaccgccaagguggccgccagcgacuggaccuuccugcacugccugccccgcaagcccgaggagguggacgacgagguguucuacagcccccgcagccugguguuccccgaggccgagaaccgcaaguggaccaucauggccgugauggugagccugcugaccgacuacagcccccagcugcagaagcccaaguucugaggucucuaguaaugagcuggagccucgguagccguuccuccugcccgcugggccucccaacgggcccuccuccccuccuugcaccggcccuuccuggucuuugaauaaagucugagugggcaucuag

SEQ ID NO: 115 - RNA, 1285 nt, Artificial Sequence
  Synthetic construct
ggcagaaaaauuugcuacauuguuucacaaacuucaaauauuauucauuuauuuagaucuauuauuacaucaaaacaaaaagccgccaccaugggaguauucaaccugcgcauccugcugaacaacgccgccuuccgcaacggccacaacuucauggugcgcaacuuccgcugcggccagccccugcagaaccgggugcagcugaagggccgcgaccugcugacccugaagaacuucaccggcgaggagauccgguacaugcuguggcugagcgccgaccugaaguuccgcaucaagcagaagggcgaguaccugccccugcugcagggcaagagccugggcaugaucuucgagaagcgcagcacccgcacccgccugagcaccgagacaggcuucgcccugcugggcggccaccccugcuuccugaccacccaggacauccaccugggcgugaacgagagccugaccgacaccgcccgcgugcugagcagcauggccgacgccgugcuggcccgcguguacaagcagagcgaccuggacacccuggccaaggaggccagcauccccaucaucaacggccugagcgaccuguaccaccccauccagauccuggccgacuaccugacccugcaggagcacuacagcagccugaagggccugacccugagcuggaucggcgacggcaacaacauccugcacagcaucaugaugagcgccgccaaguucggcaugcaccugcaggccgccacccccaagggcuacgagcccgacgccagcgugaccaagcuggccgagcaguacgccaaggagaacggcaccaagcugcugcugaccaacgacccccuggaggccgcccacggcggcaacgugcugaucaccgacaccuggaucagcaugggccaggaggaggagaagaagaagcgccugcaggccuuccagggcuaccaggugaccaugaagaccgccaagguggccgccagcgacuggaccuuccugcacugccugccccgcaagcccgaggagguggacgacgagguguucuacagcccccgcagccugguguuccccgaggccgagaaccgcaaguggaccaucauggccgugauggugagccugcugaccgacuacagcccccagcugcagaagcccaaguucugaggucucuaguaaugagcuggagccucgguagccguuccuccugcccgcugggccucccaacgggcccuccuccccuccuugcaccggcccuuccuggucuuugaauaaagucugagugggcaucuag

SEQ ID NO: 116 - RNA, 1285 nt, Artificial Sequence
  Synthetic construct
ggcagaaaaauuugcuacauuguuucacaaacuucaaauauuauucauuuauuuagaucuauuauuacaucaaaacaaaaagccgccaccaugcugguauucaaccugcgcauccugcugaacaacgccgccuuccgcaacggccacaacuucauggugcgcaacuuccgcugcggccagccccugcagaaccgggugcagcugaagggccgcgaccugcugacccugaagaacuucaccggcgaggagauccgguacaugcuguggcugagcgccgaccugaaguuccgcaucaagcagaagggcgaguaccugccccugcugcagggcaagagccugggcaugaucuucgagaagcgcagcacccgcacccgccugagcaccgagacaggcuucgcccugcugggcggccaccccugcuuccugaccacccaggacauccaccugggcgugaacgagagccugaccgacaccgcccgcgugcugagcagcauggccgacgccgugcuggcccgcguguacaagcagagcgaccuggacacccuggccaaggaggccagcauccccaucaucaacggccugagcgaccuguaccaccccauccagauccuggccgacuaccugacccugcaggagcacuacagcagccugaagggccugacccugagcuggaucggcgacggcaacaacauccugcacagcaucaugaugagcgccgccaaguucggcaugcaccugcaggccgccacccccaagggcuacgagcccgacgccagcgugaccaagcuggccgagcaguacgccaaggagaacggcaccaagcugcugcugaccaacgacccccuggaggccgcccacggcggcaacgugcugaucaccgacaccuggaucagcaugggccaggaggaggagaagaagaagcgccugcaggccuuccagggcuaccaggugaccaugaagaccgccaagguggccgccagcgacuggaccuuccugcacugccugccccgcaagcccgaggagguggacgacgagguguucuacagcccccgcagccugguguuccccgaggccgagaaccgcaaguggaccaucauggccgugauggugagccugcugaccgacuacagcccccagcugcagaagcccaaguucugaggucucuaguaaugagcuggagccucgguagccguuccuccugcccgcugggccucccaacgggcccuccuccccuccuugcaccggcccuuccuggucuuugaauaaagucugagugggcaucuag

SEQ ID NO: 117 - RNA, 1225 nt, Artificial Sequence
  Synthetic construct
auuauuacaucaaaacaaaaagccgccaccaugggaguauucaaccugcgcauccugcugaacaacgccgccuuccgcaacggccacaacuucauggugcgcaacuuccgcugcggccagccccugcagaacaaggugcagcugaagggccgcgaccugcugacccugaagaacuucaccggcgaggagaucaaguacaugcuguggcugagcgccgaccugaaguuccgcaucaagcagaagggcgaguaccugccccugcugcagggcaagagccugggcaugaucuucgagaagcgcagcacccgcacccgccugagcaccgagacaggcuucgcccugcugggcggccaccccugcuuccugaccacccaggacauccaccugggcgugaacgagagccugaccgacaccgcccgcgugcugagcagcauggccgacgccgugcuggcccgcguguacaagcagagcgaccuggacacccuggccaaggaggccagcauccccaucaucaacggccugagcgaccuguaccaccccauccagauccuggccgacuaccugacccugcaggagcacuacagcagccugaagggccugacccugagcuggaucggcgacggcaacaacauccugcacagcaucaugaugagcgccgccaaguucggcaugcaccugcaggccgccacccccaagggcuacgagcccgacgccagcgugaccaagcuggccgagcaguacgccaaggagaacggcaccaagcugcugcugaccaacgacccccuggaggccgcccacggcggcaacgugcugaucaccgacaccuggaucagcaugggccaggaggaggagaagaagaagcgccugcaggccuuccagggcuaccaggugaccaugaagaccgccaagguggccgccagcgacuggaccuuccugcacugccugccccgcaagcccgaggagguggacgacgagguguucuacagcccccgcagccugguguuccccgaggccgagaaccgcaaguggaccaucauggccgugauggugagccugcugaccgacuacagcccccagcugcagaagcccaaguucugaggucucuaguaaugagcuggagccucgguagccguuccuccugcccgcugggccucccaacgggcccuccuccccuccuugcaccggcccuuccuggucuuugaauaaagucugagugggcaucuag

SEQ ID NO: 118 - RNA, 1225 nt, Artificial Sequence
  Synthetic construct
auuauuacaucaaaacaaaaagccgccaccaugggaguauucaaccugcgcauccugcugaacaacgccgccuuccgcaacggccacaacuucauggugcgcaacuuccgcugcggccagccccugcagaaccgggugcagcugaagggccgcgaccugcugacccugaagaacuucaccggcgaggagauccgguacaugcuguggcugagcgccgaccugaaguuccgcaucaagcagaagggcgaguaccugccccugcugcagggcaagagccugggcaugaucuucgagaagcgcagcacccgcacccgccugagcaccgagacaggcuucgcccugcugggcggccaccccugcuuccugaccacccaggacauccaccugggcgugaacgagagccugaccgacaccgcccgcgugcugagcagcauggccgacgccgugcuggcccgcguguacaagcagagcgaccuggacacccuggccaaggaggccagcauccccaucaucaacggccugagcgaccuguaccaccccauccagauccuggccgacuaccugacccugcaggagcacuacagcagccugaagggccugacccugagcuggaucggcgacggcaacaacauccugcacagcaucaugaugagcgccgccaaguucggcaugcaccugcaggccgccacccccaagggcuacgagcccgacgccagcgugaccaagcuggccgagcaguacgccaaggagaacggcaccaagcugcugcugaccaacgacccccuggaggccgcccacggcggcaacgugcugaucaccgacaccuggaucagcaugggccaggaggaggagaagaagaagcgccugcaggccuuccagggcuaccaggugaccaugaagaccgccaagguggccgccagcgacuggaccuuccugcacugccugccccgcaagcccgaggagguggacgacgagguguucuacagcccccgcagccugguguuccccgaggccgagaaccgcaaguggaccaucauggccgugauggugagccugcugaccgacuacagcccccagcugcagaagcccaaguucugaggucucuaguaaugagcuggagccucgguagccguuccuccugcccgcugggccucccaacgggcccuccuccccuccuugcaccggcccuuccuggucuuugaauaaagucugagugggcaucuag

SEQ ID NO: 119 - RNA, 1225 nt, Artificial Sequence
  Synthetic construct
auuauuacaucaaaacaaaaagccgccaccaugcugguauucaaccugcgcauccugcugaacaacgccgccuuccgcaacggccacaacuucauggugcgcaacuuccgcugcggccagccccugcagaaccgggugcagcugaagggccgcgaccugcugacccugaagaacuucaccggcgaggagauccgguacaugcuguggcugagcgccgaccugaaguuccgcaucaagcagaagggcgaguaccugccccugcugcagggcaagagccugggcaugaucuucgagaagcgcagcacccgcacccgccugagcaccgagacaggcuucgcccugcugggcggccaccccugcuuccugaccacccaggacauccaccugggcgugaacgagagccugaccgacaccgcccgcgugcugagcagcauggccgacgccgugcuggcccgcguguacaagcagagcgaccuggacacccuggccaaggaggccagcauccccaucaucaacggccugagcgaccuguaccaccccauccagauccuggccgacuaccugacccugcaggagcacuacagcagccugaagggccugacccugagcuggaucggcgacggcaacaacauccugcacagcaucaugaugagcgccgccaaguucggcaugcaccugcaggccgccacccccaagggcuacgagcccgacgccagcgugaccaagcuggccgagcaguacgccaaggagaacggcaccaagcugcugcugaccaacgacccccuggaggccgcccacggcggcaacgugcugaucaccgacaccuggaucagcaugggccaggaggaggagaagaagaagcgccugcaggccuuccagggcuaccaggugaccaugaagaccgccaagguggccgccagcgacuggaccuuccugcacugccugccccgcaagcccgaggagguggacgacgagguguucuacagcccccgcagccugguguuccccgaggccgagaaccgcaaguggaccaucauggccgugauggugagccugcugaccgacuacagcccccagcugcagaagcccaaguucugaggucucuaguaaugagcuggagccucgguagccguuccuccugcccgcugggccucccaacgggcccuccuccccuccuugcaccggcccuuccuggucuuugaauaaagucugagugggcaucuag

SEQ ID NO: 120 - RNA, 1376 nt, Artificial Sequence
  Synthetic construct
ucaacacaacauauacaaaacaaacgaaucucaagcaaucaagcauucuacuucuauugcagcaauuuaaaucauuucuuuuaaagcaaaagcaauuuucugaaaauuuucaccauuuacgaacgauagccaccauguuguucaacuugaggaucuuguugaacaacgccgccuucaggaacggacacaacuucaugguaaggaacuucaggugcggacagcccuugcagaacaaaguacaguugaaaggaagggacuuguugacauugaaaaacuucacaggagaagaaaucaaauacauguugugguugucggccgacuugaaauucaggaucaaacagaaaggagaauacuugcccuuguugcagggaaaaucguugggaaugaucuucgaaaaaaggucgacaaggacaagguugucgacagaaacaggauucgccuuguugggaggacaccccugcuucuugacaacacaggacauccacuugggaguaaacgaaucguugacagacacagccaggguauugucgucgauggccgacgccguauuggccaggguauacaaacagucggacuuggacacauuggccaaagaagccucgauccccaucaucaacggauugucggacuuguaccaccccauccagaucuuggccgacuacuugacauugcaggaacacuacucgucguugaaaggauugacauugucguggaucggagacggaaacaacaucuugcacucgaucaugaugucggccgccaaauucggaaugcacuugcaggccgccacacccaaaggauacgaacccgacgccucgguaacaaaauuggccgaacaguacgccaaagaaaacggaacaaaauuguuguugacaaacgaccccuuggaagccgcccacggaggaaacguauugaucacagacacauggaucucgaugggacaggaagaagaaaaaaaaaaaagguugcaggccuuccagggauaccagguaacaaugaaaacagccaaaguagccgccucggacuggacauucuugcacugcuugcccaggaaacccgaagaaguagacgacgaaguauucuacucgcccaggucguugguauuccccgaagccgaaaacaggaaauggacaaucauggccguaaugguaucguuguugacagacuacucgccccaguugcagaaacccaaauucugaauagugaacucgagcuagugacugacuaggaucugguuaccacuaaaccagccucaagaacacccgaauggagucucuaagcuacauaauaccaacuuacacuuacaaaauguugucccccaaaauguagccauucguaucugcuccuaauaaaaagaaaguuucuucacauucuag

SEQ ID NO: 121 - RNA, 1222 nt, Artificial Sequence
  Synthetic construct
auuauuacaucaaaacaaaaagccgccaccaugcuguucaaccugcgcauccugcugaacaacgccgccuuccgcaacggccacaacuucauggugcgcaacuuccgcugcggccagccccugcagggcaaggugcagcugaagggccgcgaccugcugacccugaagaacuucaccggcgaggagaucaaguacaugcuguggcugagcgccgaccugaaguuccgcaucaagcagaagggcgaguaccugccccugcugcagggcaagagccugggcaugaucuucgagaagcgcagcacccgcacccgccugagcaccgagacaggcuucgcccugcugggcggccaccccugcuuccugaccacccaggacauccaccugggcgugaacgagagccugaccgacaccgcccgcgugcugagcagcauggccgacgccgugcuggcccgcguguacaagcagagcgaccuggacacccuggccaaggaggccagcauccccaucaucaacggccugagcgaccuguaccaccccauccagauccuggccgacuaccugacccugcaggagcacuacagcagccugaagggccugacccugagcuggaucggcgacggcaacaacauccugcacagcaucaugaugagcgccgccaaguucggcaugcaccugcaggccgccacccccaagggcuacgagcccgacgccagcgugaccaagcuggccgagcaguacgccaaggagaacggcaccaagcugcugcugaccaacgacccccuggaggccgcccacggcggcaacgugcugaucaccgacaccuggaucagcaugggccaggaggaggagaagaagaagcgccugcaggccuuccagggcuaccaggugaccaugaagaccgccaagguggccgccagcgacuggaccuuccugcacugccugccccgcaagcccgaggagguggacgacgagguguucuacagcccccgcagccugguguuccccgaggccgagaaccgcaaguggaccaucauggccgugauggugagccugcugaccgacuacagcccccagcugcagaagcccaaguucugaggucucuaguaaugagcuggagccucgguagccguuccuccugcccgcugggccucccaacgggcccuccuccccuccuugcaccggcccuuccuggucuuugaauaaagucugagugggcaucuag

SEQ ID NO: 122 - RNA, 1222 nt, Artificial Sequence
  Synthetic construct
auuauuacaucaaaacaaaaagccgccaccaugcuguucaaccugcgcauccugcugaacaacgccgccuuccgcaacggccacaacuucauggugcgcaacuuccgcugcggccagccccugcagggccgggugcagcugaagggccgcgaccugcugacccugaagaacuucaccggcgaggagaucaaguacaugcuguggcugagcgccgaccugaaguuccgcaucaagcagaagggcgaguaccugccccugcugcagggcaagagccugggcaugaucuucgagaagcgcagcacccgcacccgccugagcaccgagacaggcuucgcccugcugggcggccaccccugcuuccugaccacccaggacauccaccugggcgugaacgagagccugaccgacaccgcccgcgugcugagcagcauggccgacgccgugcuggcccgcguguacaagcagagcgaccuggacacccuggccaaggaggccagcauccccaucaucaacggccugagcgaccuguaccaccccauccagauccuggccgacuaccugacccugcaggagcacuacagcagccugaagggccugacccugagcuggaucggcgacggcaacaacauccugcacagcaucaugaugagcgccgccaaguucggcaugcaccugcaggccgccacccccaagggcuacgagcccgacgccagcgugaccaagcuggccgagcaguacgccaaggagaacggcaccaagcugcugcugaccaacgacccccuggaggccgcccacggcggcaacgugcugaucaccgacaccuggaucagcaugggccaggaggaggagaagaagaagcgccugcaggccuuccagggcuaccaggugaccaugaagaccgccaagguggccgccagcgacuggaccuuccugcacugccugccccgcaagcccgaggagguggacgacgagguguucuacagcccccgcagccugguguuccccgaggccgagaaccgcaaguggaccaucauggccgugauggugagccugcugaccgacuacagcccccagcugcagaagcccaaguucugaggucucuaguaaugagcuggagccucgguagccguuccuccugcccgcugggccucccaacgggcccuccuccccuccuugcaccggcccuuccuggucuuugaauaaagucugagugggcaucuag

SEQ ID NO: 123 - RNA, 1222 nt, Artificial Sequence
  Synthetic construct
auuauuacaucaaaacaaaaagccgccaccaugcuguucaaccugcgcauccugcugaacaacgccgccuuccgcaacggccacaacuucauggugcgcaacuuccgcugcggccagccccugcagggccgggugcagcugaagggccgcgaccugcugacccugaagaacuucaccggcgaggagauccgguacaugcuguggcugagcgccgaccugaaguuccgcaucaagcagaagggcgaguaccugccccugcugcagggcaagagccugggcaugaucuucgagaagcgcagcacccgcacccgccugagcaccgagacaggcuucgcccugcugggcggccaccccugcuuccugaccacccaggacauccaccugggcgugaacgagagccugaccgacaccgcccgcgugcugagcagcauggccgacgccgugcuggcccgcguguacaagcagagcgaccuggacacccuggccaaggaggccagcauccccaucaucaacggccugagcgaccuguaccaccccauccagauccuggccgacuaccugacccugcaggagcacuacagcagccugaagggccugacccugagcuggaucggcgacggcaacaacauccugcacagcaucaugaugagcgccgccaaguucggcaugcaccugcaggccgccacccccaagggcuacgagcccgacgccagcgugaccaagcuggccgagcaguacgccaaggagaacggcaccaagcugcugcugaccaacgacccccuggaggccgcccacggcggcaacgugcugaucaccgacaccuggaucagcaugggccaggaggaggagaagaagaagcgccugcaggccuuccagggcuaccaggugaccaugaagaccgccaagguggccgccagcgacuggaccuuccugcacugccugccccgcaagcccgaggagguggacgacgagguguucuacagcccccgcagccugguguuccccgaggccgagaaccgcaaguggaccaucauggccgugauggugagccugcugaccgacuacagcccccagcugcagaagcccaaguucugaggucucuaguaaugagcuggagccucgguagccguuccuccugcccgcugggccucccaacgggcccuccuccccuccuugcaccggcccuuccuggucuuugaauaaagucugagugggcaucuag

SEQ ID NO: 124 - RNA, 1282 nt, Artificial Sequence
  Synthetic construct
ggcagaaaaauuugcuacauuguuucacaaacuucaaauauuauucauuuauuuagaucuauuauuacaucaaaacaaaaagccgccaccaugcuguucaaccugcgcauccugcugaacaacgccgccuuccgcaacggccacaacuucauggugcgcaacuuccgcugcggccagccccugcagggcaaggugcagcugaagggccgcgaccugcugacccugaagaacuucaccggcgaggagaucaaguacaugcuguggcugagcgccgaccugaaguuccgcaucaagcagaagggcgaguaccugccccugcugcagggcaagagccugggcaugaucuucgagaagcgcagcacccgcacccgccugagcaccgagacaggcuucgcccugcugggcggccaccccugcuuccugaccacccaggacauccaccugggcgugaacgagagccugaccgacaccgcccgcgugcugagcagcauggccgacgccgugcuggcccgcguguacaagcagagcgaccuggacacccuggccaaggaggccagcauccccaucaucaacggccugagcgaccuguaccaccccauccagauccuggccgacuaccugacccugcaggagcacuacagcagccugaagggccugacccugagcuggaucggcgacggcaacaacauccugcacagcaucaugaugagcgccgccaaguucggcaugcaccugcaggccgccacccccaagggcuacgagcccgacgccagcgugaccaagcuggccgagcaguacgccaaggagaacggcaccaagcugcugcugaccaacgacccccuggaggccgcccacggcggcaacgugcugaucaccgacaccuggaucagcaugggccaggaggaggagaagaagaagcgccugcaggccuuccagggcuaccaggugaccaugaagaccgccaagguggccgccagcgacuggaccuuccugcacugccugccccgcaagcccgaggagguggacgacgagguguucuacagcccccgcagccugguguuccccgaggccgagaaccgcaaguggaccaucauggccgugauggugagccugcugaccgacuacagcccccagcugcagaagcccaaguucugaggucucuaguaaugagcuggagccucgguagccguuccuccugcccgcugggccucccaacgggcccuccuccccuccuugcaccggcccuuccuggucuuugaauaaagucugagugggcaucuag

SEQ ID NO: 125 - RNA, 21 nt, Artificial Sequence
  Synthetic construct
cacaaagaguaaagaagaaca

SEQ ID NO: 126 - RNA, 21 nt, Artificial Sequence
  Synthetic construct
aacacuaaaaguagaagaaaa

SEQ ID NO: 127 - RNA, 21 nt, Artificial Sequence
  Synthetic construct
cucagaaagauaagaucagcc

SEQ ID NO: 128 - DNA, 1065 bp, Artificial Sequence; identical to SEQ ID NO: 2
  Synthetic construct

SEQ ID NO: 129 - DNA, 1065 bp, Artificial Sequence
  Synthetic construct
atgctctttaatctgcgcatcttactgaacaacgccgcattccggaacggtcacaacttcatggtccgcaatttccgctgtggccagccgcttcaaaacaaggtccagctgaagggacgggatctgctgacactgaagaacttcaccggagaagagatcaagtacatgctgtggctcagcgcagacttgaagttccggatcaagcagaagggagaatacttgcccctgctgcaaggaaagtcgctgggaatgatttttgagaagcggtcaactcgcaccagactctccaccgaaactggtttcgcactgcttggcgggcacccttgcttcctgacgactcaggacatccacctcggcgtgaacgaatcgctaaccgataccgccagagtgctttcttccatggccgacgcggtgctggccagggtgtacaagcagtccgacctcgataccttggcaaaggaggcttccattcccatcatcaacggcctgagcgacctgtaccacccaatccaaatcctggctgactacctgaccctgcaagagcactacagcagcctgaagggtctgaccctgtcatggattggcgatggaaacaatattctgcactccatcatgatgtccgccgcgaagttcggaatgcatctgcaagccgccactccaaaaggatacgaaccggatgcgtccgtgaccaagttggcggaacagtacgcgaaggagaacggaaccaagcttctgctgactaacgaccccctcgaggctgcgcatgggggcaacgtgctgattaccgacacctggatctccatggggcaggaggaagagaagaagaagagactgcaggcattccaggggtaccaggtcaccatgaaaaccgcaaaagtggcagcttcggactggactttcctgcattgcctgccgaggaagccggaggaagtcgacgacgaagtgttctactcgcctcggtccctggtgttccccgaggccgaaaaccggaagtggaccatcatggccgtgatggtgtccttgctgactgactatagcccgcagctgcagaagcctaagttctag

SEQ ID NO: 130 - DNA, 1065 bp, Artificial Sequence
  Synthetic construct
atgctgtttaacctacgtattttgctcaacaatgcagcctttagaaacggacataactttatggttcgaaactttcgctgcgggcagccactgcagaacaaggtccagctgaaagggagagatttgctcacgctgaagaactttactggcgaagaaatcaagtatatgctgtggttgtccgcggacctcaagtttcggattaagcagaaaggggagtatctgccactgctgcaaggaaagagcctcggcatgatcttcgagaagcggagcactcggaccaggctgagtaccgaaactggcttcgcattgttgggtggacatccatgttttctgacaacgcaggacattcatctgggcgtgaacgagagtctgacggacacagctcgcgttctgtcctctatggctgatgcggtgttggcccgggtctataagcagtccgatttggacaccttggctaaggaagctagcataccgattatcaatgggctgtccgacctgtatcaccctattcaaatcctggccgactacctcacactgcaagaacactatagctcattgaagggactgaccctgagctggataggggacggaaacaacatcctacatagcattatgatgtccgctgccaagtttggcatgcatcttcaagccgccacgccaaagggttatgagcccgacgcgtcagtgacaaagctggccgagcagtacgctaaggagaatggtaccaaattactgctgactaatgatccactggaggctgcacatggcggcaatgtactgatcaccgacacatggatctcgatgggccaggaggaagaaaagaagaagaggcttcaggccttccaaggctaccaggtcaccatgaaaacagctaaggttgcagcatctgattggacctttctgcactgtctgccaaggaagcccgaagaggtggacgatgaagtattctatagcccacggagtttggtgttccctgaggctgaaaataggaagtggacaattatggccgtaatggtgtccctgttaaccgactactctccgcaactgcagaaacctaagttttag

SEQ ID NO: 131 - DNA, 1065 bp, Artificial Sequence
  Synthetic construct
atgctgtttaacttaaggatcctgctgaacaacgccgcttttcgtaacggtcataactttatggtccggaactttagatgtggccagccgctgcagaacaaggttcagctgaaggggagggatctgctgaccttgaagaactttaccggcgaagagatcaagtacatgttgtggctgagcgccgatctgaagtttaggattaagcagaagggggagtatttgccactgctgcaaggaaaatccttggggatgatcttcgagaagcgctccactagaacccggctaagcacagaaaccggcttcgcacttctgggtggacatccctgttttctgacgacgcaggatatacacctgggcgtgaatgagagtctgacggacacagctagggtgttgagcagcatggccgatgcagtactggcccgcgtttataagcagagcgacttggacacactggccaaggaagcgtcaattccgattatcaatgggctgtcagacctgtatcatcccattcaaatcttggctgactatctgaccctgcaagaacattacagctccctgaagggcctcacgttgtcctggattggcgacggaaacaacattctgcattcgatcatgatgagcgctgctaagtttggcatgcacctccaagccgctacacctaagggatatgagcctgatgccagcgtaaccaagctggccgaacagtacgcgaaggagaatggcacgaaactgctgttgacaaatgacccactggaggcagctcacggtggcaacgtgctgatcaccgacacgtggatatctatgggacaggaagaagagaagaagaagcggctgcaggcattccaagggtatcaggtcaccatgaaaacggccaaggttgctgcatccgactggacatttctgcattgcttgccccgcaaaccagaagaagtagacgacgaagtcttttattccccacggtcgctggtgttccccgaggcggagaatcgaaagtggacgattatggccgtgatggtgtccctgctgactgattactctccccaactgcaaaagcctaagttttag

SEQ ID NO: 132 - DNA, 1065 bp, Artificial Sequence
  Synthetic construct
atgcttttcaacctgaggatcctcctgaacaacgccgcctttcgcaatggtcacaactttatggtccggaacttcagatgcggccagccgctgcagaacaaggtccagctgaagggacgggatctgctgactctgaagaacttcaccggagaagagatcaagtacatgctgtggctgtcggccgacctgaagttcaggatcaagcagaagggagaatacctcccgctgctgcaaggaaagtccctgggcatgattttcgagaagcgctcgaccagaactcggttgtccaccgaaaccgggtttgcgctgctgggcggacatccttgcttcctgacgactcaggatattcacctgggagtgaacgagtcgctgaccgacaccgccagagtgctgagctcgatggccgacgccgtgttggcacgcgtgtacaagcagtccgatctggataccctggccaaagaagcttccatcccgatcattaacgggctgagcgacctctaccaccccattcaaatcctggccgactacctgactctgcaagaacactacagctcgctgaaggggttgactctgtcctggatcggcgacggaaacaacatcctgcactccatcatgatgtcggccgcaaagttcggcatgcatttgcaagccgccaccccaaagggctacgaaccagacgcgagcgtcaccaagctggccgaacagtacgcgaaggaaaatggtactaagctgctgctgaccaacgacccattggaagctgcccatggtggaaacgtgctgatcaccgacacctggatctcgatgggccaggaagaggagaagaagaagcggctgcaggcgttccaggggtatcaggtcaccatgaaaacagccaaagtggcagcgtcagactggaccttcctccactgtctgcctcgcaagccagaggaggtggacgacgaggtgttctactcccctcggtccctcgtgttccctgaggctgagaaccggaagtggaccattatggccgtgatggtgtcactcctgactgattactccccgcaactgcagaagcccaagttctag

SEQ ID NO: 133 - DNA, 1065 bp, Artificial Sequence
  Synthetic construct
atgctgtttaacctgaggatcctattgaacaatgctgcttttcgtaatggccataactttatggttcggaactttagatgcgggcagccactgcagaacaaggtccagttgaaaggccgcgatctgttgacattgaagaactttaccggcgaagagattaagtatatgctgtggctgtctgctgacctcaagtttcgaatcaagcagaagggcgaatatctccccctgctgcaaggaaagtctctcggcatgatctttgagaagcggagtacccgaacacggctgagcaccgaaacgggcttcgcactgctggggggccatccctgttttctgacaacgcaggacatccacttgggggttaacgaatcattgactgataccgcccgcgtactgtcatccatggccgacgctgtgctggctagggtgtacaagcagtcagatctggatacactggccaaggaagctagcataccaatcatcaatggactgagtgacctttatcacccgattcaaatactagccgattatctgaccctgcaagagcattactcctcgctgaaaggcctcacgctgtcctggatcggcgacggcaacaacattctgcatagtattatgatgtctgctgccaaattcggcatgcatctgcaagctgctacgccgaagggttatgaacccgacgcgtcagttacgaagctcgctgagcagtatgcaaaggagaatggcacaaagctgttgcttaccaacgatcccctggaagctgctcatggcggcaatgtgctgattactgacacctggatttcaatgggccaggaggaggagaagaagaagaggttacaggcttttcaaggttaccaagtcacgatgaaaaccgctaaggtcgcagccagcgactggacattcctgcactgtctgccaagaaagccggaagaagtggacgacgaggtgttctattccccgcggtctttggtgtttccggaggccgaaaacaggaaatggaccattatggccgtgatggtatcgttgctgacggactacagccctcagttgcaaaagcccaagttctag

SEQ ID NO: 134 - DNA, 1065 bp, Artificial Sequence
  Synthetic construct
atgctctttaacctccgcatcctcctcaacaacgccgccttccggaatgggcataacttcatggtccggaacttcagatgcggccagcccctgcaaaacaaggtccagttgaagggacgggacctccttacgctgaagaactttaccggagaagagattaagtacatgctgtggttgtccgctgacctcaagttccgcattaagcagaagggagaatatctgccgctgctgcaaggaaagagcctgggcatgatcttcgaaaagcgctccactagaacccggctgtcgactgagactggattcgccttgctcggtggacacccgtgcttcctgacgacccaggacatccacctgggagtgaacgagtcacttacggataccgcgagggtgctgtcctcaatggccgacgcagtgctcgcgcgcgtgtacaagcagtcagatctggataccctggccaaggaagccagcattcccatcatcaacggactgagcgacctttaccacccaatccagatcctcgccgactacttaaccctgcaagagcactacagctccctgaagggactgactctgtcctggatcggggatggaaacaacatcctgcactccatcatgatgtctgccgctaagtttgggatgcatctgcaagccgcaacccctaagggatacgagcccgacgcctcggtgaccaaacttgcggaacagtacgccaaggaaaacggtaccaagctgctgctgaccaacgaccctctggaagcggcccacggaggaaatgtgctgattaccgacacctggatttcgatgggccaggaggaggagaagaagaagagactgcaggcgttccagggatatcaggtcaccatgaaaaccgccaaggtcgccgccagcgactggaccttcctgcactgtctccctcggaaaccggaagaagtggatgacgaggtgttctactccccgcgctcgctggtgttcccggaggctgaaaacaggaagtggacaatcatggccgtgatggtgtccctgttgaccgactactccccacaactgcagaagcccaagttctag

SEQ ID NO: 135 - DNA, 1065 bp, Artificial Sequence
  Synthetic construct
atgcttttcaatctgcgcatcctcctgaacaacgccgccttccgcaatggacacaactttatggtccgcaacttccgctgtgggcagccgctgcagaacaaggtccagctcaaggggagagatctcctgaccctgaagaacttcactggagaggagatcaagtacatgctgtggctgtccgccgacctgaaatttcggattaagcagaagggcgaatacctcccactgctgcaaggaaagtctttgggcatgatcttcgaaaagagaagcacccggacccggttgagcaccgaaactgggttcgcgctcctcggtggacacccgtgcttcctgaccacccaagatattcatctgggtgtcaacgaaagcctgaccgacaccgccagggtgctgtcatccatggctgacgcagtgctcgcccgggtgtacaagcagtcagacctggacaccctcgccaaggaagcttcgatccctatcatcaacggactttccgacctgtaccaccccatccaaattctggccgactacctgactctgcaagaacactatagctcgctgaaaggacttactctgtcctggatcggggacggcaacaacattctccattccatcatgatgtccgctgccaagttcggaatgcaccttcaagcagcgactcccaagggatacgaacctgatgcctccgtgactaagctggcagagcagtacgccaaggagaacggtacaaagctgctgctcacgaacgaccccctggaggcggcccacggcggaaacgtgctgattaccgatacctggatctcaatgggccaggaagaggagaagaagaagcggctccaggcgtttcaaggctaccaggtcaccatgaaaaccgcgaaggtcgccgcctccgactggactttcttgcactgcctgccgcggaagcccgaggaagtggatgacgaagtgttctactcgccgagatcgttggtgttccctgaggccgaaaacaggaagtggaccatcatggccgtgatggtgtccctgctgactgattacagcccacagctgcagaagcctaagttctag

SEQ ID NO: 136 - DNA, 1065 bp, Artificial Sequence
  Synthetic construct
atgcttttcaatctccgcatcctccttaacaacgccgcgtttagaaacggccacaacttcatggtccggaacttcagatgtggccagccgcttcaaaacaaggtccagctgaagggccgggatcttctgaccctgaagaactttactggcgaagagatcaagtacatgctctggctctccgcggacttgaagttccgcattaagcagaagggggaataccttccgctgcttcaaggaaagagcctcggcatgatctttgagaagcgctcaaccaggacccgcctttctactgaaactgggttcgcgctgctcggtggccacccctgcttcctgacgacccaggacatccacctcggagtgaacgaatccctcaccgataccgcccgggtgttatcgagcatggcagatgccgtgctggccagggtgtacaaacagtccgatctggacactctggccaaggaggcgtcaattcctattatcaacggccttagtgacctctaccatccgattcagatcctggccgattacctcaccctgcaagaacactacagctccctgaagggtctgacattgtcctggatcggcgacggcaacaacattctccattccatcatgatgtccgccgcaaaattcggcatgcatcttcaagccgccacgccgaagggttacgagcccgacgcttccgtgactaagctcgccgagcagtacgctaaggagaacggaaccaagcttctgctgactaacgacccactagaagcagcccacgggggcaacgtgcttattactgacacctggatctccatgggccaggaagaagagaaaaagaagcggctgcaggcgttccagggatatcaggtcaccatgaaaaccgccaaggtcgctgcctccgactggaccttcctgcactgcctgcctcgcaagcctgaagaagtggacgacgaggtgttctactcgccacggagcctcgtgttccccgaggccgagaatagaaagtggaccatcatggccgtgatggtgtcactgctcaccgactacagcccgcagcttcagaagcccaagttctag

SEQ ID NO: 137 - DNA, 1065 bp, Artificial Sequence
  Synthetic construct
atgcttttcaacctgagaatcctcctgaacaacgccgccttccgcaatggtcataacttcatggtccgcaactttcgctgcggacagcctctccaaaacaaggtccagctcaaggggcgcgacctcctcacactgaagaacttcactggagaagaaatcaagtacatgctgtggctgagcgccgatctgaagttccggatcaagcagaagggagagtaccttcctctgctgcaagggaagtccttgggaatgattttcgagaagcggtccacccggaccaggctgagcactgaaactggcttcgccctgctgggaggccacccttgtttcctgaccactcaggacatccacctgggcgtgaacgagtccctgaccgatactgccagagtgctgtcctccatggccgacgccgtgctcgcccgggtgtacaagcagtcagacctcgatacgctggccaaggaagcctccattcccattatcaatggtctgtcggacctctaccatccaatccaaatcctcgccgactacctgactctgcaagaacactacagctcactcaagggcctcaccctctcctggatcggcgacggaaacaacatccttcactcgattatgatgtcggccgcgaagttcgggatgcacctccaagctgccactccaaaaggctacgagccggatgcctcagtgactaagttggcggaacagtatgcgaaggagaacggtaccaagctcctgctgactaacgacccgctggaggccgcccacgggggaaacgtgctcatcaccgatacttggatttccatgggacaggaggaagagaagaagaagcggttgcaggcatttcagggctaccaggtcaccatgaaaactgccaaagtcgccgccagcgactggaccttcctgcactgcctgccccgcaagcctgaagaagtggacgacgaggtgttctactctccccggtccctcgtgttccctgaggccgaaaacaggaagtggaccatcatggctgtgatggtgtccctcctgaccgactacagccctcagctccaaaaacccaagttttag

SEQ ID NO: 138 - DNA, 1065 bp, Artificial Sequence
  Synthetic construct
atgcttttcaacctgagaatcctcttgaacaatgctgcttttcggaatggccacaactttatggttcggaacttccgttgcggccagcctttacaaaacaaggtccagctgaagggccgggatttgctcacactgaagaactttactggggaggagattaagtatatgctgtggctgtccgctgacctgaagtttaggatcaagcagaagggcgaatatctgccgctgctgcaagggaaaagtctgggcatgatttttgaaaagcgctctacccggaccagactgtctacggaaacaggctttgccctgctgggcggccacccctgttttctgacaacgcaggacatccatctgggcgtgaacgaatcactgaccgatactgctcgggtactcagttctatggctgacgcagtgctggctagggtgtacaagcagagcgacttggacacactggctaaggaggccagcatccccattatcaatggcctgtctgatttgtaccatcccattcaaatcctggctgattatctgacactacaagagcattactcaagtctgaagggtttgactctctcctggatcggcgacggcaacaacattttacattccattatgatgagtgctgctaagtttggcatgcatttgcaagctgctaccccaaagggctatgaacctgacgctagcgtaaccaagttggccgaacagtatgctaaagagaatggcaccaagctgctcctgacgaatgaccccctggaagctgctcatggcggaaacgtacttataactgatacatggattagcatgggccaggaagaggagaagaagaagagactgcaggccttccaaggctatcaggtcaccatgaaaactgccaaggttgcagctagcgactggaccttcctgcactgtttgccgaggaaacccgaggaggtggacgatgaagtcttttattctccccgctccttggtgtttcccgaggctgaaaatcgaaagtggacgataatggcagtgatggtgtccctactgaccgactattctccacaactgcagaagcctaaattctag

SEQ ID NO: 139 - DNA, 1065 bp, Artificial Sequence
  Synthetic construct
atgcttttcaatctgaggatcctgctgaacaacgctgcttttcgcaacggtcataactttatggttcgcaattttcgttgtggccagccgctgcagaacaaggttcagctgaagggcagagatctgctgactctgaagaacttcactggggaagaaatcaagtatatgttatggctgtccgcggatctgaaatttcgaatcaagcagaagggcgaatatcttcccctgctgcaagggaaatccttgggcatgatttttgagaagaggagcactaggactagattgtcaacagaaacaggctttgctttgttgggcggacatccctgctttctgacgacacaggatatccacctcggcgtaaacgagtccctcaccgacactgctagggtactgagcagcatggccgacgctgtgctagcccgggtttacaagcagtcagacctggacacccttgccaaggaagcttctattccaattatcaacggcctgagtgacctgtatcaccctattcaaatactcgccgactatttgacgcttcaagaacattacagcagcctcaagggcttaaccttgagttggataggcgacggcaacaatatcctgcattccattatgatgtctgccgctaagtttggcatgcatctacaagccgcaacacccaagggctatgaacccgacgctagcgtgaccaagctggccgagcagtatgctaaggaaaatggcacaaagctccttcttaccaacgatcccctggaggctgctcacggcggcaacgtgctgattaccgatacatggattagcatgggccaggaggaggagaaaaagaagcggctccaggcttttcaaggctatcaggtcaccatgaaaactgcaaaggtcgctgcctccgactggactttcctgcattgtctaccccgcaagcctgaggaagtggacgatgaggtgttctactccccacggagtctggtgttcccggaagcagagaatcggaagtggaccatcatggctgtcatggtgtcgctcttgactgactattctccccaactgcaaaaacccaagttttag

SEQ ID NO: 140 - DNA, 1065 bp, Artificial Sequence; identical to SEQ ID NO: 139
  Synthetic construct

SEQ ID NO: 141 - DNA, 1065 bp, Artificial Sequence
  Synthetic construct
atgctttttaatctccgcatcctccttaacaacgccgcgtttagaaacggccacaacttcatggtccggaacttcagatgtggccagccgcttcaaaacaaggtccagctgaagggccgggatcttctgaccctgaagaactttactggcgaagagatcaagtacatgctctggctctccgcggacttgaagttccgcattaagcagaagggggaataccttccgctgcttcaaggaaagagcctcggcatgatctttgagaagcgctcaaccaggacccgcctttctactgaaactgggttcgcgctgctcggtggccacccctgcttcctgacgacccaggacatccacctcggagtgaacgaatccctcaccgataccgcccgggtgttatcgagcatggcagatgccgtgctggccagggtgtacaaacagtccgatctggacactctggccaaggaggcgtcaattcccatcatcaacggcctgagcgacctgtaccacccaatccaaatcctggctgactacctgaccctgcaagagcactacagcagcctgaagggtctgaccctgtcatggattggcgatggaaacaatattctgcactccatcatgatgtccgccgcgaagttcggaatgcatctgcaagccgccacgccaaaaggatacgaaccggatgcgtccgtgacgaagttggcggaacagtacgcgaaggagaacggaaccaagcttctgctgactaacgaccccctcgaggctgcgcatgggggcaacgtgctgattaccgacacctggatctccatggggcaggaggaagagaagaagaagagactgcaggcattccaggggtaccaggtcaccatgaaaaccgcaaaagtggcagcttcggactggactttcctgcattgcctgccgaggaagccggaggaagtcgacgacgaagtgttctactcgcctcggtccctggtgttccccgaggccgaaaaccggaagtggaccatcatggccgtgatggtgtccttgctgactgactatagcccgcagctgcagaagcctaagttctag

SEQ ID NO: 142 - DNA, 1065 bp, Artificial Sequence
  Synthetic construct
atgcttttcaacctgagaatcctcttgaacaatgctgcttttcggaatggccacaactttatggttcggaacttccgttgcggccagcctttacaaaacaaggtccagctgaagggccgggatttgctcacactgaagaactttactggagaagagatcaagtacatgctgtggctgtcggccgacctgaagttcaggatcaagcagaagggagaataccttccgctgcttcaaggaaagagcctcggcatgatctttgagaagcgctcaaccaggacccgcctttctactgaaactgggttcgcgctgctcggtggccacccctgcttcctgacgacccaggacatccacctcggagtgaacgaatccctcaccgataccgcccgggtgttatcgagcatggcagatgccgtgctggccagggtgtacaaacagtccgatctcgataccttggcaaaggaggcttccattcccatcatcaacggcctgagcgacctgtaccacccaatccaaatcctggctgactacctgaccctgcaagagcactacagcagcctgaagggtctgaccctgtcatggattggcgatggaaacaatattctgcactccatcatgatgtccgccgcgaagttcggaatgcatctgcaagccgccactccaaaaggatacgaaccggatgcgtccgtgaccaagttggcggaacagtacgcgaaggagaacggaaccaagcttctgctgactaacgaccccctcgaggctgcgcatgggggcaacgtgctgattaccgacacctggatctccatggggcaggaggaagagaagaagaagagactgcaggcattccaggggtaccaggtcaccatgaaaaccgcaaaagtggcagcttcggactggactttcctgcattgcctgccgaggaagccggaggaagtcgacgacgaagtgttctactcgcctcggtccctggtgttccccgaggccgaaaaccggaagtggaccatcatggccgtgatggtgtccttgctgactgactatagcccgcagctgcagaagcctaagttctag

SEQ ID NO: 143 - DNA, 1065 bp, Artificial Sequence
  Synthetic construct
atgcttttcaacctgagaatcctcttgaacaatgctgcttttcggaatggccacaactttatggttcggaacttccgttgcggccagcctttacaaaacaaggtccagctgaagggccgggatttgctcacactaaagaactttactggagaagagatcaagtacatgctatggctgtcggccgacctgaagttccgtatcaagcagaagggagaataccttccgctgcttcaaggaaagagcctcggcatgatctttgagaagcgctcaaccaggacccgcctttctactgaaactgggttcgcgctgctcggtggccacccctgcttcctgacgacccaggacatccacctcggagtgaacgaatccctcaccgataccgcccgggtgttatcgagcatggcagatgccgtgctggccagggtgtacaaacagtccgatctcgataccttggcaaaggaggcttccattcccatcatcaacggcctgagcgacctgtaccacccaatccaaatcctggctgactacctgaccctgcaagagcactacagcagcctgaagggtctgaccctgtcatggattggcgatggaaacaatattctgcactccatcatgatgtccgccgcgaagttcggaatgcatctgcaagccgccactccaaaaggatacgaaccggatgcatccgtgaccaagttggcggaacagtacgcgaaggagaacggaaccaagctcctgctgactaacgacccgctcgaggctgcgcatgggggtaacgtgctgattacggacacctggatctccatggggcaggaggaagagaagaagaagagactgcaggcattccaggggtaccaggtcaccatgaaaaccgcaaaagtggcagcttcggactggactttcctgcattgcctgccgaggaagccggaggaagtcgacgacgaagtgttctactcgcctcggtccctggtgttccccgaggccgaaaaccggaagtggaccatcatggccgtgatggtgtccttgctgactgactatagcccgcagctgcagaagcctaagttctag

SEQ ID NO: 144 - DNA, 1065 bp, Artificial Sequence
  Synthetic construct
atgcttttcaacctgagaatcctcttgaacaatgctgcttttcggaatggccacaactttatggttcggaacttccgttgcggccagcctttacaaaacaaggtccagctgaagggccgggatttgctcacactaaagaactttactggagaagagatcaagtacatgctatggctgtcggccgacctgaagttccgtatcaagcagaagggagaataccttccgctgcttcaaggaaagagcctcggcatgatctttgagaagcgctcaaccaggacccgcctttctactgaaactgggttcgcgctgctcggtggccacccctgcttcctgacgacccaggacatccacctcggagtgaacgaatccctcaccgataccgcccgggtgttatcgagcatggcagatgccgtgctggccagggtgtacaaacagtccgatctcgataccttggcaaaggaggcttccattcccatcatcaacggcctgagcgacctgtaccacccaatccaaatcctggctgactacctgaccctgcaagagcactacagcagcctgaagggtctgaccctgtcatggattggcgatggaaacaatattctgcactccatcatgatgtccgccgcgaagttcggaatgcatctgcaagccgccactccaaaaggatacgaaccggatgcgtccgtgaccaagttggcggaacagtacgcgaaggagaacggaaccaagcttctgctgactaacgaccccctcgaggctgcgcatgggggcaacgtgctgattaccgacacctggatctccatggggcaggaggaagagaagaagaagagactgcaggcattccaggggtaccaggtcaccatgaaaaccgcaaaagtggcagcttcggactggactttcctgcattgcctgccgaggaagccggaggaagtcgacgacgaagtgttctactcgcctcggtccctggtgttccccgaggccgaaaaccggaagtggaccatcatggccgtgatggtgtccttgctgactgactatagcccgcagctgcagaagcctaagttctag

SEQ ID NO: 145 - DNA, 1065 bp, Artificial Sequence
  Synthetic construct
atgctgttcaacctgcgaatcctgctgaacaacgccgcttttcggaacgggcacaactttatggtgaggaactttcgctgcggacagcccctccagaataaggtccagctgaagggcagggacctgctgaccctgaaaaatttcacaggggaggaaatcaagtatatgctgtggctgtcagctgatctgaagttccggatcaagcagaagggcgaatatctgcctctgctccagggcaaaagcctggggatgatcttcgaaaagcgcagtactcggaccagactgtcaaccgagactggattcgctctgctgggaggacacccttgttttctgaccactcaggacattcacctgggagtgaacgagtccctgaccgacactgctcgcgtcctgagctctatggccgacgctgtgctggctcgagtctacaaacagtccgacctggataccctggccaaggaagcttctatcccaattattaacggcctgtcagacctgtatcaccccatccagattctggccgattacctgaccctccaggagcactattctagtctgaaagggctgacactgagttggattggggacggaaacaatatcctgcactctattatgatgtcagccgccaagtttggaatgcacctccaggctgcaaccccaaaaggctacgaacccgatgcctcagtgacaaagctggctgaacagtacgccaaagagaacggcactaagctgctgctgaccaacgaccctctggaggccgctcacggaggcaacgtgctgatcaccgatacctggattagtatgggacaggaggaagagaagaagaagcggctccaggccttccagggctaccaggtgacaatgaaaaccgctaaggtcgcagccagcgattggacctttctgcactgcctgcccagaaagcccgaagaggtggacgacgaggtcttctactctcccagaagcctggtgtttcccgaagctgagaataggaagtggacaattatggcagtgatggtcagcctgctgactgattattcacctcagctccagaaaccaaagttctga

SEQ ID NO: 146 - DNA, 1065 bp, Artificial Sequence
  Synthetic construct
atgctgttcaacctgcgcatcctgctgaacaacgccgccttccgcaacggccacaacttcatggtgcgcaacttccgctgcggccagcccctgcagaacaaggtgcagctgaagggccgcgacctgctgaccctgaagaacttcaccggcgaggagatcaagtacatgctgtggctgagcgccgacctgaagttccgcatcaagcagaagggcgagtacctgcccctgctgcagggcaagagcctgggcatgatcttcgagaagcgcagcacccgcacccgcctgagcaccgagacaggcctggccctgctgggcggccacccctgcttcctgaccacccaggacatccacctgggcgtgaacgagagcctgaccgacaccgcccgcgtgctgagcagcatggccgacgccgtgctggcccgcgtgtacaagcagagcgacctggacaccctggccaaggaggccagcatccccatcatcaacggcctgagcgacctgtaccaccccatccagatcctggccgactacctgaccctgcaggagcactacagcagcctgaagggcctgaccctgagctggatcggcgacggcaacaacatcctgcacagcatcatgatgagcgccgccaagttcggcatgcacctgcaggccgccacccccaagggctacgagcccgacgccagcgtgaccaagctggccgagcagtacgccaaggagaacggcaccaagctgctgctgaccaacgaccccctggaggccgcccacggcggcaacgtgctgatcaccgacacctggatcagcatgggccaggaggaggagaagaagaagcgcctgcaggccttccagggctaccaggtgaccatgaagaccgccaaggtggccgccagcgactggaccttcctgcactgcctgccccgcaagcccgaggaggtggacgacgaggtgttctacagcccccgcagcctggtgttccccgaggccgagaaccgcaagtggaccatcatggccgtgatggtgagcctgctgaccgactacagcccccagctgcagaagcccaagttctga

SEQ ID NO: 147 - DNA, 1065 bp, Artificial Sequence
  Synthetic construct
atgctgttcaacctgcgaatcctgctgaacaacgccgcttttcggaacgggcacaactttatggtgaggaactttcgctgcggacagcccctccagaataaggtccagctgaagggcagggacctgctgaccctgaaaaatttcacaggggaggaaatcaagtatatgctgtggctgtcagctgatctgaagttccggatcaagcagaagggcgaatatctgcctctgctccagggcaaaagcctggggatgatcttcgaaaagcgcagtactcggaccagactgtcaaccgagactggattcgctctgctgggaggacacccttgttttctgaccactcaggacattcacctgggagtgaacgagtccctgaccgacactgctcgcgtcctgagctctatggccgacgctgtgctagctcgagtctacaaacagtccgacctggataccctggccaaggaagcttctatcccaattattaacggcctgtcagacctgtatcaccccatccagattctggccgattacctgaccctccaggagcactattctagtctgaaagggctgacactgagttggattggggacggaaacaatatcctgcactctattatgatgtcagccgccaagtttggaatgcacctccaggctgcaaccccaaaaggctacgaacccgatgcctcagtgacaaagctggctgaacagtacgccaaagagaacggcactaagctgctgctgaccaacgaccctctggaggccgctcacggaggcaacgtgctgatcaccgatacctggattagtatgggacaggaggaagagaagaagaagcggctccaggccttccagggctaccaggtgacaatgaaaaccgctaaggtcgcagccagcgattggacctttctgcactgcctgcccagaaagcccgaagaggtggacgacgaggtcttctactctcccagaagcctggtgtttcccgaagctgagaataggaagtggacaattatggcagtgatggtcagcctgctgactgattattcacctcagctccagaaaccaaagttctga

SEQ ID NO: 148 - DNA, 1065 bp, Artificial Sequence
  Synthetic construct
atgctgttcaacctgcgaatcctgctgaacaatgccgcttttcggaacgggcacaatttcatggtgaggaactttcgctgcggacagcccctccagaacaaggtccagctgaagggcagggacctgctgaccctgaaaaatttcacaggggaggaaatcaagtacatgctgtggctgtcagccgatctgaagttccggatcaagcagaagggcgaatatctgcctctgctccagggcaaaagcctggggatgatcttcgaaaagcgcagtactcggaccagactgtcaacagagactggattcgcactgctgggaggacacccatgttttctgaccacacaggacattcatctgggagtgaacgagtccctgaccgacacagcacgcgtcctgagctccatggctgatgcagtgctggctcgagtctacaaacagtctgacctggataccctggccaaggaagcttctatcccaatcattaatggcctgagtgacctgtatcaccccatccagattctggccgattacctgaccctccaggagcattattctagtctgaaagggctgacactgagctggattggggacggaaacaatatcctgcactccattatgatgagcgccgccaagtttggaatgcacctccaggctgcaaccccaaaaggctacgaacccgatgcctccgtgacaaagctggcagaacagtatgccaaagagaacggcactaagctgctgctgaccaatgaccctctggaggccgctcacggaggcaacgtgctgatcactgatacctggattagtatgggacaggaggaagagaagaagaagcggctccaggccttccagggctaccaggtgacaatgaaaactgctaaggtcgcagccagcgactggacctttctgcattgcctgcccagaaagcctgaagaggtggacgatgaggtcttctactcacccagaagcctggtgtttcctgaagctgagaataggaagtggacaatcatggcagtgatggtcagcctgctgactgattattcccctcagctccagaaaccaaagttctga

SEQ ID NO: 149 - DNA, 1065 bp, Artificial Sequence
  Synthetic construct
atgcttttcaaccttcgcattctcctcaacaacgccgcgtttagaaacggacacaacttcatggtccgcaacttccgctgcggacagccgctgcagaacaaggtccagctcaagggtcgggatctcctgacgctgaagaactttaccggcgaagagattaagtacatgctgtggctgtccgccgaccttaagttccggatcaagcagaagggcgaataccttcccctgctgcaaggaaagtccctgggcatgatcttcgagaagcgcagtaccagaaccagactctccactgaaaccgggttcgcgctgcttggcggccacccgtgtttcctcactacgcaagacatccatcttggcgtgaacgagtcccttaccgacaccgccagggtgctgtcaagcatggccgacgccgtccttgcgcgcgtgtacaagcagtcagaccttgatactctggccaaggaagcctccatccctattatcaacggcctatccgacctttaccacccgatccagatcctcgctgactacctgaccctgcaagaacactacagcagcctcaagggactgactctgtcctggatcggcgacgggaacaacatcctgcactcaatcatgatgagcgcagccaagttcggcatgcatctccaagccgctacacccaagggttatgaaccggacgcctctgtgaccaagttggcagaacagtacgccaaggagaacggtactaagctccttttaaccaacgaccccctcgaagcagcccatggcgggaatgtgctcattaccgatacctggatttcgatgggccaggaggaggagaagaagaagcggctgcaggcgttccagggctaccaggtcaccatgaaaactgccaaagtggccgcctcggattggacctttctccactgcctgcctcggaagcctgaggaggtggacgacgaagtgttctactccccacggtccctcgtgttccccgaggccgaaaataggaagtggaccatcatggccgtgatggtgtccctcttgaccgattacagcccgcagcttcagaagcctaaattctag

SEQ ID NO: 150 - DNA, 1065 bp, Artificial Sequence
  Synthetic construct
atgcttttcaatcttcgcatcctgttgaacaacgccgccttccgcaatggtcacaacttcatggtccggaacttcagatgtggacagcctctccaaaacaaggtccagctgaagggaagggacctcttaaccctcaaaaactttactggagaggagatcaagtacatgctgtggcttagcgccgaccttaagttccggatcaagcagaagggagagtacctcccgctgctgcaaggaaagagtcttggaatgatcttcgagaagcggtccaccagaactcgcctctccactgaaaccggattcgcactcctgggtggacacccgtgctttctgaccacccaagacatccacctcggagtgaacgagagcctcacggacaccgcgagagtgctgtcatccatggccgacgccgtgcttgcacgggtctacaagcagtccgatctggacactcttgccaaggaagcctccattcctatcattaacggtctgtcggatctgtaccacccgattcagatccttgcggactacctcacacttcaagaacactattcaagcctaaagggtctgaccctgtcctggatcggagatggaaacaacattctccattccatcatgatgagcgctgccaagttcggaatgcatctccaagcagcgactcctaagggttacgagccggacgcctcagtgactaagctggccgagcagtacgccaaggagaacggtaccaaactgttgcttactaacgacccgcttgaagcggcccatggaggaaacgtgctgattaccgacacctggatttcgatgggacaggaagaggagaagaagaagcggctccaggcgttccagggataccaggtcaccatgaaaacggccaaagtggccgctagcgattggacctttctgcactgcctcccgcgcaagcctgaagaagtggacgacgaagtgttctactcccctcgctctcttgtgttcccggaagccgaaaacaggaagtggaccatcatggccgtgatggtgtccctcctgaccgattacagcccgcagctgcagaagcctaagttctag

SEQ ID NO: 151 - DNA, 1065 bp, Artificial Sequence
  Synthetic construct
atgcttttcaatctccgcatcctcctcaacaacgccgcgtttagaaacggccacaacttcatggtccggaacttcagatgtggccagccgcttcagaacaaggtccagctcaagggccgggatcttctgaccctgaagaactttactggcgaagaaatcaagtacatgctctggctctccgccgacttgaagttccgcattaagcagaagggggaataccttccgctgctgcaaggaaagtcgctcggcatgatctttgagaagcgctcaacccgcaccaggctgtccactgaaaccgggttcgcgctgcttggtggccacccctgcttcctgaccacccaagacattcacctcggagtgaacgaatcgctcactgatactgcccgggtgctgtcgtcgatggccgatgcagtgctggccagggtgtacaaacagtccgatctggacactctggccaaggaggcgtccatccctattatcaacggcctttccgacctctaccacccgattcagatccttgccgattacctcaccctgcaagaacactactcgtcactgaagggtctgaccttgtcctggatcggcgacggcaacaacatcctccattccattatgatgtccgccgccaaattcggcatgcatcttcaagccgcaacccctaagggttacgagccggacgcttccgtgaccaagctcgccgagcagtacgctaaggagaacggaaccaagcttctgctgactaacgaccccctagaggcagcccacgggggcaacgtgcttattactgacacctggatctccatgggacaggaagaagagaagaagaagcggttacaggcgttccagggctatcaggtcaccatgaaaaccgccaaggtcgctgcctcggactggaccttcctgcattgcctgcctcgcaagcccgaagaagtggacgacgaggtgttctactcgccacggtcccttgtgttccctgaggccgagaatagaaagtggaccattatggccgtgatggtgtcccttctcaccgactactcgccgcaactgcagaaacccaagttctag

SEQ ID NO: 152 - DNA, 1065 bp, Artificial Sequence
  Synthetic construct
atgcttttcaatcttcgcatcctcctcaacaacgccgccttccggaacggtcacaacttcatggtccggaacttccgctgcggccagccgctccaaaacaaagtgcagcttaagggccgcgatctcctgaccctgaagaacttcaccggagaggaaatcaagtacatgctgtggctctcggcggacctgaagtttaggattaagcagaagggggagtatctgccgctgctccaagggaagtcccttggcatgatcttcgaaaagaggtccacccggactcggctcagcaccgaaacaggttttgcacttctggggggccacccgtgcttcctgacgacccaggacatccatctgggtgtcaacgagagtttgaccgacactgccagagtgctgtcatccatggcggacgcggtgctcgcgagagtgtacaagcagtccgatcttgacaccctggcaaaagaggcttcaatcccgatcattaacggactctcggatctgtaccaccctatccaaatcttggccgactacctgaccctgcaagaacactacagctccctgaagggcctgactctttcctggattggcgatggaaacaacattctccattctattatgatgtccgccgccaagttcggcatgcaccttcaagccgccaccccgaagggctacgaacctgacgcctccgtgactaagctagccgaacagtacgctaaggagaacggcactaagcttctccttaccaacgatccgctggaggcggcccatggcggaaatgtgcttatcaccgacacctggattagcatggggcaggaagaagagaagaagaaacggctccaggcattccagggctaccaggtcaccatgaaaactgccaaggtcgccgctagcgactggaccttcctccactgtctgcctcgcaagcctgaagaagtggacgacgaggtgttctactccccgcgctccctcgtgtttcctgaggccgagaacagaaagtggaccatcatggccgtgatggtgtcattacttacggactacagcccgcagctgcagaagccgaagttctag

SEQ ID NO: 153 - DNA, 1065 bp, Artificial Sequence
  Synthetic construct
atgctttttaacttgagaatccttctgaacaacgccgctttccgcaacggtcataacttcatggtccggaacttcagatgtggccagcccctccaaaacaaagtgcagctgaagggccgggaccttcttacgctgaagaatttcaccggcgaagaaatcaagtacatgctctggctgtccgccgatcttaagttccgcattaagcagaagggggaatacctcccgctgctgcaagggaagtcgctgggcatgatttttgagaagcggtcaactcgcacccgcctgtccactgaaactggattcgcactgctcggtggccatccctgcttcctgaccacccaagacatccacctcggcgtgaacgagtccctgactgacaccgcccgggtcttatcctcgatggccgatgctgtgcttgcgagggtgtacaagcagtccgacctcgacacactcgcgaaggaggcctccatccccatcatcaacggcctgtccgacctttaccacccaattcagatcctcgccgattacctgaccctgcaagagcactactcgtcgctcaaggggcttaccctctcgtggattggcgacggcaacaacatccttcactccatcatgatgtcggcagcgaagttcggcatgcatctgcaagccgccacgcctaagggttatgaaccggatgcctcagtgaccaagctcgccgaacagtacgcgaaagagaatggaaccaagctacttctgaccaacgaccccctggaggccgctcacggcggcaacgtcctcattaccgatacttggatttcgatgggacaggaagaggaaaagaagaagagactgcaggcgttccagggataccaggtcaccatgaaaactgccaaagtggcagcctccgactggaccttccttcactgcctgccgaggaagcctgaagaggtggacgacgaggtgttctactccccgcgctccttggtgtttcctgaggccgaaaaccggaagtggactatcatggccgtgatggtgtccctcctcaccgactactcgccgcaactgcagaagcctaagttctag

SEQ ID NO: 154 - DNA, 1065 bp, Artificial Sequence
  Synthetic construct
atgttattcaaccttagaattctccttaacaacgccgccttccggaatgggcataactttatggtccgcaatttccgctgtggacagcctctgcaaaacaaggtccagctcaagggccgggatctgctgactctcaagaacttcactggggaagaaatcaagtacatgctctggctgagcgccgacctcaagttccgcatcaagcagaagggagagtacctcccgctgctccaagggaagtccctgggcatgatcttcgagaagagatccacccgcaccagactttccactgagactggcttcgccttgctgggaggccacccatgcttcctgacgacccaggacattcaccttggcgtgaacgagtccctgactgacaccgcaagggtgttgtcctcgatggccgacgccgtgcttgcccgggtgtacaagcagagcgatcttgacaccctggctaaggaagcttccattcccatcatcaacggtctgagcgacctgtaccacccgattcagatcctggcggactacctaaccctgcaagagcactatagctccctgaagggcctcacactttcatggatcggcgacggcaacaacatcctgcactctattatgatgagcgctgccaaattcggcatgcacctccaagccgccacgcctaaaggctacgagcccgacgcctcggtgaccaagcttgcggagcagtacgcgaaggaaaacggcaccaagctgcttctcaccaacgatcctctggaagcggcccatggtggcaacgtgctcattaccgacacttggatctccatgggacaggaggaggaaaagaagaagcggctccaggcgtttcagggttaccaggtcaccatgaaaaccgccaaggtcgcagcctccgactggaccttccttcattgccttccgcgcaagcccgaagaagtggacgatgaagtgttttactcacctcggtcactcgtgttcccggaagcagagaacaggaaatggaccattatggccgtgatggtgtccctgctcaccgattacagtccgcaactgcagaagcccaagttctag

SEQ ID NO: 155 - DNA, 1065 bp, Artificial Sequence
  Synthetic construct
atgcttttcaatctccgcatcctccttaacaacgccgcgtttagaaacggccacaacttcatggtccggaacttcagatgtggccagccgcttcaaaacaaggtccagctgaagggccgggatcttctgaccctgaagaactttactggcgaagagatcaagtacatgctctggctctccgcggacttgaagttccgcattaagcagaagggggaataccttccgctgcttcaaggaaagagcctcggcatgatctttgagaagcgctcaaccaggacccgcctttctactgaaactgggttcgcgctgctcggtggccacccctgcttcctgacgacccaggacatccacctcggagtgaacgaatccctcaccgataccgcccgggtgttatcgagcatggcagatgccgtgctggccagggtgtacaaacagtccgatctggacactctggccaaggaggcgtcaattcctattatcaacggccttagtgacctctaccatccgattcaaatcctggccgattacctcaccctgcaagaacactacagctccctgaagggtctgacattgtcctggatcggcgacggcaacaacattctccattccatcatgatgtccgccgcaaaattcggcatgcatcttcaagccgccacgcctaagggttacgaacccgacgcttccgtgactaagctcgccgagcagtacgctaaggagaacggaaccaagctgctgctgactaacgacccgctagaagcagcccacgggggcaacgtgcttattactgacacctggatctccatgggccaggaggaagagaaaaagaagcggctgcaggcgttccagggatatcaggtcaccatgaaaaccgccaaggtcgctgcctccgactggaccttcctgcactgcctgcctcgcaagcctgaagaagtggacgacgaggtgttctactcgccacggagcctcgtgttccccgaggccgagaatagaaagtggaccatcatggccgtgatggtgtcacttctcaccgactacagcccgcagcttcagaagcccaagttctag

SEQ ID NO: 156 - DNA, 1065 bp, Artificial Sequence
  Synthetic construct
atgcttttcaatctccgcatcctccttaacaacgccgcgtttagaaacggccacaacttcatggtccggaacttcagatgtggccagccgcttcaaaacaaggtccagcttaagggccgggatctcctcacccttaaaaacttcaccggcgaagagatcaagtacatgctctggctctccgcggaccttaagttccgcattaagcagaagggggaataccttccgctgcttcaaggaaagagcctcggcatgatctttgagaagcgctcaaccaggaccaggctttctactgaaactgggttcgcgcttctcggcggtcatccctgcttcctcacgacccaagacatccacctcggagtgaacgaatccctcacggatactgcccgcgtgctttcgagcatggcagacgccgtgctcgcccgggtgtacaaacagtccgatctcgacactctcgccaaggaggcgtcaattcctattatcaacggtcttagtgacctttaccacccgatccagatcctcgccgattacctcacactccaagaacactacagctcccttaagggtcttaccctctcctggatcggcgacggcaacaacattctccactccatcatgatgtccgccgcaaagttcggcatgcatcttcaagccgccaccccgaagggctacgagcctgatgcttccgtgactaagctcgccgagcagtacgctaaggagaacggaaccaagcttcttctcactaacgacccactcgaagcagcccatgggggcaacgtgcttatcactgacacctggatctccatgggccaggaagaagagaagaagaagcggctccaggcgttccagggatatcaggtcaccatgaaaaccgccaaggtcgctgcctccgactggacctttctccactgcctccctcgcaaacctgaagaagtggacgacgaggtgttctactcgccccggagcctcgtgttccccgaggccgagaatagaaagtggaccattatggccgtgatggtgtcactcctcaccgactacagcccgcagcttcagaagcccaagttctag

SEQ ID NO: 157 - DNA, 1065 bp, Artificial Sequence
  Synthetic construct
atgcttttcaatctccgcatcctccttaacaacgccgcgtttagaaacggacataacttcatggtccggaacttcagatgtggacagccgcttcaaaacaaggtccagctgaagggtcgggatcttctgaccctgaagaactttaccggagaagagatcaagtacatgctctggctctccgcggacttgaagttccgcattaagcagaagggagaatacctcccgctgcttcaaggaaagagcctcggaatgatttttgagaagcgctcaaccaggacccgcctttctactgaaactggattcgcgctgctgggtggacacccctgcttcctgacgacccaggacatccacctcggagtgaacgaatccctcactgataccgcccgggtgttatcgagcatggcagatgccgtgctggccagggtgtacaaacagtccgatctggacactctggccaaggaggcgtcaattcctatcatcaacggacttagtgacctctaccatccgattcaaatcctggccgactacctcaccctgcaagaacactacagctccctgaagggtctgacattgtcctggatcggagatggaaacaacattctccactccatcatgatgtccgccgcaaaattcggaatgcatcttcaagccgccacgcctaagggttacgaacccgacgcttccgtgactaagctcgccgagcagtacgctaaggagaacggtaccaagcttctcctgaccaacgacccactagaagcagcccacggtggaaacgtgcttattactgacacttggatctccatgggacaggaggaagagaaaaagaagcggctgcaggcgttccagggatatcaggtcaccatgaaaaccgccaaggtcgctgcctccgactggaccttcctgcactgcctgcctcgcaagcctgaagaagtggacgacgaggtgttctactcgccgcggagcctcgtgttccccgaggccgagaatagaaagtggaccatcatggccgtgatggtgtcactgctcaccgactacagcccgcagcttcagaagcccaagttctag

SEQ ID NO: 158 - DNA, 1065 bp, Artificial Sequence
  Synthetic construct
atgcttttcaacctccgcattctcctcaacaacgctgccttccggaatggacataacttcatggtccggaacttcagatgcggacagccgcttcagaacaaggtccagcttaaggggagagatctccttaccctcaaaaacttcactggcgaagaaatcaagtacatgctctggcttagtgcggatctcaagttccgcatcaagcagaagggagaatacctcccgctccttcaaggaaagagcctcggcatgatttttgagaagaggtccaccagaactcgcctttcaaccgagactgggttcgccctgcttggcggtcacccctgcttcctcactacccaagacatccacctcggcgtgaacgagagccttaccgacaccgcccgcgtgctctcctcaatggccgacgctgtgctcgcccgggtgtacaagcagtccgaccttgatactctcgccaaggaggcctccatcccaattatcaacgggctctctgatctctaccaccctatccaaatcctcgcggactacctcaccctccaagagcactatagctcgctcaagggcctcaccctttcctggattggcgacggcaacaacattcttcactcgatcatgatgtccgccgccaagttcggcatgcatctccaagccgcgacccccaagggctacgagcctgacgcatccgtgaccaagctcgccgagcagtacgcgaaggaaaatggcaccaagcttcttctcaccaacgacccccttgaggccgctcatggcggcaacgtgctcatcactgacacttggatcagcatgggccaggaggaggaaaagaagaagcgccttcaggcattccagggttaccaggtcaccatgaaaaccgccaaagtggccgcctccgactggacctttcttcactgtctcccgcggaagcctgaagaagtggatgacgaagtgttttactcccctcggtcactcgtgttcccggaagcagaaaacaggaagtggaccattatggcggtcatggtgtccctcctcaccgactacagcccgcagcttcagaaacccaagttctag

SEQ ID NO: 159 - DNA, 1065 bp, Artificial Sequence
  Synthetic construct
atgcttttcaatctccgcatcctccttaacaacgcagcgtttagaaacggtcacaacttcatggtccggaacttccgctgtggacagccgcttcaaaacaaggtccagctgaagggtcgggaccttctgaccctgaagaactttactggagaagagatcaagtacatgctttggctgtccgcggacttgaagttccgcattaagcagaagggagaataccttccgctgctccaaggaaagagcctgggaatgatctttgagaagcgctcaaccaggacccgcctttctactgaaactggattcgcgctgctgggtggtcacccttgcttcctgacgacccaggacattcacctcggagtgaacgagtccctcactgataccgccagagtgttatcgagcatggcagatgccgtgctggctagggtgtacaaacagtccgatctggacaccctggccaaggaggcatcaattcctattatcaacggacttagtgacctctaccatccgattcaaatcctggccgattacctcaccctgcaagaacactacagctccctgaagggtctgacattgtcctggatcggagatggaaacaacattctccattccatcatgatgtccgcggccaagttcggaatgcatctccaagccgccacgccgaaaggatacgagccggacgcttccgtgactaagctcgccgagcagtacgctaaggagaacggaaccaagcttctgctgactaacgacccgctagaagccgcccacggtggaaacgtgcttattactgacacctggatctccatgggacaggaagaagagaaaaagaagcggctgcaggcgttccagggatatcaggtcaccatgaaaaccgccaaggtcgccgcctccgactggaccttccttcactgcctgcctcggaagcctgaagaagtggacgacgaggtgttctactcgccgcggagcctcgtgttccctgaggccgagaatagaaagtggaccatcatggccgtgatggtgtcactcctcaccgactacagcccgcagcttcagaagcctaagttctag

SEQ ID NO: 160 - DNA, 1065 bp, Artificial Sequence
  Synthetic construct
atgcttttcaatctccgcattctcctcaacaacgcagcctttagaaacggccacaacttcatggtccggaacttcagatgtggccagccgcttcagaacaaggtccagctcaagggccgggacctcctcaccctcaaaaactttaccggcgaagagatcaagtacatgctctggctttcggccgaccttaagttccgcatcaagcagaagggggaataccttccgctgcttcaaggaaagtccctcggcatgatctttgaaaagcgctcgaccaggacccgcctttccactgaaaccgggttcgcgcttctcggtggccacccctgcttcctcaccacccaagacattcacctcggagtgaacgaatcccttaccgataccgcaagagtgctttcgtcgatggccgatgccgtgcttgcgcgggtgtacaagcagtcagatctcgacactctcgccaaggaggcgtccattcctattatcaacggcctttccgacctttaccacccgattcagatcctcgccgattacctcaccctgcaagagcactactcgtcactcaagggtcttaccctctcctggatcggcgacggaaacaacatcctccattcgatcatgatgtccgccgccaaattcggcatgcacctccaagccgcgaccccgaagggttacgagcccgacgcttccgtgaccaagctcgccgaacagtacgctaaggaaaacggcaccaagctcctcctcactaacgaccctctcgaagcagcccatgggggcaacgtgctcattactgacacttggatctcgatgggccaggaagaggagaaaaagaagcggcttcaggcgttccagggatatcaggtcaccatgaaaaccgccaaggtcgctgcctcggactggaccttccttcactgccttccgcgcaagcctgaagaggtggacgatgaggtgttctactccccacggtcccttgtgttccccgaggccgagaataggaagtggaccatcatggccgtgatggtgtcgctcctcactgactactccccgcaacttcagaagcctaagttctag

SEQ ID NO: 161 - DNA, 1065 bp, Artificial Sequence
  Synthetic construct
atgctgtttaatctgagaatacttctaaacaacgccgccttccggaatggccataactttatggttcggaatttccgctgcggccagccgctgcagaacaaggtccagctgaagggaagagacttgctgaccctcaagaacttcaccggagaagaaatcaagtatatgctgtggctgtccgccgacctgaaattccgcatcaagcagaagggcgaatatctgccgctgttgcaagggaagtccctggggatgatcttcgagaagaggtccaccagaacacggctttcaaccgaaaccgggtttgcactgctgggtggacacccctgttttctgaccactcaagatatccacctgggcgtgaacgagtcccttaccgacactgctagggtgttgtccagcatggccgatgccgtcctggctcgcgtgtacaagcagtccgacctggataccctggcaaaggaagcgtccattcccattatcaacgggctgtccgacctgtaccatccgattcaaatcctggcggactacctgactctgcaagagcattacagcagcttgaaggggcttactctctcgtggatcggcgacgggaacaacatcctgcactccatcatgatgtccgccgccaagttcgggatgcatttgcaagctgcgaccccgaaaggttacgagcccgatgctagcgtaactaagcttgccgaacagtacgccaaagagaatggtacaaaactgcttctgactaacgacccgctggaagcagcccacggcgggaacgtgctgataaccgacacctggatttcaatggggcaggaggaagagaagaagaagcgactgcaggcgttccaaggctatcaggttaccatgaaaaccgccaaagtggcagccagcgattggactttcctgcactgtctgccgcggaagcccgaggaagttgatgacgaagtattctactcaccccggagcctcgtgttccccgaggccgaaaaccggaagtggactattatggccgtgatggtgtcgctgttgaccgactacagcccgcaactgcagaagccgaagttttag

SEQ ID NO: 162 - DNA, 1065 bp, Artificial Sequence
  Synthetic construct
atgcttttcaacctgaggatccttttgaacaacgccgcctttcgcaacggccacaactttatggtccgcaatttccgctgcgggcagccgctgcagaacaaggtccagctgaagggccgggatctgctgaccctgaagaacttcaccggggaggaaatcaagtacatgctttggctctccgccgatctgaagttcagaatcaagcagaagggagagtacctcccgttgctgcaaggaaagtcactcggaatgattttcgaaaagagaagcactaggacccgcctctcaactgaaaccgggttcgcgctgctcgggggccatccgtgtttcctgactacccaagacatccacctgggagtgaacgagtcgctgaccgacaccgcacgcgtgctgtcatccatggcggacgcagtgcttgcccgggtgtacaagcagtcggacctggacactcttgccaaggaggcatcaatccccatcattaacggactgtccgatctctaccacccgattcagatcctggctgactacctaaccctgcaagagcactactcaagcctgaaggggctgaccctgtcgtggatcggggacggcaacaacattctgcactccatcatgatgtcggcggctaagttcgggatgcatttgcaagcggcaactccgaagggttatgaacccgacgcctccgtgaccaagctggccgaacagtacgccaaggaaaacggaaccaagttgctgctgactaatgatcccctggaggcggcccacggggggaacgtgctgataaccgatacctggatctccatggggcaggaagaagagaagaaaaagcggctgcaggcattccagggataccaggtcaccatgaaaaccgcaaaagtggcagccagcgactggactttcctccattgcctgccgcgaaagccggaggaggtcgatgacgaggtgttctactccccgcggtcgctggtgttcccggaggcggaaaaccggaagtggaccattatggccgtgatggtgtcactcctgactgactacagcccgcaactgcagaagccgaagttctag

SEQ ID NO: 163 - DNA, 1074 bp, Artificial Sequence
  Synthetic construct
atgcttttcaatctccgcatcctccttaacaacgccgcgtttagaaacggccacaacttcatggtccggaacttcagatgtggccagccgcttcaaaacaaggtccagctgaagggccgggatcttctgaccctgaagaactttactggcgaagagatcaagtacatgctctggctctccgcggacttgaagttccgcattaagcagaagggggaataccttccgctgcttcaaggaaagagcctcggcatgatctttgagaagcgctcaaccaggacccgcctttctactgaaactgggttcgcgctgctcggtggccacccctgcttcctgacgacccaggacatccacctcggagtgaacgaatccctcaccgataccgcccgggtgttatcgagcatggcagatgccgtgctggccagggtgtacaaacagtccgatctggacactctggccaaggaggcgtcaattcctattatcaacggccttagtgacctctaccatccgattcagatcctggccgattacctcaccctgcaagaacactacagctccctgaagggtctgacattgtcctggatcggcgacggcaacaacattctccattccatcatgatgtccgccgcaaaattcggcatgcatcttcaagccgccacgccgaagggttacgagcccgacgcttccgtgactaagctcgccgagcagtacgctaaggagaacggaaccaagcttctgctgactaacgacccactagaagcagcccacgggggcaacgtgcttattactgacacctggatctccatgggccaggaagaagagaaaaagaagcggctgcaggcgttccagggatatcaggtcaccatgaaaaccgccaaggtcgctgcctccgactggaccttcctgcactgcctgcctcgcaagcctgaagaagtggacgacgaggtgttctactcgccacggagcctcgtgttccccgaggccgagaatagaaagtggaccatcatggccgtgatggtgtcactgctcaccgactacagcccgcagcttcagaagcccaagttctagataagtgaa

SEQ ID NO: 164 - DNA, 1073 bp, Artificial Sequence
  Synthetic construct
atgctgttcaacctgcgcatcctgctgaacaacgccgccttccgcaacggccacaacttcatggtgcgcaacttccgctgcggccagcccctgcagaacaaggtgcagctgaagggccgcgacctgctgaccctgaagaacttcaccggcgaggagatcaagtacatgctgtggctgagcgccgacctgaagttccgcatcaagcagaagggcgagtacctgcccctgctgcagggcaagagcctgggcatgatcttcgagaagcgcagcacccgcacccgcctgagcaccgagacaggcctggccctgctgggcggccacccctgcttcctgaccacccaggacatccacctgggcgtgaacgagagcctgaccgacaccgcccgcgtgctgagcagcatggccgacgccgtgctggcccgcgtgtacaagcagagcgacctggacaccctggccaaggaggccagcatccccatcatcaacggcctgagcgacctgtaccaccccatccagatcctggccgactacctgaccctgcaggagcactacagcagcctgaagggcctgaccctgagctggatcggcgacggcaacaacatcctgcacagcatcatgatgagcgccgccaagttcggcatgcacctgcaggccgccacccccaagggctacgagcccgacgccagcgtgaccaagctggccgagcagtacgccaaggagaacggcaccaagctgctgctgaccaacgaccccctggaggccgcccacggcggcaacgtgctgatcaccgacacctggatcagcatgggccaggaggaggagaagaagaagcgcctgcaggccttccagggctaccaggtgaccatgaagaccgccaaggtggccgccagcgactggaccttcctgcactgcctgccccgcaagcccgaggaggtggacgacgaggtgttctacagcccccgcagcctggtgttccccgaggccgagaaccgcaagtggaccatcatggccgtgatggtgagcctgctgaccgactacagcccccagctgcagaagcccaagttctgaataagtga

SEQ ID NO: 165 - DNA, 1073 bp, Artificial Sequence; identical to SEQ ID NO: 164
  Synthetic construct

SEQ ID NO: 166 - DNA, 1074 bp, Artificial Sequence; identical to SEQ ID NO: 163
  Synthetic construct

SEQ ID NO: 167 - DNA, 1073 bp, Artificial Sequence
  Synthetic construct
atgcttttcaacctgagaatcctcttgaacaatgctgcttttcggaatggccacaactttatggttcggaacttccgttgcggccagcctttacaaaacaaggtccagctgaagggccgggatttgctcacactaaagaactttactggagaagagatcaagtacatgctatggctgtcggccgacctgaagttccgtatcaagcagaagggagaataccttccgctgcttcaaggaaagagcctcggcatgatctttgagaagcgctcaaccaggacccgcctttctactgaaactgggttcgcgctgctcggtggccacccctgcttcctgacgacccaggacatccacctcggagtgaacgaatccctcaccgataccgcccgggtgttatcgagcatggcagatgccgtgctggccagggtgtacaaacagtccgatctcgataccttggcaaaggaggcttccattcccatcatcaacggcctgagcgacctgtaccacccaatccaaatcctggctgactacctgaccctgcaagagcactacagcagcctgaagggtctgaccctgtcatggattggcgatggaaacaatattctgcactccatcatgatgtccgccgcgaagttcggaatgcatctgcaagccgccactccaaaaggatacgaaccggatgcatccgtgaccaagttggcggaacagtacgcgaaggagaacggaaccaagctcctgctgactaacgacccgctcgaggctgcgcatgggggtaacgtgctgattacggacacctggatctccatggggcaggaggaagagaagaagaagagactgcaggcattccaggggtaccaggtcaccatgaaaaccgcaaaagtggcagcttcggactggactttcctgcattgcctgccgaggaagccggaggaagtcgacgacgaagtgttctactcgcctcggtccctggtgttccccgaggccgaaaaccggaagtggaccatcatggccgtgatggtgtccttgctgactgactatagcccgcagctgcagaagcctaagttctagataagtga

SEQ ID NO: 168 - DNA, 1073 bp, Artificial Sequence; identical to SEQ ID NO: 164
  Synthetic construct

SEQ ID NO: 169 - DNA, 1074 bp, Artificial Sequence; identical to SEQ ID NO: 163
  Synthetic construct

SEQ ID NO: 170 - DNA, 1073 bp, Artificial Sequence; identical to SEQ ID NO: 164
  Synthetic construct

SEQ ID NO: 171 - DNA, 1073 bp, Artificial Sequence; identical to SEQ ID NO: 167
  Synthetic construct

SEQ ID NO: 172 - DNA, 1074 bp, Artificial Sequence; identical to SEQ ID NO: 163
  Synthetic construct

SEQ ID NO: 173 - DNA, 1073 bp, Artificial Sequence; identical to SEQ ID NO: 164
  Synthetic construct

SEQ ID NO: 174 - DNA, 1073 bp, Artificial Sequence; identical to SEQ ID NO: 167
  Synthetic construct

SEQ ID NO: 175 - DNA, 1065 bp, Artificial Sequence
  Synthetic construct
atgctgttcaacctgcgcatcctgctgaacaacgccgccttccgcaacggccacaacttcatggtgcgcaacttccgctgcggccagcccctgcagaacaaggtgcagctgaagggccgcgacctgctgaccctgaagaacttcaccggcgaggagatcaagtacatgctgtggctgagcgccgacctgaagttccgcatcaagcagaagggcgagtacctgcccctgctgcagggcaagagcctgggcatgatcttcgagaagcgcagcacccgcacccgcctgagcaccgagacaggcttcgccctgctgggcggccacccctgcttcctgaccacccaggacatccacctgggcgtgaacgagagcctgaccgacaccgcccgcgtgctgagcagcatggccgacgccgtgctggcccgcgtgtacaagcagagcgacctggacaccctggccaaggaggccagcatccccatcatcaacggcctgagcgacctgtaccaccccatccagatcctggccgactacctgaccctgcaggagcactacagcagcctgaagggcctgaccctgagctggatcggcgacggcaacaacatcctgcacagcatcatgatgagcgccgccaagttcggcatgcacctgcaggccgccacccccaagggctacgagcccgacgccagcgtgaccaagctggccgagcagtacgccaaggagaacggcaccaagctgctgctgaccaacgaccccctggaggccgcccacggcggcaacgtgctgatcaccgacacctggatcagcatgggccaggaggaggagaagaagaagcgcctgcaggccttccagggctaccaggtgaccatgaagaccgccaaggtggccgccagcgactggaccttcctgcactgcctgccccgcaagcccgaggaggtggacgacgaggtgttctacagcccccgcagcctggtgttccccgaggccgagaaccgcaagtggaccatcatggccgtgatggtgagcctgctgaccgactacagcccccagctgcagaagcccaagttctga

SEQ ID NO: 176 - DNA, 1065 bp, Artificial Sequence; identical to SEQ ID NO: 175
  Synthetic construct

SEQ ID NO: 177 - DNA, 1065 bp, Artificial Sequence; identical to SEQ ID NO: 175
  Synthetic construct

SEQ ID NO: 178 - DNA, 1074 bp, Artificial Sequence
  Synthetic construct
atgctgttcaacctgcgcatcctgctgaacaacgccgccttccgcaacggccacaacttcatggtgcgcaacttccgctgcggccagcccctgcagaacaaggtgcagctgaagggccgcgacctgctgaccctgaagaacttcaccggcgaggagatcaagtacatgctgtggctgagcgccgacctgaagttccgcatcaagcagaagggcgagtacctgcccctgctgcagggcaagagcctgggcatgatcttcgagaagcgcagcacccgcacccgcctgagcaccgagacaggcttcgccctgctgggcggccacccctgcttcctgaccacccaggacatccacctgggcgtgaacgagagcctgaccgacaccgcccgcgtgctgagcagcatggccgacgccgtgctggcccgcgtgtacaagcagagcgacctggacaccctggccaaggaggccagcatccccatcatcaacggcctgagcgacctgtaccaccccatccagatcctggccgactacctgaccctgcaggagcactacagcagcctgaagggcctgaccctgagctggatcggcgacggcaacaacatcctgcacagcatcatgatgagcgccgccaagttcggcatgcacctgcaggccgccacccccaagggctacgagcccgacgccagcgtgaccaagctggccgagcagtacgccaaggagaacggcaccaagctgctgctgaccaacgaccccctggaggccgcccacggcggcaacgtgctgatcaccgacacctggatcagcatgggccaggaggaggagaagaagaagcgcctgcaggccttccagggctaccaggtgaccatgaagaccgccaaggtggccgccagcgactggaccttcctgcactgcctgccccgcaagcccgaggaggtggacgacgaggtgttctacagcccccgcagcctggtgttccccgaggccgagaaccgcaagtggaccatcatggccgtgatggtgagcctgctgaccgactacagcccccagctgcagaagcccaagttctgaataagtgaa

SEQ ID NO: 179 - DNA, 1077 bp, Artificial Sequence
  Synthetic construct
atgggcgtcttcaacctgcggatcctgctgaacaacgccgccttccggaacggccacaacttcatggtccgcaacttcagatgcggccagcccctgcagaacaaggtgcagctgaagggccgggacctgctgaccctgaagaacttcaccggcgaagagatcaagtacatgctgtggctgagcgccgacctgaagttccggatcaagcagaagggcgagtacctgcccctgctgcaaggcaagagcctgggcatgatcttcgagaagcggagcacccggacccggctgagcaccgagacaggctttgccctgctgggaggccacccctgctttctgaccacccaggacatccacctgggcgtgaacgagagcctgaccgacaccgccagagtgctgagcagcatggccgacgccgtgctggcccgggtgtacaagcagagcgacctggacaccctggccaaagaggccagcatccccatcatcaacggcctgagcgacctgtaccaccccatccagatcctggccgactacctgaccctgcaggaacactacagctccctgaagggcctgaccctgagctggatcggcgacggcaacaacatcctgcacagcatcatgatgagcgccgccaagttcggcatgcatctgcaggccgccacccccaagggctacgagcctgatgccagcgtgaccaagctggccgagcagtacgccaaagagaacggcaccaagctgctgctgaccaacgaccccctggaagccgcccacggcggcaacgtgctgatcaccgacacctggatcagcatgggccaggaagaggaaaagaagaagcggctgcaggccttccagggctaccaggtcacaatgaagaccgccaaggtggccgccagcgactggaccttcctgcactgcctgccccggaagcccgaagaggtggacgacgaggtgttctacagcccccggtccctggtgttccccgaggccgagaaccggaagtggaccattatggccgtgatggtgtccctgctgaccgactactccccccagctgcagaagcccaagttctagataagtgaa

SEQ ID NO: 180 - DNA, 1077 bp, Artificial Sequence
  Synthetic construct
atgggcgtcttcaacctgcggatcctgctgaacaacgccgccttccggaacggccacaacttcatggtccgcaacttcagatgcggccagcccctgcagaacagggtgcagctgaagggccgggacctgctgaccctgaagaacttcaccggcgaagagatcaggtacatgctgtggctgagcgccgacctgaagttccggatcaagcagaagggcgagtacctgcccctgctgcaaggcaagagcctgggcatgatcttcgagaagcggagcacccggacccggctgagcaccgagacaggctttgccctgctgggaggccacccctgctttctgaccacccaggacatccacctgggcgtgaacgagagcctgaccgacaccgccagagtgctgagcagcatggccgacgccgtgctggcccgggtgtacaagcagagcgacctggacaccctggccaaagaggccagcatccccatcatcaacggcctgagcgacctgtaccaccccatccagatcctggccgactacctgaccctgcaggaacactacagctccctgaagggcctgaccctgagctggatcggcgacggcaacaacatcctgcacagcatcatgatgagcgccgccaagttcggcatgcatctgcaggccgccacccccaagggctacgagcctgatgccagcgtgaccaagctggccgagcagtacgccaaagagaacggcaccaagctgctgctgaccaacgaccccctggaagccgcccacggcggcaacgtgctgatcaccgacacctggatcagcatgggccaggaagaggaaaagaagaagcggctgcaggccttccagggctaccaggtcacaatgaagaccgccaaggtggccgccagcgactggaccttcctgcactgcctgccccggaagcccgaagaggtggacgacgaggtgttctacagcccccggtccctggtgttccccgaggccgagaaccggaagtggaccattatggccgtgatggtgtccctgctgaccgactactccccccagctgcagaagcccaagttctagataagtgaa

SEQ ID NO: 181 - DNA, 1077 bp, Artificial Sequence
  Synthetic construct
atgctggtcttcaacctgcggatcctgctgaacaacgccgccttccggaacggccacaacttcatggtccgcaacttcagatgcggccagcccctgcagaacagggtgcagctgaagggccgggacctgctgaccctgaagaacttcaccggcgaagagatcaggtacatgctgtggctgagcgccgacctgaagttccggatcaagcagaagggcgagtacctgcccctgctgcaaggcaagagcctgggcatgatcttcgagaagcggagcacccggacccggctgagcaccgagacaggctttgccctgctgggaggccacccctgctttctgaccacccaggacatccacctgggcgtgaacgagagcctgaccgacaccgccagagtgctgagcagcatggccgacgccgtgctggcccgggtgtacaagcagagcgacctggacaccctggccaaagaggccagcatccccatcatcaacggcctgagcgacctgtaccaccccatccagatcctggccgactacctgaccctgcaggaacactacagctccctgaagggcctgaccctgagctggatcggcgacggcaacaacatcctgcacagcatcatgatgagcgccgccaagttcggcatgcatctgcaggccgccacccccaagggctacgagcctgatgccagcgtgaccaagctggccgagcagtacgccaaagagaacggcaccaagctgctgctgaccaacgaccccctggaagccgcccacggcggcaacgtgctgatcaccgacacctggatcagcatgggccaggaagaggaaaagaagaagcggctgcaggccttccagggctaccaggtcacaatgaagaccgccaaggtggccgccagcgactggaccttcctgcactgcctgccccggaagcccgaagaggtggacgacgaggtgttctacagcccccggtccctggtgttccccgaggccgagaaccggaagtggaccattatggccgtgatggtgtccctgctgaccgactactccccccagctgcagaagcccaagttctagataagtgaa

SEQ ID NO: 182 - DNA, 1074 bp, Artificial Sequence
  Synthetic construct
atgctgttcaacctgaggatcctgctgaacaacgcagctttcaggaacggccacaacttcatggtgaggaacttccggtgcggccagcccctgcagaacaaggtgcagctgaagggcagggacctgctgaccctgaagaacttcaccggagaggagatcaagtacatgctgtggctgagcgcagacctgaagttcaggatcaagcagaagggagagtacctgcccctgctgcaggggaagtccctgggcatgatcttcgagaagaggagtaccaggaccaggctgagcaccgaaaccggcttcgccctgctgggaggacacccctgcttcctgaccacccaggacatccacctgggcgtgaacgagagtctgaccgacaccgccagggtgctgtctagcatggccgacgccgtgctggccagggtgtacaagcagtcagacctggacaccctggctaaggaggccagcatccccatcatcaacggcctgagcgacctgtaccaccccatccagatcctggctgactacctgaccctgcaggagcactacagctctctgaagggcctgaccctgagctggatcggcgacgggaacaacatcctgcacagcatcatgatgagcgccgccaagttcggcatgcacctgcaggccgctacccccaagggttacgagcccgacgccagcgtgaccaagctggcagagcagtacgccaaggagaacggcaccaagctgctgctgaccaacgaccccctggaggccgcccacggaggcaacgtgctgatcaccgacacctggatcagcatgggacaggaggaggagaagaagaagcggctgcaggctttccagggttaccaggtgaccatgaagaccgccaaggtggctgccagcgactggaccttcctgcactgcctgcccaggaagcccgaggaggtggacgacgaggtgttctactctcccaggagcctggtgttccccgaggccgagaacaggaagtggaccatcatggctgtgatggtgtccctgctgaccgactacagcccccagctgcagaagcccaagttctgaataagtgaa

SEQ ID NO: 183 - DNA, 1074 bp, Artificial Sequence
  Synthetic construct
atgctgttcaacctgaggatcctgctgaacaacgcagctttcaggaacggccacaacttcatggtgaggaacttccggtgcggccagcccctgcagaacaaggtgcagctgaagggcagggacctgctgaccctgaagaacttcaccggagaggagatcaagtacatgctgtggctgagcgcagacctgaagttcaggatcaagcagaagggagagtacctgcccctgctgcaggggaagtccctgggcatgatcttcgagaagaggagtaccaggaccaggctgagcaccgaaaccggcttcgccctgctgggaggacacccctgcttcctgacgacccaggacatccacctcggagtgaacgaatccctcaccgataccgcccgggtgttatcaagcatggcagatgccgtgctggccagggtgtacaaacagtccgatctggacactctggctaaggaggccagcatccccatcatcaacggcctgagcgacctgtaccaccccatccagatcctggctgactacctgaccctgcaggagcactacagctctctgaagggcctgaccctgagctggatcggcgacgggaacaacatcctgcactccatcatgatgtccgccgcgaagttcggaatgcatctgcaagccgccacgccaaaaggatacgaaccggatgcgcccgtgacaaagttggcggaacagtacgctaaggagaacggaaccaagctgctgctgaccaacgaccccctggaggccgcccacggaggcaacgtgctgatcaccgacacctggatcagcatgggacaggaggaggagaagaagaagcggctgcaggctttccagggttaccaggtgaccatgaagaccgccaaggtggctgccagcgactggaccttcctgcactgcctgcccaggaagcccgaggaggtggacgacgaggtgttctactctcccaggagcctggtgttccccgaggccgagaacaggaagtggaccatcatggctgtgatggtgtccctgctgaccgactacagcccccagctgcagaagcccaagttctgaataagtgaa

SEQ ID NO: 184 - DNA, 1074 bp, Artificial Sequence; identical to SEQ ID NO: 178
  Synthetic construct

SEQ ID NO: 185 - DNA, 1074 bp, Artificial Sequence; identical to SEQ ID NO: 178
  Synthetic construct

SEQ ID NO: 186 - DNA, 1065 bp, Artificial Sequence
  Synthetic construct
atgcttttcaacttgagaatcctgctgaacaacgccgcctttcgcaacggtcacaattttatggtcagaaacttcagatgcggacagcccctccaaaacaaggtccagctgaagggccgcgatctcctcaccctgaagaacttcacgggggaggagatcaagtacatgctgtggctctccgctgacctgaagttcaggatcaagcagaagggagaatatctgccgctgctgcaagggaagtccctggggatgattttcgagaagcggagcacccggactcggctctccactgaaactggtttcgcccttctgggcggtcacccctgcttcctgaccactcaagacattcacctcggagtgaacgagtccttgactgacaccgcccgggtgctgtcgagcatggcagacgccgtgctagcccgcgtgtacaagcagtcagacctcgataccctggccaaggaggcttcgatcccgatcatcaacgggttgtccgacctgtaccacccgattcagattctcgccgactacctcaccctgcaagagcattacagctccctgaaggggcttaccctgtcctggattggcgacggaaacaacatcctgcactccattatgatgtcggcggccaagttcggcatgcacctccaagccgcgacccctaagggttacgaaccagacgcgtcagtgactaagctggccgaacagtacgcaaaggaaaatggcacgaagctgctcctgaccaacgatccgttggaagccgcccatggcggaaatgtgctcatcaccgacacctggatctcgatgggacaggaggaagagaagaagaagcggctgcaggcgttccagggctaccaggtcaccatgaaaactgccaaggtggccgccagcgactggaccttcctgcactgccttccgcgcaagcctgaggaggtggacgatgaagtgttctactctccacggtccctggtgttccccgaggcggagaaccgcaaatggaccatcatggctgtgatggtcagcctgctgaccgattacagccctcagttgcaaaagccgaagttttga

SEQ ID NO: 187 - DNA, 1065 bp, Artificial Sequence
  Synthetic construct
atgctgttcaacctccgcatcctcctcaacaacgccgcattcagaaacgggcacaacttcatggtcagaaacttccgctgcgggcaacccctacaaaacaaggtccagctcaaggggcgggacctcctgaccctgaagaacttcaccggcgaagagatcaagtacatgctgtggctctccgccgacctgaagttccgcatcaagcagaagggagagtacctcccgctgctgcaagggaagtcgctggggatgatcttcgagaagcggtcaaccagaacccggctgtcaaccgaaaccgggttcgcactgctggggggacacccgtgcttcctgaccacccaagacatccacctgggagtgaacgaatcgctgaccgacaccgcccgcgtgctgagctcaatggcggacgccgtgctggcccgcgtgtacaagcagtccgacctggacaccctggccaaggaagcgtccatcccgatcatcaacggactgtccgacctgtaccacccgatccagatcctggcagactacctgaccctgcaagaacactacagctccctgaagggcctgaccctgtcatggatcggggacgggaacaacatcctgcactccataatgatgtcagccgccaagttcggaatgcacctccaagccgcaaccccgaagggctacgaaccggacgcatcagtgaccaaactggccgagcagtacgccaaggaaaacggcaccaagctcctgctgaccaacgacccgctggaggccgcacacggggggaacgtgctgatcaccgacacctggatctccatgggacaggaggaggaaaagaagaagcggctgcaggcgttccaggggtaccaggtcaccatgaaaaccgcgaaggtcgcggcatcagactggaccttcctgcactgcctgccccggaagccggaagaggtggacgacgaggtgttctactcgccgcgctcgctggtgttccccgaggcggagaacaggaagtggaccatcatggcggtgatggtcagcctcctgaccgactactcgccgcagctgcagaagccgaagttctga

SEQ ID NO: 188 - DNA, 1074 bp, Artificial Sequence
  Synthetic construct
atgcttttcaatctccgcatcctccttaacaacgccgcgtttagaaacggccacaacttcatggtccggaacttcagatgtggccagccgcttcaaaacaaggtccagctgaagggccgggatcttctgaccctgaagaactttactggcgaagagatcaagtacatgctctggctctccgcggacttgaagttccgcattaagcagaagggggaataccttccgctgcttcaaggaaagagcctcggcatgatctttgagaagcgctcaaccaggacccgcctttctactgaaactgggttcgcgctgctcggtggccacccctgcttcctgacgacccaggacatccacctcggagtgaacgaatccctcaccgataccgcccgggtgttatcgagcatggcagatgccgtgctggccagggtgtacaaacagtccgatctggacactctggccaaggaggcgtcaattcctattatcaacggccttagtgacctctaccatccgattcagatcctggccgattacctcaccctgcaagaacactacagctccctgaagggtctgacattgtcctggatcggcgacggcaacaacattctccattccatcatgatgtccgccgcaaaattcggcatgcatcttcaagccgccacgccgaagggttacgagcccgacgcttccgtgactaagctcgccgagcagtacgctaaggagaacggaaccaagcttctgctgactaacgacccactagaagcagcccacgggggcaacgtgcttattactgacacctggatctccatgggccaggaagaagagaaaaagaagcggctgcaggcgttccagggatatcaggtcaccatgaaaaccgccaaggtcgctgcctccgactggaccttcctgcactgcctgcctcgcaagcctgaagaagtggacgacgaggtgttctactcgccacggagcctcgtgttccccgaggccgagaatagaaagtggaccatcatggccgtgatggtgtcactgctcaccgactacagcccgcagcttcagaagcccaagttctgaataagtaga

SEQ ID NO: 189 - DNA, 1074 bp, Artificial Sequence
  Synthetic construct
atgcttttcaacctgagaatcctcttgaacaatgctgcttttcggaatggccacaactttatggttcggaacttccgttgcggccagcctttacaaaacaaggtccagctgaagggccgggatttgctcacactaaagaactttactggagaagagatcaagtacatgctatggctgtcggccgacctgaagttccgtatcaagcagaagggagaataccttccgctgcttcaaggaaagagcctcggcatgatctttgagaagcgctcaaccaggacccgcctttctactgaaactgggttcgcgctgctcggtggccacccctgcttcctgacgacccaggacatccacctcggagtgaacgaatccctcaccgataccgcccgggtgttatcgagcatggcagatgccgtgctggccagggtgtacaaacagtccgatctcgataccttggcaaaggaggcttccattcccatcatcaacggcctgagcgacctgtaccacccaatccaaatcctggctgactacctgaccctgcaagagcactacagcagcctgaagggtctgaccctgtcatggattggcgatggaaacaatattctgcactccatcatgatgtccgccgcgaagttcggaatgcatctgcaagccgccactccaaaaggatacgaaccggatgcatccgtgaccaagttggcggaacagtacgcgaaggagaacggaaccaagctcctgctgactaacgacccgctcgaggctgcgcatgggggtaacgtgctgattacggacacctggatctccatggggcaggaggaagagaagaagaagagactgcaggcattccaggggtaccaggtcaccatgaaaaccgcaaaagtggcagcttcggactggactttcctgcattgcctgccgaggaagccggaggaagtcgacgacgaagtgttctactcgcctcggtccctggtgttccccgaggccgaaaaccggaagtggaccatcatggccgtgatggtgtccttgctgactgactatagcccgcagctgcagaagcctaagttctgaataagtaga

SEQ ID NO: 190 - DNA, 1074 bp, Artificial Sequence
  Synthetic construct
atgctgttcaacctgcgcatcctgctgaacaacgccgccttccgcaacggccacaacttcatggtgcgcaacttccgctgcggccagcccctgcagaacaaggtgcagctgaagggccgcgacctgctgaccctgaagaacttcaccggcgaggagatcaagtacatgctgtggctgagcgccgacctgaagttccgcatcaagcagaagggcgagtacctgcccctgctgcagggcaagagcctgggcatgatcttcgagaagcgcagcacccgcacccgcctgagcaccgagacaggcctggccctgctgggcggccacccctgcttcctgaccacccaggacatccacctgggcgtgaacgagagcctgaccgacaccgcccgcgtgctgagcagcatggccgacgccgtgctggcccgcgtgtacaagcagagcgacctggacaccctggccaaggaggccagcatccccatcatcaacggcctgagcgacctgtaccaccccatccagatcctggccgactacctgaccctgcaggagcactacagcagcctgaagggcctgaccctgagctggatcggcgacggcaacaacatcctgcacagcatcatgatgagcgccgccaagttcggcatgcacctgcaggccgccacccccaagggctacgagcccgacgccagcgtgaccaagctggccgagcagtacgccaaggagaacggcaccaagctgctgctgaccaacgaccccctggaggccgcccacggcggcaacgtgctgatcaccgacacctggatcagcatgggccaggaggaggagaagaagaagcgcctgcaggccttccagggctaccaggtgaccatgaagaccgccaaggtggccgccagcgactggaccttcctgcactgcctgccccgcaagcccgaggaggtggacgacgaggtgttctacagcccccgcagcctggtgttccccgaggccgagaaccgcaagtggaccatcatggccgtgatggtgagcctgctgaccgactacagcccccagctgcagaagcccaagttctgaataagtaga

SEQ ID NO: 191 - DNA, 1065 bp, Artificial Sequence; identical to SEQ ID NO: 136
  Synthetic construct

SEQ ID NO: 192 - DNA, 1065 bp, Artificial Sequence; identical to SEQ ID NO: 136
  Synthetic construct

SEQ ID NO: 193 - DNA, 1065 bp, Artificial Sequence; identical to SEQ ID NO: 136
  Synthetic construct

SEQ ID NO: 194 - DNA, 1065 bp, Artificial Sequence; identical to SEQ ID NO: 136
  Synthetic construct

SEQ ID NO: 195 - DNA, 1065 bp, Artificial Sequence; identical to SEQ ID NO: 136
  Synthetic construct

SEQ ID NO: 196 - DNA, 1065 bp, Artificial Sequence
  Synthetic construct
atggtgttcaacctccgcatcctcctcaacaacgccgcattcagaaacgggcacaacttcatggtcagaaacttccgctgcgggcaacccctacaaaacaaggtccagctcaaggggcgggacctcctgaccctgaagaacttcaccggcgaagagatcaagtacatgctgtggctctccgccgacctgaagttccgcatcaagcagaagggagagtacctcccgctgctgcaagggaagtcgctggggatgatcttcgagaagcggtcaaccagaacccggctgtcaaccgaaaccgggttcgcactgctggggggacacccgtgcttcctgaccacccaagacatccacctgggagtgaacgaatcgctgaccgacaccgcccgcgtgctgagctcaatggcggacgccgtgctggcccgcgtgtacaagcagtccgacctggacaccctggccaaggaagcgtccatcccgatcatcaacggactgtccgacctgtaccacccgatccagatcctggcagactacctgaccctgcaagaacactacagctccctgaagggcctgaccctgtcatggatcggggacgggaacaacatcctgcactccataatgatgtcagccgccaagttcggaatgcacctccaagccgcaaccccgaagggctacgaaccggacgcatcagtgaccaaactggccgagcagtacgccaaggaaaacggcaccaagctcctgctgaccaacgacccgctggaggccgcacacggggggaacgtgctgatcaccgacacctggatctccatgggacaggaggaggaaaagaagaagcggctgcaggcgttccaggggtaccaggtcaccatgaaaaccgcgaaggtcgcggcatcagactggaccttcctgcactgcctgccccggaagccggaagaggtggacgacgaggtgttctactcgccgcgctcgctggtgttccccgaggcggagaacaggaagtggaccatcatggcggtgatggtcagcctcctgaccgactactcgccgcagctgcagaagccgaagttctga

SEQ ID NO: 197 - DNA, 1065 bp, Artificial Sequence
  Synthetic construct
atggtgttcaacctccgcatcctcctcaacaacgccgcattcagaaacgggcacaacttcatggtcagaaacttccgctgcgggcaacccctacaaaaccgggtccagctcaaggggcgggacctcctgaccctgaagaacttcaccggcgaagagatcaagtacatgctgtggctctccgccgacctgaagttccgcatcaagcagaagggagagtacctcccgctgctgcaagggaagtcgctggggatgatcttcgagaagcggtcaaccagaacccggctgtcaaccgaaaccgggttcgcactgctggggggacacccgtgcttcctgaccacccaagacatccacctgggagtgaacgaatcgctgaccgacaccgcccgcgtgctgagctcaatggcggacgccgtgctggcccgcgtgtacaagcagtccgacctggacaccctggccaaggaagcgtccatcccgatcatcaacggactgtccgacctgtaccacccgatccagatcctggcagactacctgaccctgcaagaacactacagctccctgaagggcctgaccctgtcatggatcggggacgggaacaacatcctgcactccataatgatgtcagccgccaagttcggaatgcacctccaagccgcaaccccgaagggctacgaaccggacgcatcagtgaccaaactggccgagcagtacgccaaggaaaacggcaccaagctcctgctgaccaacgacccgctggaggccgcacacggggggaacgtgctgatcaccgacacctggatctccatgggacaggaggaggaaaagaagaagcggctgcaggcgttccaggggtaccaggtcaccatgaaaaccgcgaaggtcgcggcatcagactggaccttcctgcactgcctgccccggaagccggaagaggtggacgacgaggtgttctactcgccgcgctcgctggtgttccccgaggcggagaacaggaagtggaccatcatggcggtgatggtcagcctcctgaccgactactcgccgcagctgcagaagccgaagttctga

SEQ ID NO: 198 - DNA, 1065 bp, Artificial Sequence
  Synthetic construct
atggtgttcaacctccgcatcctcctcaacaacgccgcattcagaaacgggcacaacttcatggtcagaaacttccgctgcgggcaacccctacaaaaccgggtccagctcaaggggcgggacctcctgaccctgaagaacttcaccggcgaagagatccggtacatgctgtggctctccgccgacctgaagttccgcatcaagcagaagggagagtacctcccgctgctgcaagggaagtcgctggggatgatcttcgagaagcggtcaaccagaacccggctgtcaaccgaaaccgggttcgcactgctggggggacacccgtgcttcctgaccacccaagacatccacctgggagtgaacgaatcgctgaccgacaccgcccgcgtgctgagctcaatggcggacgccgtgctggcccgcgtgtacaagcagtccgacctggacaccctggccaaggaagcgtccatcccgatcatcaacggactgtccgacctgtaccacccgatccagatcctggcagactacctgaccctgcaagaacactacagctccctgaagggcctgaccctgtcatggatcggggacgggaacaacatcctgcactccataatgatgtcagccgccaagttcggaatgcacctccaagccgcaaccccgaagggctacgaaccggacgcatcagtgaccaaactggccgagcagtacgccaaggaaaacggcaccaagctcctgctgaccaacgacccgctggaggccgcacacggggggaacgtgctgatcaccgacacctggatctccatgggacaggaggaggaaaagaagaagcggctgcaggcgttccaggggtaccaggtcaccatgaaaaccgcgaaggtcgcggcatcagactggaccttcctgcactgcctgccccggaagccggaagaggtggacgacgaggtgttctactcgccgcgctcgctggtgttccccgaggcggagaacaggaagtggaccatcatggcggtgatggtcagcctcctgaccgactactcgccgcagctgcagaagccgaagttctga

SEQ ID NO: 199 - DNA, 1065 bp, Artificial Sequence
  Synthetic construct
atgctggtcaacctccgcatcctcctcaacaacgccgcattcagaaacgggcacaacttcatggtcagaaacttccgctgcgggcaacccctacaaaacaaggtccagctcaaggggcgggacctcctgaccctgaagaacttcaccggcgaagagatcaagtacatgctgtggctctccgccgacctgaagttccgcatcaagcagaagggagagtacctcccgctgctgcaagggaagtcgctggggatgatcttcgagaagcggtcaaccagaacccggctgtcaaccgaaaccgggttcgcactgctggggggacacccgtgcttcctgaccacccaagacatccacctgggagtgaacgaatcgctgaccgacaccgcccgcgtgctgagctcaatggcggacgccgtgctggcccgcgtgtacaagcagtccgacctggacaccctggccaaggaagcgtccatcccgatcatcaacggactgtccgacctgtaccacccgatccagatcctggcagactacctgaccctgcaagaacactacagctccctgaagggcctgaccctgtcatggatcggggacgggaacaacatcctgcactccataatgatgtcagccgccaagttcggaatgcacctccaagccgcaaccccgaagggctacgaaccggacgcatcagtgaccaaactggccgagcagtacgccaaggaaaacggcaccaagctcctgctgaccaacgacccgctggaggccgcacacggggggaacgtgctgatcaccgacacctggatctccatgggacaggaggaggaaaagaagaagcggctgcaggcgttccaggggtaccaggtcaccatgaaaaccgcgaaggtcgcggcatcagactggaccttcctgcactgcctgccccggaagccggaagaggtggacgacgaggtgttctactcgccgcgctcgctggtgttccccgaggcggagaacaggaagtggaccatcatggcggtgatggtcagcctcctgaccgactactcgccgcagctgcagaagccgaagttctga

SEQ ID NO: 200 - DNA, 1065 bp, Artificial Sequence
  Synthetic construct
atgctggtcaacctccgcatcctcctcaacaacgccgcattcagaaacgggcacaacttcatggtcagaaacttccgctgcgggcaacccctacaaaaccgggtccagctcaaggggcgggacctcctgaccctgaagaacttcaccggcgaagagatcaagtacatgctgtggctctccgccgacctgaagttccgcatcaagcagaagggagagtacctcccgctgctgcaagggaagtcgctggggatgatcttcgagaagcggtcaaccagaacccggctgtcaaccgaaaccgggttcgcactgctggggggacacccgtgcttcctgaccacccaagacatccacctgggagtgaacgaatcgctgaccgacaccgcccgcgtgctgagctcaatggcggacgccgtgctggcccgcgtgtacaagcagtccgacctggacaccctggccaaggaagcgtccatcccgatcatcaacggactgtccgacctgtaccacccgatccagatcctggcagactacctgaccctgcaagaacactacagctccctgaagggcctgaccctgtcatggatcggggacgggaacaacatcctgcactccataatgatgtcagccgccaagttcggaatgcacctccaagccgcaaccccgaagggctacgaaccggacgcatcagtgaccaaactggccgagcagtacgccaaggaaaacggcaccaagctcctgctgaccaacgacccgctggaggccgcacacggggggaacgtgctgatcaccgacacctggatctccatgggacaggaggaggaaaagaagaagcggctgcaggcgttccaggggtaccaggtcaccatgaaaaccgcgaaggtcgcggcatcagactggaccttcctgcactgcctgccccggaagccggaagaggtggacgacgaggtgttctactcgccgcgctcgctggtgttccccgaggcggagaacaggaagtggaccatcatggcggtgatggtcagcctcctgaccgactactcgccgcagctgcagaagccgaagttctga

SEQ ID NO: 201 - DNA, 1065 bp, Artificial Sequence
  Synthetic construct
atgctggtcaacctccgcatcctcctcaacaacgccgcattcagaaacgggcacaacttcatggtcagaaacttccgctgcgggcaacccctacaaaaccgggtccagctcaaggggcgggacctcctgaccctgaagaacttcaccggcgaagagatccggtacatgctgtggctctccgccgacctgaagttccgcatcaagcagaagggagagtacctcccgctgctgcaagggaagtcgctggggatgatcttcgagaagcggtcaaccagaacccggctgtcaaccgaaaccgggttcgcactgctggggggacacccgtgcttcctgaccacccaagacatccacctgggagtgaacgaatcgctgaccgacaccgcccgcgtgctgagctcaatggcggacgccgtgctggcccgcgtgtacaagcagtccgacctggacaccctggccaaggaagcgtccatcccgatcatcaacggactgtccgacctgtaccacccgatccagatcctggcagactacctgaccctgcaagaacactacagctccctgaagggcctgaccctgtcatggatcggggacgggaacaacatcctgcactccataatgatgtcagccgccaagttcggaatgcacctccaagccgcaaccccgaagggctacgaaccggacgcatcagtgaccaaactggccgagcagtacgccaaggaaaacggcaccaagctcctgctgaccaacgacccgctggaggccgcacacggggggaacgtgctgatcaccgacacctggatctccatgggacaggaggaggaaaagaagaagcggctgcaggcgttccaggggtaccaggtcaccatgaaaaccgcgaaggtcgcggcatcagactggaccttcctgcactgcctgccccggaagccggaagaggtggacgacgaggtgttctactcgccgcgctcgctggtgttccccgaggcggagaacaggaagtggaccatcatggcggtgatggtcagcctcctgaccgactactcgccgcagctgcagaagccgaagttctga

SEQ ID NO: 202 - DNA, 1065 bp, Artificial Sequence
  Synthetic construct
atgctggtcaacctgcgcatcctgctgaacaacgccgccttccgcaacggccacaacttcatggtgcgcaacttccgctgcggccagcccctgcagaacaaggtgcagctgaagggccgcgacctgctgaccctgaagaacttcaccggcgaggagatcaagtacatgctgtggctgagcgccgacctgaagttccgcatcaagcagaagggcgagtacctgcccctgctgcagggcaagagcctgggcatgatcttcgagaagcgcagcacccgcacccgcctgagcaccgagacaggcttcgccctgctgggcggccacccctgcttcctgaccacccaggacatccacctgggcgtgaacgagagcctgaccgacaccgcccgcgtgctgagcagcatggccgacgccgtgctggcccgcgtgtacaagcagagcgacctggacaccctggccaaggaggccagcatccccatcatcaacggcctgagcgacctgtaccaccccatccagatcctggccgactacctgaccctgcaggagcactacagcagcctgaagggcctgaccctgagctggatcggcgacggcaacaacatcctgcacagcatcatgatgagcgccgccaagttcggcatgcacctgcaggccgccacccccaagggctacgagcccgacgccagcgtgaccaagctggccgagcagtacgccaaggagaacggcaccaagctgctgctgaccaacgaccccctggaggccgcccacggcggcaacgtgctgatcaccgacacctggatcagcatgggccaggaggaggagaagaagaagcgcctgcaggccttccagggctaccaggtgaccatgaagaccgccaaggtggccgccagcgactggaccttcctgcactgcctgccccgcaagcccgaggaggtggacgacgaggtgttctacagcccccgcagcctggtgttccccgaggccgagaaccgcaagtggaccatcatggccgtgatggtgagcctgctgaccgactacagcccccagctgcagaagcccaagttctga

SEQ ID NO: 203 - DNA, 1065 bp, Artificial Sequence
  Synthetic construct
atgctggtcaacctgcgcatcctgctgaacaacgccgccttccgcaacggccacaacttcatggtgcgcaacttccgctgcggccagcccctgcagaaccgggtgcagctgaagggccgcgacctgctgaccctgaagaacttcaccggcgaggagatcaagtacatgctgtggctgagcgccgacctgaagttccgcatcaagcagaagggcgagtacctgcccctgctgcagggcaagagcctgggcatgatcttcgagaagcgcagcacccgcacccgcctgagcaccgagacaggcttcgccctgctgggcggccacccctgcttcctgaccacccaggacatccacctgggcgtgaacgagagcctgaccgacaccgcccgcgtgctgagcagcatggccgacgccgtgctggcccgcgtgtacaagcagagcgacctggacaccctggccaaggaggccagcatccccatcatcaacggcctgagcgacctgtaccaccccatccagatcctggccgactacctgaccctgcaggagcactacagcagcctgaagggcctgaccctgagctggatcggcgacggcaacaacatcctgcacagcatcatgatgagcgccgccaagttcggcatgcacctgcaggccgccacccccaagggctacgagcccgacgccagcgtgaccaagctggccgagcagtacgccaaggagaacggcaccaagctgctgctgaccaacgaccccctggaggccgcccacggcggcaacgtgctgatcaccgacacctggatcagcatgggccaggaggaggagaagaagaagcgcctgcaggccttccagggctaccaggtgaccatgaagaccgccaaggtggccgccagcgactggaccttcctgcactgcctgccccgcaagcccgaggaggtggacgacgaggtgttctacagcccccgcagcctggtgttccccgaggccgagaaccgcaagtggaccatcatggccgtgatggtgagcctgctgaccgactacagcccccagctgcagaagcccaagttctga

SEQ ID NO: 204 - DNA, 1065 bp, Artificial Sequence
  Synthetic construct
atgcttgtcaatctccgcatcctccttaacaacgccgcgtttagaaacggccacaacttcatggtccggaacttcagatgtggccagccgcttcaaaacaaggtccagctgaagggccgggatcttctgaccctgaagaactttactggcgaagagatcaagtacatgctctggctctccgcggacttgaagttccgcattaagcagaagggggaataccttccgctgcttcaaggaaagagcctcggcatgatctttgagaagcgctcaaccaggacccgcctttctactgaaactgggttcgcgctgctcggtggccacccctgcttcctgacgacccaggacatccacctcggagtgaacgaatccctcaccgataccgcccgggtgttatcgagcatggcagatgccgtgctggccagggtgtacaaacagtccgatctggacactctggccaaggaggcgtcaattcctattatcaacggccttagtgacctctaccatccgattcagatcctggccgattacctcaccctgcaagaacactacagctccctgaagggtctgacattgtcctggatcggcgacggcaacaacattctccattccatcatgatgtccgccgcaaaattcggcatgcatcttcaagccgccacgccgaagggttacgagcccgacgcttccgtgactaagctcgccgagcagtacgctaaggagaacggaaccaagcttctgctgactaacgacccactagaagcagcccacgggggcaacgtgcttattactgacacctggatctccatgggccaggaagaagagaaaaagaagcggctgcaggcgttccagggatatcaggtcaccatgaaaaccgccaaggtcgctgcctccgactggaccttcctgcactgcctgcctcgcaagcctgaagaagtggacgacgaggtgttctactcgccacggagcctcgtgttccccgaggccgagaatagaaagtggaccatcatggccgtgatggtgtcactgctcaccgactacagcccgcagcttcagaagcccaagttctag

SEQ ID NO: 205 - DNA, 1065 bp, Artificial Sequence
  Synthetic construct
atgcttgtcaatctccgcatcctccttaacaacgccgcgtttagaaacggccacaacttcatggtccggaacttcagatgtggccagccgcttcaaaaccgggtccagctgaagggccgggatcttctgaccctgaagaactttactggcgaagagatcaagtacatgctctggctctccgcggacttgaagttccgcattaagcagaagggggaataccttccgctgcttcaaggaaagagcctcggcatgatctttgagaagcgctcaaccaggacccgcctttctactgaaactgggttcgcgctgctcggtggccacccctgcttcctgacgacccaggacatccacctcggagtgaacgaatccctcaccgataccgcccgggtgttatcgagcatggcagatgccgtgctggccagggtgtacaaacagtccgatctggacactctggccaaggaggcgtcaattcctattatcaacggccttagtgacctctaccatccgattcagatcctggccgattacctcaccctgcaagaacactacagctccctgaagggtctgacattgtcctggatcggcgacggcaacaacattctccattccatcatgatgtccgccgcaaaattcggcatgcatcttcaagccgccacgccgaagggttacgagcccgacgcttccgtgactaagctcgccgagcagtacgctaaggagaacggaaccaagcttctgctgactaacgacccactagaagcagcccacgggggcaacgtgcttattactgacacctggatctccatgggccaggaagaagagaaaaagaagcggctgcaggcgttccagggatatcaggtcaccatgaaaaccgccaaggtcgctgcctccgactggaccttcctgcactgcctgcctcgcaagcctgaagaagtggacgacgaggtgttctactcgccacggagcctcgtgttccccgaggccgagaatagaaagtggaccatcatggccgtgatggtgtcactgctcaccgactacagcccgcagcttcagaagcccaagttctag

SEQ ID NO: 206 - DNA, 1068 bp, Artificial Sequence
  Synthetic construct
atgggccttgtcaatctccgcatcctccttaacaacgccgcgtttagaaacggccacaacttcatggtccggaacttcagatgtggccagccgcttcaaaacaaggtccagctgaagggccgggatcttctgaccctgaagaactttactggcgaagagatcaagtacatgctctggctctccgcggacttgaagttccgcattaagcagaagggggaataccttccgctgcttcaaggaaagagcctcggcatgatctttgagaagcgctcaaccaggacccgcctttctactgaaactgggttcgcgctgctcggtggccacccctgcttcctgacgacccaggacatccacctcggagtgaacgaatccctcaccgataccgcccgggtgttatcgagcatggcagatgccgtgctggccagggtgtacaaacagtccgatctggacactctggccaaggaggcgtcaattcctattatcaacggccttagtgacctctaccatccgattcagatcctggccgattacctcaccctgcaagaacactacagctccctgaagggtctgacattgtcctggatcggcgacggcaacaacattctccattccatcatgatgtccgccgcaaaattcggcatgcatcttcaagccgccacgccgaagggttacgagcccgacgcttccgtgactaagctcgccgagcagtacgctaaggagaacggaaccaagcttctgctgactaacgacccactagaagcagcccacgggggcaacgtgcttattactgacacctggatctccatgggccaggaagaagagaaaaagaagcggctgcaggcgttccagggatatcaggtcaccatgaaaaccgccaaggtcgctgcctccgactggaccttcctgcactgcctgcctcgcaagcctgaagaagtggacgacgaggtgttctactcgccacggagcctcgtgttccccgaggccgagaatagaaagtggaccatcatggccgtgatggtgtcactgctcaccgactacagcccgcagcttcagaagcccaagttctag

SEQ ID NO: 207 - DNA, 1068 bp, Artificial Sequence
  Synthetic construct
atgggccttgtcaatctccgcatcctccttaacaacgccgcgtttagaaacggccacaacttcatggtccggaacttcagatgtggccagccgcttcaaaaccgggtccagctgaagggccgggatcttctgaccctgaagaactttactggcgaagagatcaagtacatgctctggctctccgcggacttgaagttccgcattaagcagaagggggaataccttccgctgcttcaaggaaagagcctcggcatgatctttgagaagcgctcaaccaggacccgcctttctactgaaactgggttcgcgctgctcggtggccacccctgcttcctgacgacccaggacatccacctcggagtgaacgaatccctcaccgataccgcccgggtgttatcgagcatggcagatgccgtgctggccagggtgtacaaacagtccgatctggacactctggccaaggaggcgtcaattcctattatcaacggccttagtgacctctaccatccgattcagatcctggccgattacctcaccctgcaagaacactacagctccctgaagggtctgacattgtcctggatcggcgacggcaacaacattctccattccatcatgatgtccgccgcaaaattcggcatgcatcttcaagccgccacgccgaagggttacgagcccgacgcttccgtgactaagctcgccgagcagtacgctaaggagaacggaaccaagcttctgctgactaacgacccactagaagcagcccacgggggcaacgtgcttattactgacacctggatctccatgggccaggaagaagagaaaaagaagcggctgcaggcgttccagggatatcaggtcaccatgaaaaccgccaaggtcgctgcctccgactggaccttcctgcactgcctgcctcgcaagcctgaagaagtggacgacgaggtgttctactcgccacggagcctcgtgttccccgaggccgagaatagaaagtggaccatcatggccgtgatggtgtcactgctcaccgactacagcccgcagcttcagaagcccaagttctag

SEQ ID NO: 208 - DNA, 1071 bp, Artificial Sequence
  Synthetic construct
atgggcggacttgtcaatctccgcatcctccttaacaacgccgcgtttagaaacggccacaacttcatggtccggaacttcagatgtggccagccgcttcaaaacaaggtccagctgaagggccgggatcttctgaccctgaagaactttactggcgaagagatcaagtacatgctctggctctccgcggacttgaagttccgcattaagcagaagggggaataccttccgctgcttcaaggaaagagcctcggcatgatctttgagaagcgctcaaccaggacccgcctttctactgaaactgggttcgcgctgctcggtggccacccctgcttcctgacgacccaggacatccacctcggagtgaacgaatccctcaccgataccgcccgggtgttatcgagcatggcagatgccgtgctggccagggtgtacaaacagtccgatctggacactctggccaaggaggcgtcaattcctattatcaacggccttagtgacctctaccatccgattcagatcctggccgattacctcaccctgcaagaacactacagctccctgaagggtctgacattgtcctggatcggcgacggcaacaacattctccattccatcatgatgtccgccgcaaaattcggcatgcatcttcaagccgccacgccgaagggttacgagcccgacgcttccgtgactaagctcgccgagcagtacgctaaggagaacggaaccaagcttctgctgactaacgacccactagaagcagcccacgggggcaacgtgcttattactgacacctggatctccatgggccaggaagaagagaaaaagaagcggctgcaggcgttccagggatatcaggtcaccatgaaaaccgccaaggtcgctgcctccgactggaccttcctgcactgcctgcctcgcaagcctgaagaagtggacgacgaggtgttctactcgccacggagcctcgtgttccccgaggccgagaatagaaagtggaccatcatggccgtgatggtgtcactgctcaccgactacagcccgcagcttcagaagcccaagttctag

SEQ ID NO: 209 - DNA, 1077 bp, Artificial Sequence
  Synthetic construct
atggcccttttcaatctccgcatcctccttaacaacgccgcgtttagaaacggccacaacttcatggtccggaacttcagatgtggccagccgcttcaaggcaaggtccagctgaagggccgggatcttctgaccctgaagaactttactggcgaagagatcaagtacatgctctggctctccgcggacttgaagttccgcattaagcagaagggggaataccttccgctgcttcaaggaaagagcctcggcatgatctttgagaagcgctcaaccaggacccgcctttctactgaaactgggttcgcgctgctcggtggccacccctgcttcctgacgacccaggacatccacctcggagtgaacgaatccctcaccgataccgcccgggtgttatcgagcatggcagatgccgtgctggccagggtgtacaaacagtccgatctggacactctggccaaggaggcgtcaattcctattatcaacggccttagtgacctctaccatccgattcagatcctggccgattacctcaccctgcaagaacactacagctccctgaagggtctgacattgtcctggatcggcgacggcaacaacattctccattccatcatgatgtccgccgcaaaattcggcatgcatcttcaagccgccacgccgaagggttacgagcccgacgcttccgtgactaagctcgccgagcagtacgctaaggagaacggaaccaagcttctgctgactaacgacccactagaagcagcccacgggggcaacgtgcttattactgacacctggatctccatgggccaggaagaagagaaaaagaagcggctgcaggcgttccagggatatcaggtcaccatgaaaaccgccaaggtcgctgcctccgactggaccttcctgcactgcctgcctcgcaagcctgaagaagtggacgacgaggtgttctactcgccacggagcctcgtgttccccgaggccgagaatagaaagtggaccatcatggccgtgatggtgtcactgctcaccgactacagcccgcagcttcagaagcccaagttctagataagtgaa

SEQ ID NO: 210 - DNA, 1077 bp, Artificial Sequence
  Synthetic construct
atggcccttttcaatctccgcatcctccttaacaacgccgcgtttagaaacggccacaacttcatggtccggaacttcagatgtggccagccgcttcaaggccgggtccagctgaagggccgggatcttctgaccctgaagaactttactggcgaagagatcaagtacatgctctggctctccgcggacttgaagttccgcattaagcagaagggggaataccttccgctgcttcaaggaaagagcctcggcatgatctttgagaagcgctcaaccaggacccgcctttctactgaaactgggttcgcgctgctcggtggccacccctgcttcctgacgacccaggacatccacctcggagtgaacgaatccctcaccgataccgcccgggtgttatcgagcatggcagatgccgtgctggccagggtgtacaaacagtccgatctggacactctggccaaggaggcgtcaattcctattatcaacggccttagtgacctctaccatccgattcagatcctggccgattacctcaccctgcaagaacactacagctccctgaagggtctgacattgtcctggatcggcgacggcaacaacattctccattccatcatgatgtccgccgcaaaattcggcatgcatcttcaagccgccacgccgaagggttacgagcccgacgcttccgtgactaagctcgccgagcagtacgctaaggagaacggaaccaagcttctgctgactaacgacccactagaagcagcccacgggggcaacgtgcttattactgacacctggatctccatgggccaggaagaagagaaaaagaagcggctgcaggcgttccagggatatcaggtcaccatgaaaaccgccaaggtcgctgcctccgactggaccttcctgcactgcctgcctcgcaagcctgaagaagtggacgacgaggtgttctactcgccacggagcctcgtgttccccgaggccgagaatagaaagtggaccatcatggccgtgatggtgtcactgctcaccgactacagcccgcagcttcagaagcccaagttctagataagtgaa

SEQ ID NO: 211 - DNA, 1077 bp, Artificial Sequence
  Synthetic construct
atggcccttttcaatctccgcatcctccttaacaacgccgcgtttagaaacggccacaacttcatggtccggaacttcagatgtggccagccgcttcaaggccgggtccagctgaagggccgggatcttctgaccctgaagaactttactggcgaagagatcaggtacatgctctggctctccgcggacttgaagttccgcattaagcagaagggggaataccttccgctgcttcaaggaaagagcctcggcatgatctttgagaagcgctcaaccaggacccgcctttctactgaaactgggttcgcgctgctcggtggccacccctgcttcctgacgacccaggacatccacctcggagtgaacgaatccctcaccgataccgcccgggtgttatcgagcatggcagatgccgtgctggccagggtgtacaaacagtccgatctggacactctggccaaggaggcgtcaattcctattatcaacggccttagtgacctctaccatccgattcagatcctggccgattacctcaccctgcaagaacactacagctccctgaagggtctgacattgtcctggatcggcgacggcaacaacattctccattccatcatgatgtccgccgcaaaattcggcatgcatcttcaagccgccacgccgaagggttacgagcccgacgcttccgtgactaagctcgccgagcagtacgctaaggagaacggaaccaagcttctgctgactaacgacccactagaagcagcccacgggggcaacgtgcttattactgacacctggatctccatgggccaggaagaagagaaaaagaagcggctgcaggcgttccagggatatcaggtcaccatgaaaaccgccaaggtcgctgcctccgactggaccttcctgcactgcctgcctcgcaagcctgaagaagtggacgacgaggtgttctactcgccacggagcctcgtgttccccgaggccgagaatagaaagtggaccatcatggccgtgatggtgtcactgctcaccgactacagcccgcagcttcagaagcccaagttctagataagtgaa

SEQ ID NO: 212 - DNA, 1077 bp, Artificial Sequence
  Synthetic construct
atggcccttgtcaatctccgcatcctccttaacaacgccgcgtttagaaacggccacaacttcatggtccggaacttcagatgtggccagccgcttcaaggcagggtccagctgaagggccgggatcttctgaccctgaagaactttactggcgaagagatcaagtacatgctctggctctccgcggacttgaagttccgcattaagcagaagggggaataccttccgctgcttcaaggaaagagcctcggcatgatctttgagaagcgctcaaccaggacccgcctttctactgaaactgggttcgcgctgctcggtggccacccctgcttcctgacgacccaggacatccacctcggagtgaacgaatccctcaccgataccgcccgggtgttatcgagcatggcagatgccgtgctggccagggtgtacaaacagtccgatctggacactctggccaaggaggcgtcaattcctattatcaacggccttagtgacctctaccatccgattcagatcctggccgattacctcaccctgcaagaacactacagctccctgaagggtctgacattgtcctggatcggcgacggcaacaacattctccattccatcatgatgtccgccgcaaaattcggcatgcatcttcaagccgccacgccgaagggttacgagcccgacgcttccgtgactaagctcgccgagcagtacgctaaggagaacggaaccaagcttctgctgactaacgacccactagaagcagcccacgggggcaacgtgcttattactgacacctggatctccatgggccaggaagaagagaaaaagaagcggctgcaggcgttccagggatatcaggtcaccatgaaaaccgccaaggtcgctgcctccgactggaccttcctgcactgcctgcctcgcaagcctgaagaagtggacgacgaggtgttctactcgccacggagcctcgtgttccccgaggccgagaatagaaagtggaccatcatggccgtgatggtgtcactgctcaccgactacagcccgcagcttcagaagcccaagttctaagtgaataga

SEQ ID NO: 213 - DNA, 1077 bp, Artificial Sequence
  Synthetic construct
atggcccttttcaatctccgcatcctccttaacaacgccgcgtttagaaacggccacaacttcatggtccggaacttcagatgtggccagccgcttcaagtcaaggtccagctgaagggccgggatcttctgaccctgaagaactttactggcgaagagatcaagtacatgctctggctctccgcggacttgaagttccgcattaagcagaagggggaataccttccgctgcttcaaggaaagagcctcggcatgatctttgagaagcgctcaaccaggacccgcctttctactgaaactgggttcgcgctgctcggtggccacccctgcttcctgacgacccaggacatccacctcggagtgaacgaatccctcaccgataccgcccgggtgttatcgagcatggcagatgccgtgctggccagggtgtacaaacagtccgatctggacactctggccaaggaggcgtcaattcctattatcaacggccttagtgacctctaccatccgattcagatcctggccgattacctcaccctgcaagaacactacagctccctgaagggtctgacattgtcctggatcggcgacggcaacaacattctccattccatcatgatgtccgccgcaaaattcggcatgcatcttcaagccgccacgccgaagggttacgagcccgacgcttccgtgactaagctcgccgagcagtacgctaaggagaacggaaccaagcttctgctgactaacgacccactagaagcagcccacgggggcaacgtgcttattactgacacctggatctccatgggccaggaagaagagaaaaagaagcggctgcaggcgttccagggatatcaggtcaccatgaaaaccgccaaggtcgctgcctccgactggaccttcctgcactgcctgcctcgcaagcctgaagaagtggacgacgaggtgttctactcgccacggagcctcgtgttccccgaggccgagaatagaaagtggaccatcatggccgtgatggtgtcactgctcaccgactacagcccgcagcttcagaagcccaagttctagataagtgaa

SEQ ID NO: 214 - DNA, 1077 bp, Artificial Sequence
  Synthetic construct
atggcccttttcaatctccgcatcctccttaacaacgccgcgtttagaaacggccacaacttcatggtccggaacttcagatgtggccagccgcttcaagtcagggtccagctgaagggccgggatcttctgaccctgaagaactttactggcgaagagatcaagtacatgctctggctctccgcggacttgaagttccgcattaagcagaagggggaataccttccgctgcttcaaggaaagagcctcggcatgatctttgagaagcgctcaaccaggacccgcctttctactgaaactgggttcgcgctgctcggtggccacccctgcttcctgacgacccaggacatccacctcggagtgaacgaatccctcaccgataccgcccgggtgttatcgagcatggcagatgccgtgctggccagggtgtacaaacagtccgatctggacactctggccaaggaggcgtcaattcctattatcaacggccttagtgacctctaccatccgattcagatcctggccgattacctcaccctgcaagaacactacagctccctgaagggtctgacattgtcctggatcggcgacggcaacaacattctccattccatcatgatgtccgccgcaaaattcggcatgcatcttcaagccgccacgccgaagggttacgagcccgacgcttccgtgactaagctcgccgagcagtacgctaaggagaacggaaccaagcttctgctgactaacgacccactagaagcagcccacgggggcaacgtgcttattactgacacctggatctccatgggccaggaagaagagaaaaagaagcggctgcaggcgttccagggatatcaggtcaccatgaaaaccgccaaggtcgctgcctccgactggaccttcctgcactgcctgcctcgcaagcctgaagaagtggacgacgaggtgttctactcgccacggagcctcgtgttccccgaggccgagaatagaaagtggaccatcatggccgtgatggtgtcactgctcaccgactacagcccgcagcttcagaagcccaagttctagataagtgaa

SEQ ID NO: 215 - DNA, 1065 bp, Artificial Sequence; identical to SEQ ID NO: 175
  Synthetic construct

SEQ ID NO: 216 - DNA, 1068 bp, Artificial Sequence
  Synthetic construct
atgggagtattcaacctgcgcatcctgctgaacaacgccgccttccgcaacggccacaacttcatggtgcgcaacttccgctgcggccagcccctgcagaacaaggtgcagctgaagggccgcgacctgctgaccctgaagaacttcaccggcgaggagatcaagtacatgctgtggctgagcgccgacctgaagttccgcatcaagcagaagggcgagtacctgcccctgctgcagggcaagagcctgggcatgatcttcgagaagcgcagcacccgcacccgcctgagcaccgagacaggcttcgccctgctgggcggccacccctgcttcctgaccacccaggacatccacctgggcgtgaacgagagcctgaccgacaccgcccgcgtgctgagcagcatggccgacgccgtgctggcccgcgtgtacaagcagagcgacctggacaccctggccaaggaggccagcatccccatcatcaacggcctgagcgacctgtaccaccccatccagatcctggccgactacctgaccctgcaggagcactacagcagcctgaagggcctgaccctgagctggatcggcgacggcaacaacatcctgcacagcatcatgatgagcgccgccaagttcggcatgcacctgcaggccgccacccccaagggctacgagcccgacgccagcgtgaccaagctggccgagcagtacgccaaggagaacggcaccaagctgctgctgaccaacgaccccctggaggccgcccacggcggcaacgtgctgatcaccgacacctggatcagcatgggccaggaggaggagaagaagaagcgcctgcaggccttccagggctaccaggtgaccatgaagaccgccaaggtggccgccagcgactggaccttcctgcactgcctgccccgcaagcccgaggaggtggacgacgaggtgttctacagcccccgcagcctggtgttccccgaggccgagaaccgcaagtggaccatcatggccgtgatggtgagcctgctgaccgactacagcccccagctgcagaagcccaagttctga

SEQ ID NO: 217 - DNA, 1068 bp, Artificial Sequence
  Synthetic construct
atgggagtattcaacctgcgcatcctgctgaacaacgccgccttccgcaacggccacaacttcatggtgcgcaacttccgctgcggccagcccctgcagaaccgggtgcagctgaagggccgcgacctgctgaccctgaagaacttcaccggcgaggagatccggtacatgctgtggctgagcgccgacctgaagttccgcatcaagcagaagggcgagtacctgcccctgctgcagggcaagagcctgggcatgatcttcgagaagcgcagcacccgcacccgcctgagcaccgagacaggcttcgccctgctgggcggccacccctgcttcctgaccacccaggacatccacctgggcgtgaacgagagcctgaccgacaccgcccgcgtgctgagcagcatggccgacgccgtgctggcccgcgtgtacaagcagagcgacctggacaccctggccaaggaggccagcatccccatcatcaacggcctgagcgacctgtaccaccccatccagatcctggccgactacctgaccctgcaggagcactacagcagcctgaagggcctgaccctgagctggatcggcgacggcaacaacatcctgcacagcatcatgatgagcgccgccaagttcggcatgcacctgcaggccgccacccccaagggctacgagcccgacgccagcgtgaccaagctggccgagcagtacgccaaggagaacggcaccaagctgctgctgaccaacgaccccctggaggccgcccacggcggcaacgtgctgatcaccgacacctggatcagcatgggccaggaggaggagaagaagaagcgcctgcaggccttccagggctaccaggtgaccatgaagaccgccaaggtggccgccagcgactggaccttcctgcactgcctgccccgcaagcccgaggaggtggacgacgaggtgttctacagcccccgcagcctggtgttccccgaggccgagaaccgcaagtggaccatcatggccgtgatggtgagcctgctgaccgactacagcccccagctgcagaagcccaagttctga

SEQ ID NO: 218 - DNA, 1068 bp, Artificial Sequence
  Synthetic construct
atgctggtattcaacctgcgcatcctgctgaacaacgccgccttccgcaacggccacaacttcatggtgcgcaacttccgctgcggccagcccctgcagaaccgggtgcagctgaagggccgcgacctgctgaccctgaagaacttcaccggcgaggagatccggtacatgctgtggctgagcgccgacctgaagttccgcatcaagcagaagggcgagtacctgcccctgctgcagggcaagagcctgggcatgatcttcgagaagcgcagcacccgcacccgcctgagcaccgagacaggcttcgccctgctgggcggccacccctgcttcctgaccacccaggacatccacctgggcgtgaacgagagcctgaccgacaccgcccgcgtgctgagcagcatggccgacgccgtgctggcccgcgtgtacaagcagagcgacctggacaccctggccaaggaggccagcatccccatcatcaacggcctgagcgacctgtaccaccccatccagatcctggccgactacctgaccctgcaggagcactacagcagcctgaagggcctgaccctgagctggatcggcgacggcaacaacatcctgcacagcatcatgatgagcgccgccaagttcggcatgcacctgcaggccgccacccccaagggctacgagcccgacgccagcgtgaccaagctggccgagcagtacgccaaggagaacggcaccaagctgctgctgaccaacgaccccctggaggccgcccacggcggcaacgtgctgatcaccgacacctggatcagcatgggccaggaggaggagaagaagaagcgcctgcaggccttccagggctaccaggtgaccatgaagaccgccaaggtggccgccagcgactggaccttcctgcactgcctgccccgcaagcccgaggaggtggacgacgaggtgttctacagcccccgcagcctggtgttccccgaggccgagaaccgcaagtggaccatcatggccgtgatggtgagcctgctgaccgactacagcccccagctgcagaagcccaagttctga

SEQ ID NO: 219 - DNA, 1068 bp, Artificial Sequence; identical to SEQ ID NO: 216
  Synthetic construct

SEQ ID NO: 220 - DNA, 1068 bp, Artificial Sequence; identical to SEQ ID NO: 217
  Synthetic construct

SEQ ID NO: 221 - DNA, 1068 bp, Artificial Sequence; identical to SEQ ID NO: 218
  Synthetic construct

SEQ ID NO: 222 - DNA, 1073 bp, Artificial Sequence
  Synthetic construct
atgttgttcaacttgaggatcttgttgaacaacgccgccttcaggaacggacacaacttcatggtaaggaacttcaggtgcggacagcccttgcagaacaaagtacagttgaaaggaagggacttgttgacattgaaaaacttcacaggagaagaaatcaaatacatgttgtggttgtcggccgacttgaaattcaggatcaaacagaaaggagaatacttgcccttgttgcagggaaaatcgttgggaatgatcttcgaaaaaaggtcgacaaggacaaggttgtcgacagaaacaggattcgccttgttgggaggacacccctgcttcttgacaacacaggacatccacttgggagtaaacgaatcgttgacagacacagccagggtattgtcgtcgatggccgacgccgtattggccagggtatacaaacagtcggacttggacacattggccaaagaagcctcgatccccatcatcaacggattgtcggacttgtaccaccccatccagatcttggccgactacttgacattgcaggaacactactcgtcgttgaaaggattgacattgtcgtggatcggagacggaaacaacatcttgcactcgatcatgatgtcggccgccaaattcggaatgcacttgcaggccgccacacccaaaggatacgaacccgacgcctcggtaacaaaattggccgaacagtacgccaaagaaaacggaacaaaattgttgttgacaaacgaccccttggaagccgcccacggaggaaacgtattgatcacagacacatggatctcgatgggacaggaagaagaaaaaaaaaaaaggttgcaggccttccagggataccaggtaacaatgaaaacagccaaagtagccgcctcggactggacattcttgcactgcttgcccaggaaacccgaagaagtagacgacgaagtattctactcgcccaggtcgttggtattccccgaagccgaaaacaggaaatggacaatcatggccgtaatggtatcgttgttgacagactactcgccccagttgcagaaacccaaattctgaatagtgaa

SEQ ID NO: 223 - DNA, 1065 bp, Artificial Sequence
  Synthetic construct
atgctgttcaacctgcgcatcctgctgaacaacgccgccttccgcaacggccacaacttcatggtgcgcaacttccgctgcggccagcccctgcagggcaaggtgcagctgaagggccgcgacctgctgaccctgaagaacttcaccggcgaggagatcaagtacatgctgtggctgagcgccgacctgaagttccgcatcaagcagaagggcgagtacctgcccctgctgcagggcaagagcctgggcatgatcttcgagaagcgcagcacccgcacccgcctgagcaccgagacaggcttcgccctgctgggcggccacccctgcttcctgaccacccaggacatccacctgggcgtgaacgagagcctgaccgacaccgcccgcgtgctgagcagcatggccgacgccgtgctggcccgcgtgtacaagcagagcgacctggacaccctggccaaggaggccagcatccccatcatcaacggcctgagcgacctgtaccaccccatccagatcctggccgactacctgaccctgcaggagcactacagcagcctgaagggcctgaccctgagctggatcggcgacggcaacaacatcctgcacagcatcatgatgagcgccgccaagttcggcatgcacctgcaggccgccacccccaagggctacgagcccgacgccagcgtgaccaagctggccgagcagtacgccaaggagaacggcaccaagctgctgctgaccaacgaccccctggaggccgcccacggcggcaacgtgctgatcaccgacacctggatcagcatgggccaggaggaggagaagaagaagcgcctgcaggccttccagggctaccaggtgaccatgaagaccgccaaggtggccgccagcgactggaccttcctgcactgcctgccccgcaagcccgaggaggtggacgacgaggtgttctacagcccccgcagcctggtgttccccgaggccgagaaccgcaagtggaccatcatggccgtgatggtgagcctgctgaccgactacagcccccagctgcagaagcccaagttctga

SEQ ID NO: 224 - DNA, 1065 bp, Artificial Sequence
  Synthetic construct
atgctgttcaacctgcgcatcctgctgaacaacgccgccttccgcaacggccacaacttcatggtgcgcaacttccgctgcggccagcccctgcagggccgggtgcagctgaagggccgcgacctgctgaccctgaagaacttcaccggcgaggagatcaagtacatgctgtggctgagcgccgacctgaagttccgcatcaagcagaagggcgagtacctgcccctgctgcagggcaagagcctgggcatgatcttcgagaagcgcagcacccgcacccgcctgagcaccgagacaggcttcgccctgctgggcggccacccctgcttcctgaccacccaggacatccacctgggcgtgaacgagagcctgaccgacaccgcccgcgtgctgagcagcatggccgacgccgtgctggcccgcgtgtacaagcagagcgacctggacaccctggccaaggaggccagcatccccatcatcaacggcctgagcgacctgtaccaccccatccagatcctggccgactacctgaccctgcaggagcactacagcagcctgaagggcctgaccctgagctggatcggcgacggcaacaacatcctgcacagcatcatgatgagcgccgccaagttcggcatgcacctgcaggccgccacccccaagggctacgagcccgacgccagcgtgaccaagctggccgagcagtacgccaaggagaacggcaccaagctgctgctgaccaacgaccccctggaggccgcccacggcggcaacgtgctgatcaccgacacctggatcagcatgggccaggaggaggagaagaagaagcgcctgcaggccttccagggctaccaggtgaccatgaagaccgccaaggtggccgccagcgactggaccttcctgcactgcctgccccgcaagcccgaggaggtggacgacgaggtgttctacagcccccgcagcctggtgttccccgaggccgagaaccgcaagtggaccatcatggccgtgatggtgagcctgctgaccgactacagcccccagctgcagaagcccaagttctga

SEQ ID NO: 225 - DNA, 1065 bp, Artificial Sequence
  Synthetic construct
atgctgttcaacctgcgcatcctgctgaacaacgccgccttccgcaacggccacaacttcatggtgcgcaacttccgctgcggccagcccctgcagggccgggtgcagctgaagggccgcgacctgctgaccctgaagaacttcaccggcgaggagatccggtacatgctgtggctgagcgccgacctgaagttccgcatcaagcagaagggcgagtacctgcccctgctgcagggcaagagcctgggcatgatcttcgagaagcgcagcacccgcacccgcctgagcaccgagacaggcttcgccctgctgggcggccacccctgcttcctgaccacccaggacatccacctgggcgtgaacgagagcctgaccgacaccgcccgcgtgctgagcagcatggccgacgccgtgctggcccgcgtgtacaagcagagcgacctggacaccctggccaaggaggccagcatccccatcatcaacggcctgagcgacctgtaccaccccatccagatcctggccgactacctgaccctgcaggagcactacagcagcctgaagggcctgaccctgagctggatcggcgacggcaacaacatcctgcacagcatcatgatgagcgccgccaagttcggcatgcacctgcaggccgccacccccaagggctacgagcccgacgccagcgtgaccaagctggccgagcagtacgccaaggagaacggcaccaagctgctgctgaccaacgaccccctggaggccgcccacggcggcaacgtgctgatcaccgacacctggatcagcatgggccaggaggaggagaagaagaagcgcctgcaggccttccagggctaccaggtgaccatgaagaccgccaaggtggccgccagcgactggaccttcctgcactgcctgccccgcaagcccgaggaggtggacgacgaggtgttctacagcccccgcagcctggtgttccccgaggccgagaaccgcaagtggaccatcatggccgtgatggtgagcctgctgaccgactacagcccccagctgcagaagcccaagttctga

SEQ ID NO: 226 - DNA, 1065 bp, Artificial Sequence; identical to SEQ ID NO: 223
  Synthetic construct

SEQ ID NO: 227 - DNA, 1065 bp, Artificial Sequence; identical to SEQ ID NO: 175
  Synthetic construct

SEQ ID NO: 228 - DNA, 1068 bp, Artificial Sequence; identical to SEQ ID NO: 218
  Synthetic construct

SEQ ID NO: 229 - DNA, 1068 bp, Artificial Sequence; identical to SEQ ID NO: 218
  Synthetic construct

SEQ ID NO: 230 - RNA, 21 nt, Artificial Sequence
  Synthetic construct
aaccaaucgaaagaaaccaaa

SEQ ID NO: 231 - RNA, 21 nt, Artificial Sequence
  Synthetic construct
cucuaaucaccaggaguaaaa

SEQ ID NO: 232 - RNA, 21 nt, Artificial Sequence
  Synthetic construct
gagagagaucuuaacaaaaaa

SEQ ID NO: 233 - RNA, 21 nt, Artificial Sequence
  Synthetic construct
uguguaacaacaacaacaaca

SEQ ID NO: 234 - RNA, 21 nt, Artificial Sequence
  Synthetic construct
ccgcaguaggaagagaaagcc

SEQ ID NO: 235 - RNA, 21 nt, Artificial Sequence
  Synthetic construct
aaaaaaaaaagaaaucauaaa

SEQ ID NO: 236 - RNA, 21 nt, Artificial Sequence
  Synthetic construct
gagagaagaaagaagaagacg

SEQ ID NO: 237 - RNA, 21 nt, Artificial Sequence
  Synthetic construct
caauuaaaaauacuuaccaaa

SEQ ID NO: 238 - RNA, 21 nt, Artificial Sequence
  Synthetic construct
gcaaacagaguaagcgaaacg

SEQ ID NO: 239 - RNA, 21 nt, Artificial Sequence
  Synthetic construct
gcgaagaagacgaacgcaaag

SEQ ID NO: 240 - RNA, 21 nt, Artificial Sequence
  Synthetic construct
uuaggacuguauugacuggcc

SEQ ID NO: 241 - RNA, 21 nt, Artificial Sequence
  Synthetic construct
aucaucggaauucggaaaaag

SEQ ID NO: 242 - RNA, 21 nt, Artificial Sequence
  Synthetic construct
aaaacaaaaguuaaagcagac

SEQ ID NO: 243 - RNA, 21 nt, Artificial Sequence
  Synthetic construct
uuuaucucaaauaagaaggca

SEQ ID NO: 244 - RNA, 21 nt, Artificial Sequence
  Synthetic construct
gguggggaggugagauuucuu

SEQ ID NO: 245 - RNA, 21 nt, Artificial Sequence
  Synthetic construct
ugauuaggaaacuacaaagcc

SEQ ID NO: 246 - RNA, 21 nt, Artificial Sequence
  Synthetic construct
cauuuuucaauuucauaaaac

SEQ ID NO: 247 - RNA, 21 nt, Artificial Sequence
  Synthetic construct
uuacuuuuaagcccaacaaaa

SEQ ID NO: 248 - RNA, 21 nt, Artificial Sequence
  Synthetic construct
ggcguguguguguguuguuga

SEQ ID NO: 249 - RNA, 21 nt, Artificial Sequence
  Synthetic construct
guggugaaggggaagguuuag

SEQ ID NO: 250 - RNA, 21 nt, Artificial Sequence
  Synthetic construct
uuguuuuuuuuugguuugguu

SEQ ID NO: 251 - RNA, 1331 nt, Artificial Sequence
  Synthetic construct
aggauuauuacaucaaaacaaaaagccgccaccaugcugguauucaaccugcgcauccugcugaacaacgccgccuuccgcaacggccacaacuucauggugcgcaacuuccgcugcggccagccccugcagaaccgggugcagcugaagggccgcgaccugcugacccugaagaacuucaccggcgaggagauccgguacaugcuguggcugagcgccgaccugaaguuccgcaucaagcagaagggcgaguaccugccccugcugcagggcaagagccugggcaugaucuucgagaagcgcagcacccgcacccgccugagcaccgagacaggcuucgcccugcugggcggccaccccugcuuccugaccacccaggacauccaccugggcgugaacgagagccugaccgacaccgcccgcgugcugagcagcauggccgacgccgugcuggcccgcguguacaagcagagcgaccuggacacccuggccaaggaggccagcauccccaucaucaacggccugagcgaccuguaccaccccauccagauccuggccgacuaccugacccugcaggagcacuacagcagccugaagggccugacccugagcuggaucggcgacggcaacaacauccugcacagcaucaugaugagcgccgccaaguucggcaugcaccugcaggccgccacccccaagggcuacgagcccgacgccagcgugaccaagcuggccgagcaguacgccaaggagaacggcaccaagcugcugcugaccaacgacccccuggaggccgcccacggcggcaacgugcugaucaccgacaccuggaucagcaugggccaggaggaggagaagaagaagcgccugcaggccuuccagggcuaccaggugaccaugaagaccgccaagguggccgccagcgacuggaccuuccugcacugccugccccgcaagcccgaggagguggacgacgagguguucuacagcccccgcagccugguguuccccgaggccgagaaccgcaaguggaccaucauggccgugauggugagccugcugaccgacuacagcccccagcugcagaagcccaaguucugaggucucuaguaaugagcuggagccucgguagccguuccuccugcccgcugggccucccaacgggcccuccuccccuccuugcaccggcccuuccuggucuuugaauaaagucugagugggcagcaucuagaaaaaaaaaaaaaaaaaaaaaaaaaaaaaaaaaaaaaaaaaaaaaaaaaaaaaaaaaaaaaaaaaaaaaaaaaaaaaaaaaaaaaaaaaaaaaaaaaaaa

SEQ ID NO: 252 - RNA, 1334 nt, Artificial Sequence
  Synthetic construct
aggauuauuacaucaaaacaaaaagccgccaccaugcugguauucaaccugcgcauccugcugaacaacgccgccuuccgcaacggccacaacuucauggugcgcaacuuccgcugcggccagccccugcagaaccgggugcagcugaagggccgcgaccugcugacccugaagaacuucaccggcgaggagauccgguacaugcuguggcugagcgccgaccugaaguuccgcaucaagcagaagggcgaguaccugccccugcugcagggcaagagccugggcaugaucuucgagaagcgcagcacccgcacccgccugagcaccgagacaggcuucgcccugcugggcggccaccccugcuuccugaccacccaggacauccaccugggcgugaacgagagccugaccgacaccgcccgcgugcugagcagcauggccgacgccgugcuggcccgcguguacaagcagagcgaccuggacacccuggccaaggaggccagcauccccaucaucaacggccugagcgaccuguaccaccccauccagauccuggccgacuaccugacccugcaggagcacuacagcagccugaagggccugacccugagcuggaucggcgacggcaacaacauccugcacagcaucaugaugagcgccgccaaguucggcaugcaccugcaggccgccacccccaagggcuacgagcccgacgccagcgugaccaagcuggccgagcaguacgccaaggagaacggcaccaagcugcugcugaccaacgacccccuggaggccgcccacggcggcaacgugcugaucaccgacaccuggaucagcaugggccaggaggaggagaagaagaagcgccugcaggccuuccagggcuaccaggugaccaugaagaccgccaagguggccgccagcgacuggaccuuccugcacugccugccccgcaagcccgaggagguggacgacgagguguucuacagcccccgcagccugguguuccccgaggccgagaaccgcaaguggaccaucauggccgugauggugagccugcugaccgacuacagcccccagcugcagaagcccaaguucugaggucucuaguaaugagcuggagccucgguagccguuccuccugcccgcugggccucccaacgggcccuccuccccuccuugcaccggcccuuccuggucuuugaauaaagucugagugggcagcaucuagaaaaaaaaaaaaaaaaaaaaaaaaaaaaaaaaaaaaaaaaaaaaaaaaaaaaaaaaaaaaaaaaaaaaaaaaaaaaaaaaaaaaaaaaaaaaaaaaaaaagcu

SEQ ID NO: 253 - RNA, 1328 nt, Artificial Sequence
  Synthetic construct
aggauuauuacaucaaaacaaaaagccgccaccaugcuguucaaccugcgcauccugcugaacaacgccgccuuccgcaacggccacaacuucauggugcgcaacuuccgcugcggccagccccugcagaacaaggugcagcugaagggccgcgaccugcugacccugaagaacuucaccggcgaggagaucaaguacaugcuguggcugagcgccgaccugaaguuccgcaucaagcagaagggcgaguaccugccccugcugcagggcaagagccugggcaugaucuucgagaagcgcagcacccgcacccgccugagcaccgagacaggcuucgcccugcugggcggccaccccugcuuccugaccacccaggacauccaccugggcgugaacgagagccugaccgacaccgcccgcgugcugagcagcauggccgacgccgugcuggcccgcguguacaagcagagcgaccuggacacccuggccaaggaggccagcauccccaucaucaacggccugagcgaccuguaccaccccauccagauccuggccgacuaccugacccugcaggagcacuacagcagccugaagggccugacccugagcuggaucggcgacggcaacaacauccugcacagcaucaugaugagcgccgccaaguucggcaugcaccugcaggccgccacccccaagggcuacgagcccgacgccagcgugaccaagcuggccgagcaguacgccaaggagaacggcaccaagcugcugcugaccaacgacccccuggaggccgcccacggcggcaacgugcugaucaccgacaccuggaucagcaugggccaggaggaggagaagaagaagcgccugcaggccuuccagggcuaccaggugaccaugaagaccgccaagguggccgccagcgacuggaccuuccugcacugccugccccgcaagcccgaggagguggacgacgagguguucuacagcccccgcagccugguguuccccgaggccgagaaccgcaaguggaccaucauggccgugauggugagccugcugaccgacuacagcccccagcugcagaagcccaaguucugaggucucuaguaaugagcuggagccucgguagccguuccuccugcccgcugggccucccaacgggcccuccuccccuccuugcaccggcccuuccuggucuuugaauaaagucugagugggcagcaucuagaaaaaaaaaaaaaaaaaaaaaaaaaaaaaaaaaaaaaaaaaaaaaaaaaaaaaaaaaaaaaaaaaaaaaaaaaaaaaaaaaaaaaaaaaaaaaaaaaaaa